European Patent Specification EP 4 090 670 B1, published June 4, 2025. Title: Peptide Inhibitors of Interleukin-23 Receptor and Their Use to Treat Inflammatory Diseases. Applicant: Janssen Biotech, Inc. Protagonist Therapeutics, Inc. Application Herewith. The sequence listing filed with the application follows.

SEQUENCE LISTING (536 sequences)

SEQ ID NO: 1 - protein, 14 aa, Artificial sequence
  Synthetic construct
  MISC_FEATURE (1)..(1): Arg is (D)- Arginine
  MISC_FEATURE (2)..(2): Xaa is Abu
  MISC_FEATURE (5)..(5): Xaa is W(7-Ph)
  MISC_FEATURE (6)..(6): Lys is Lys(Ac)
  MISC_FEATURE (8)..(8): Phe is Phe[4-(2-aminoethoxy)]
  MISC_FEATURE (9)..(9): Xaa is 2-Nal
  MISC_FEATURE (10)..(10): Lys is a-MeLys
  MISC_FEATURE (11)..(11): Lys is Lys(Ac)
  MISC_FEATURE (13)..(13): Xaa is dK
  MISC_FEATURE (14)..(14): Xaa is Sarc
RXQTXKCFXKKNXX

SEQ ID NO: 2 - protein, 13 aa, Artificial sequence
  Synthetic construct
  MISC_FEATURE (1)..(1): Xaa is pennicillamine
  MISC_FEATURE (4)..(4): Xaa is 7-methyltryptophan
  MISC_FEATURE (5)..(5): Lys is Lys(Ac)
  MISC_FEATURE (6)..(6): Xaa is Pen
  MISC_FEATURE (7)..(7): Xaa is Phe[4-(2-aminoethoxy)]
  MISC_FEATURE (8)..(8): Xaa is 3-Quin
  MISC_FEATURE (9)..(9): Lys is a-MeLys
  MISC_FEATURE (10)..(10): Lys is Lys(Ac)
  MISC_FEATURE (12)..(12): Leu is (D)Leu
  MISC_FEATURE (13)..(13): Xaa is Sarc
XNTXKXFXKKNLX

SEQ ID NO: 3 - protein, 13 aa, Artificial sequence
  Synthetic construct
  MISC_FEATURE (1)..(1): Xaa is Pen
  MISC_FEATURE (4)..(4): Xaa is W(7-Me)
  MISC_FEATURE (5)..(5): Lys is Lys(Ac)
  MISC_FEATURE (6)..(6): Xaa is Pen
  MISC_FEATURE (7)..(7): Xaa is Phe[4-(2-aminoethoxy)]
  MISC_FEATURE (8)..(8): Xaa is 3-Quin
  MISC_FEATURE (9)..(9): Xaa is THP
  MISC_FEATURE (12)..(12): Lys is D(Lys)
  MISC_FEATURE (13)..(13): Xaa is Sarc
XNTXKXFXXENKX

SEQ ID NO: 4 - protein, 13 aa, Artificial sequence
  Synthetic construct
  MISC_FEATURE (1)..(1): Xaa is Pen
  MISC_FEATURE (4)..(4): Xaa is W(7-Me)
  MISC_FEATURE (5)..(5): Lys is Lys(Ac)
  MISC_FEATURE (6)..(6): Xaa is Pen
  MISC_FEATURE (7)..(7): Phe is Phe[4-(2-aminoethoxy)]
  MISC_FEATURE (8)..(8): Xaa is 3-Quin
  MISC_FEATURE (9)..(9): Lys is a-MeLys
  MISC_FEATURE (10)..(10): Lys is Lys(Ac)
  MISC_FEATURE (12)..(12): His is (D)His
  MISC_FEATURE (13)..(13): Xaa is Sarc
XNTXKXFXKKNHX

SEQ ID NO: 5 - protein, 13 aa, Artificial sequence
  Synthetic construct
  MISC_FEATURE (1)..(1): Xaa is Pen
  MISC_FEATURE (4)..(4): Xaa is W(7-Me)
  MISC_FEATURE (5)..(5): Lys is Lys(Ac)
  MISC_FEATURE (6)..(6): Xaa is Pen
  MISC_FEATURE (7)..(7): Phe is Phe[4-(2-aminoethoxy)]
  MISC_FEATURE (8)..(8): Xaa is 3-Quin
  MISC_FEATURE (9)..(9): Lys is a-MeLys
  MISC_FEATURE (10)..(10): Lys is Lys(Ac)
  MISC_FEATURE (13)..(13): Xaa is Sarc
XNTXKXFXKKNHX

SEQ ID NO: 6 - protein, 13 aa, Artificial sequence
  Synthetic construct
  MISC_FEATURE (1)..(1): Xaa is Pen
  MISC_FEATURE (4)..(4): Xaa is W(7-Me)
  MISC_FEATURE (5)..(5): Lys is Lys(Ac)
  MISC_FEATURE (6)..(6): Xaa is Pen
  MISC_FEATURE (7)..(7): Phe is Phe[4-(2-aminoethoxy)]
  MISC_FEATURE (8)..(8): Xaa is 3-Quin
  MISC_FEATURE (9)..(9): Xaa is THP
  MISC_FEATURE (12)..(12): Leu is (D)Leu
  MISC_FEATURE (13)..(13): Xaa is Sarc
XNTXKXFXXENLX

SEQ ID NO: 7 - protein, 13 aa, Artificial sequence
  Synthetic construct
  MISC_FEATURE (1)..(1): Xaa is Pen
  MISC_FEATURE (4)..(4): Xaa is W(7-Me)
  MISC_FEATURE (5)..(5): Lys is Lys(Ac)
  MISC_FEATURE (6)..(6): Xaa is Pen
  MISC_FEATURE (7)..(7): Phe is Phe[4-(2-aminoethoxy)]
  MISC_FEATURE (8)..(8): Xaa is 3-Quin
  MISC_FEATURE (9)..(9): Lys is a-MeLys
  MISC_FEATURE (10)..(10): Lys is Lys(Ac)
  MISC_FEATURE (12)..(12): Lys is (D)Lys
  MISC_FEATURE (13)..(13): Xaa is Sarc
XNTXKXFXKKNKX

SEQ ID NO: 8 - protein, 14 aa, Artificial sequence
  Synthetic construct
  MISC_FEATURE (1)..(1): Arg is (D)Arg
  MISC_FEATURE (2)..(2): Xaa is Abu
  MISC_FEATURE (8)..(8): Phe is Phe[4-(2-aminoethoxy)]
  MISC_FEATURE (9)..(9): Xaa is 2-Nal
  MISC_FEATURE (10)..(10): Xaa is THP
  MISC_FEATURE (14)..(14): Tyr is (D)NMeTyr
RXQTWQCFXXENNY

SEQ ID NO: 9 - protein, 14 aa, Artificial sequence
  Synthetic construct
  MISC_FEATURE (1)..(1): Arg is (D)Arg
  MISC_FEATURE (2)..(2): Xaa is Pen
  MISC_FEATURE (7)..(7): Xaa is Pen
  MISC_FEATURE (8)..(8): Phe is Phe[4-(2-aminoethoxy)]
  MISC_FEATURE (9)..(9): Xaa is 2-Nal
  MISC_FEATURE (10)..(10): Xaa is THP
  MISC_FEATURE (14)..(14): Tyr is (D)NMeTyr]
RXQTWQXFXXENNY

SEQ ID NO: 10 - protein, 14 aa, Artificial sequence
  Synthetic construct
  MISC_FEATURE (1)..(1): Arg is (D)Arg
  MISC_FEATURE (2)..(2): Xaa is Pen
  MISC_FEATURE (7)..(7): Xaa is Pen
  MISC_FEATURE (8)..(8): Phe is Phe[4-(2-aminoethoxy)]
  MISC_FEATURE (9)..(9): Xaa is 2-Nal
  MISC_FEATURE (10)..(10): Xaa is THP
  MISC_FEATURE (11)..(11): Glu is aMeGlu
  MISC_FEATURE (14)..(14): Tyr is (D)NMeTyr
RXQTWQXFXXENFY

SEQ ID NO: 11 - protein, 13 aa, Artificial sequence
  Synthetic construct
  MISC_FEATURE (1)..(1): Xaa is Pen
  MISC_FEATURE (4)..(4): Xaa is [W(7-Ph)]
  MISC_FEATURE (5)..(5): Lys is Lys(Ac)
  MISC_FEATURE (6)..(6): Xaa is Pen
  MISC_FEATURE (7)..(7): Phe is Phe[4-(2-aminoethoxy)]
  MISC_FEATURE (8)..(8): Xaa is 3-Quin
  MISC_FEATURE (9)..(9): Xaa is THP
  MISC_FEATURE (12)..(12): Lys is (D)Lys
  MISC_FEATURE (13)..(13): Xaa is Sarc
XNTXKXFXXENKX

SEQ ID NO: 12 - protein, 13 aa, Artificial sequence
  Synthetic construct
  MISC_FEATURE (1)..(1): Xaa is Pen
  MISC_FEATURE (4)..(4): Xaa is W(7-Ph)
  MISC_FEATURE (5)..(5): Lys is Lys(Ac)
  MISC_FEATURE (6)..(6): Xaa is Pen
  MISC_FEATURE (7)..(7): Phe is Phe[4-(2-aminoethoxy)]
  MISC_FEATURE (8)..(8): Xaa is 3-Quin
  MISC_FEATURE (9)..(9): Lys is a-MeLys
  MISC_FEATURE (10)..(10): Lys is Lys(Ac)
  MISC_FEATURE (12)..(12): Lys is (D)Lys
  MISC_FEATURE (13)..(13): Xaa is Sarc
XNTXKXFXKKNKX

SEQ ID NO: 13 - protein, 13 aa, Artificial sequence
  Synthetic construct
  MISC_FEATURE (1)..(1): Xaa is Pen
  MISC_FEATURE (4)..(4): Xaa is W(7-Ph)
  MISC_FEATURE (5)..(5): Lys is Lys(Ac)
  MISC_FEATURE (6)..(6): Xaa is Pen
  MISC_FEATURE (7)..(7): Phe is Phe[4-(2-aminoethoxy)]
  MISC_FEATURE (8)..(8): Xaa is 3-Quin
  MISC_FEATURE (9)..(9): Xaa is THP
  MISC_FEATURE (12)..(12): Leu is (D)Leu
  MISC_FEATURE (13)..(13): Xaa is Sarc
XNTXKXFXXENLX

SEQ ID NO: 14 - protein, 13 aa, Artificial sequence
  Synthetic construct
  MISC_FEATURE (1)..(1): Xaa is Pen
  MISC_FEATURE (4)..(4): Xaa is W(7-Ph)
  MISC_FEATURE (5)..(5): Lys is Lys(Ac)
  MISC_FEATURE (6)..(6): Xaa is Pen
  MISC_FEATURE (7)..(7): Phe is Phe[4-(2-aminoethoxy)]
  MISC_FEATURE (8)..(8): Xaa is 3-Quin
  MISC_FEATURE (9)..(9): Lys is a-MeLys
  MISC_FEATURE (10)..(10): Lys is Lys(Ac)
  MISC_FEATURE (12)..(12): Leu is (D)Leu
  MISC_FEATURE (13)..(13): Xaa is Sarc
XNTXKXFXKKNLX

SEQ ID NO: 15 - protein, 13 aa, Artificial sequence
  Synthetic construct
  MISC_FEATURE (1)..(1): Xaa is Pen
  MISC_FEATURE (4)..(4): Xaa is W(7-Ph)
  MISC_FEATURE (5)..(5): Lys is Lys(Ac)
  MISC_FEATURE (6)..(6): Xaa is Pen
  MISC_FEATURE (7)..(7): Phe is Phe[4-(2-aminoethoxy)]
  MISC_FEATURE (8)..(8): Xaa is 3-quin
  MISC_FEATURE (9)..(9): Xaa is THP
  MISC_FEATURE (13)..(13): Xaa is Sarc
XNTXKXFXXENHX

SEQ ID NO: 16 - protein, 13 aa, Artificial sequence
  Synthetic construct
  MISC_FEATURE (1)..(1): Xaa is Pen
  MISC_FEATURE (4)..(4): Xaa is W(7-Ph)
  MISC_FEATURE (5)..(5): Lys is Lys(Ac)
  MISC_FEATURE (6)..(6): Xaa is Pen
  MISC_FEATURE (7)..(7): Phe is Phe[4-(2-aminoethoxy)]
  MISC_FEATURE (8)..(8): Xaa is 3-Quin
  MISC_FEATURE (9)..(9): Lys is a-MeLys
  MISC_FEATURE (10)..(10): Lys is Lys(Ac)
  MISC_FEATURE (13)..(13): Xaa is Sarc
XNTXKXFXKKNHX

SEQ ID NO: 17 - protein, 13 aa, Artificial sequence
  Synthetic construct
  MISC_FEATURE (1)..(1): Xaa is Abu
  MISC_FEATURE (4)..(4): Xaa is W(7-Me)
  MISC_FEATURE (5)..(5): Lys is Lys(Ac)
  MISC_FEATURE (7)..(7): Phe is Phe[4-(2-aminoethoxy)]
  MISC_FEATURE (8)..(8): Xaa is 2-Nal
  MISC_FEATURE (9)..(9): Lys is a-MeLys
  MISC_FEATURE (10)..(10): Lys is Lys(Ac)
  MISC_FEATURE (12)..(12): Lys is (D)Lys
  MISC_FEATURE (13)..(13): Xaa is Sarc
XQTXKCFXKKNKX

SEQ ID NO: 18 - protein, 13 aa, Artificial sequence
  Synthetic construct
  MISC_FEATURE (1)..(1): Xaa is Abu
  MISC_FEATURE (4)..(4): Xaa is W(7-Ph)
  MISC_FEATURE (5)..(5): Lys is Lys(Ac)
  MISC_FEATURE (7)..(7): Phe is Phe[4-(2-aminoethoxy)]
  MISC_FEATURE (8)..(8): Xaa is 2-Nal
  MISC_FEATURE (9)..(9): Lys is a-MeLys
  MISC_FEATURE (10)..(10): Lys is Lys(Ac)
  MISC_FEATURE (12)..(12): Lys is (D)Lys
  MISC_FEATURE (13)..(13): Xaa is Sarc
XQTXKCFXKKNKX

SEQ ID NO: 19 - protein, 13 aa, Artificial sequence
  Synthetic construct
  MISC_FEATURE (1)..(1): Xaa is Pen
  MISC_FEATURE (4)..(4): Xaa is W(7-Me)
  MISC_FEATURE (5)..(5): Lys is Lys(Ac)
  MISC_FEATURE (6)..(6): Xaa is Pen
  MISC_FEATURE (7)..(7): Phe is Phe[4-(2-aminoethoxy)]
  MISC_FEATURE (8)..(8): Xaa is 2-Nal
  MISC_FEATURE (9)..(9): Lys is a-MeLys
  MISC_FEATURE (10)..(10): Lys is Lys(Ac)
  MISC_FEATURE (12)..(12): Leu is (D)Leu
  MISC_FEATURE (13)..(13): Leu is NMeLeu
XNTXKXFXKKNLL

SEQ ID NO: 20 - protein, 13 aa, Artificial sequence
  Synthetic construct
  MISC_FEATURE (1)..(1): Xaa is Pen
  MISC_FEATURE (4)..(4): Xaa is W(7-Me)
  MISC_FEATURE (5)..(5): Lys is Lys(Ac)
  MISC_FEATURE (6)..(6): Xaa is Pen
  MISC_FEATURE (7)..(7): Phe is Phe[4-(2-aminoethoxy)]
  MISC_FEATURE (8)..(8): Xaa is 2-Nal
  MISC_FEATURE (9)..(9): Lys is a-MeLys
  MISC_FEATURE (10)..(10): Lys is Lys(Ac)
  MISC_FEATURE (12)..(12): Leu is (D)Leu
  MISC_FEATURE (13)..(13): Xaa is Sarc
XNTXKXFXKKNLX

SEQ ID NO: 21 - protein, 13 aa, Artificial sequence
  Synthetic construct
  MISC_FEATURE (1)..(1): Xaa is Pen
  MISC_FEATURE (4)..(4): Xaa is W(7-Me)
  MISC_FEATURE (5)..(5): Lys is Lys(Ac)
  MISC_FEATURE (6)..(6): Xaa is Pen
  MISC_FEATURE (7)..(7): Phe is Phe[4-(2-aminoethoxy)]
  MISC_FEATURE (8)..(8): Xaa is 2-Nal
  MISC_FEATURE (9)..(9): Lys is a-MeLys
  MISC_FEATURE (10)..(10): Lys is Lys(Ac)
  MISC_FEATURE (12)..(12): Lys is (D)Lys
  MISC_FEATURE (13)..(13): Xaa is Sarc
XNTXKXFXKKNKX

SEQ ID NO: 22 - protein, 13 aa, Artificial sequence
  Synthetic construct
  MISC_FEATURE (1)..(1): Xaa is Pen
  MISC_FEATURE (4)..(4): Xaa is W(7-Me)
  MISC_FEATURE (5)..(5): Lys is Lys(Ac)
  MISC_FEATURE (6)..(6): Xaa is Pen
  MISC_FEATURE (7)..(7): Phe is Phe[4-(2-aminoethoxy)]
  MISC_FEATURE (8)..(8): Xaa is 2-Nal
  MISC_FEATURE (9)..(9): Xaa is THP
  MISC_FEATURE (13)..(13): Xaa is Sarc
XNTXKXFXXENHX

SEQ ID NO: 23 - protein, 13 aa, Artificial sequence
  Synthetic construct
  MISC_FEATURE (1)..(1): Xaa is Pen
  MISC_FEATURE (4)..(4): Xaa is W(7-Me)
  MISC_FEATURE (5)..(5): Lys is Lys(Ac)
  MISC_FEATURE (6)..(6): Xaa is Pen
  MISC_FEATURE (7)..(7): Phe is Phe[4-(2-aminoethoxy)]
  MISC_FEATURE (8)..(8): Xaa is 2-Nal
  MISC_FEATURE (9)..(9): Lys is a-MeLys
  MISC_FEATURE (10)..(10): Lys is Lys(Ac)
  MISC_FEATURE (13)..(13): Xaa is Sarc
XNTXKXFXKKNHX

SEQ ID NO: 24 - protein, 13 aa, Artificial sequence
  Synthetic construct
  MISC_FEATURE (1)..(1): Xaa is Pen
  MISC_FEATURE (4)..(4): Xaa is W(7-Me)
  MISC_FEATURE (5)..(5): Lys is Lys(Ac)
  MISC_FEATURE (6)..(6): Xaa is Pen
  MISC_FEATURE (7)..(7): Phe is Phe[4-(2-aminoethoxy)]
  MISC_FEATURE (8)..(8): Xaa is 2-Nal
  MISC_FEATURE (9)..(9): Xaa is THP
  MISC_FEATURE (12)..(12): Leu is (D)Leu
  MISC_FEATURE (13)..(13): Xaa is Sarc
XNTXKXFXXENLX

SEQ ID NO: 25 - protein, 13 aa, Artificial sequence
  Synthetic construct
  MISC_FEATURE (1)..(1): Xaa is Pen
  MISC_FEATURE (4)..(4): Xaa is W(7-Me)
  MISC_FEATURE (5)..(5): Lys is Lys(Ac)
  MISC_FEATURE (6)..(6): Xaa is Pen
  MISC_FEATURE (7)..(7): Phe is Phe[4-(2-aminoethoxy)]
  MISC_FEATURE (8)..(8): Xaa is 2-Nal
  MISC_FEATURE (9)..(9): Lys is a-MeLys
  MISC_FEATURE (10)..(10): Lys is Lys(Ac)
  MISC_FEATURE (12)..(12): Leu is (D)Leu
  MISC_FEATURE (13)..(13): Xaa is Sarc
XNTXKXFXKKNLX

SEQ ID NO: 26 - protein, 13 aa, Artificial sequence
  Synthetic construct
  MISC_FEATURE (1)..(1): Xaa is Pen
  MISC_FEATURE (4)..(4): Xaa is W(7-Me)
  MISC_FEATURE (5)..(5): Lys is Lys(Gly)
  MISC_FEATURE (6)..(6): Xaa is Pen
  MISC_FEATURE (7)..(7): Phe is Phe[4-(2-aminoethoxy)]
  MISC_FEATURE (8)..(8): Xaa is 2-Nal
  MISC_FEATURE (9)..(9): Xaa is THP
  MISC_FEATURE (13)..(13): Xaa is Sarc
XNTXKXFXXENHX

SEQ ID NO: 27 - protein, 13 aa, Artificial sequence
  Synthetic construct
  MISC_FEATURE (1)..(1): Xaa is Pen
  MISC_FEATURE (4)..(4): Xaa is W(7-Me)
  MISC_FEATURE (5)..(5): Lys is Lys(Gly)
  MISC_FEATURE (6)..(6): Xaa is Pen
  MISC_FEATURE (7)..(7): Phe is Phe[4-(2-aminoethoxy)]
  MISC_FEATURE (8)..(8): Xaa is 2-Nal
  MISC_FEATURE (9)..(9): Lys is a-MeLys
  MISC_FEATURE (10)..(10): Lys is Lys(Ac)
  MISC_FEATURE (13)..(13): Xaa is Sarc
XNTXKXFXKKNHX

SEQ ID NO: 28 - protein, 13 aa, Artificial sequence
  Synthetic construct
  MISC_FEATURE (1)..(1): Xaa is Pen
  MISC_FEATURE (4)..(4): Xaa is W(7-Me)
  MISC_FEATURE (5)..(5): Lys is Lys(Gly)
  MISC_FEATURE (6)..(6): Xaa is Pen
  MISC_FEATURE (7)..(7): Phe is Phe[4-(2-aminoethoxy)]
  MISC_FEATURE (8)..(8): Xaa is 2-Nal
  MISC_FEATURE (9)..(9): Xaa is THP
  MISC_FEATURE (12)..(12): Leu is (D)Leu
  MISC_FEATURE (13)..(13): Xaa is SARC
XNTXKXFXXENLX

SEQ ID NO: 29 - protein, 13 aa, Artificial sequence
  Synthetic construct
  MISC_FEATURE (1)..(1): Xaa is Pen
  MISC_FEATURE (4)..(4): Xaa is W(7-Me)
  MISC_FEATURE (5)..(5): Lys is Lys(Gly)
  MISC_FEATURE (6)..(6): Xaa is Pen
  MISC_FEATURE (7)..(7): Phe is Phe[4-(2-aminoethoxy)]
  MISC_FEATURE (8)..(8): Xaa is 2-Nal
  MISC_FEATURE (9)..(9): Lys is a-MeLys
  MISC_FEATURE (10)..(10): Lys is Lys(Ac)
  MISC_FEATURE (12)..(12): Leu is (D)Leu
  MISC_FEATURE (13)..(13): Xaa is Sarc
XNTXKXFXKKNLX

SEQ ID NO: 30 - protein, 13 aa, Artificial sequence
  Synthetic construct
  MISC_FEATURE (1)..(1): Xaa is Pen
  MISC_FEATURE (4)..(4): Xaa is W(7-Me)
  MISC_FEATURE (5)..(5): Lys is Lys(bAla)
  MISC_FEATURE (6)..(6): Xaa is Pen
  MISC_FEATURE (7)..(7): Phe is Phe[4-(2-aminoethoxy)]
  MISC_FEATURE (8)..(8): Xaa is 2-Nal
  MISC_FEATURE (9)..(9): Xaa is THP
  MISC_FEATURE (13)..(13): Xaa is Sarc
XNTXKXFXXENHX

SEQ ID NO: 31 - protein, 13 aa, Artificial sequence
  Synthetic construct
  MISC_FEATURE (1)..(1): Xaa is Pen
  MISC_FEATURE (4)..(4): Xaa isW(7-Me)
  MISC_FEATURE (5)..(5): Lys is Lys(bAla)
  MISC_FEATURE (6)..(6): Xaa is Pen
  MISC_FEATURE (7)..(7): Phe is Phe[4-(2-aminoethoxy)]
  MISC_FEATURE (8)..(8): Xaa is 2-Nal
  MISC_FEATURE (9)..(9): Lys is a-MeLys
  MISC_FEATURE (10)..(10): Lys is Lys(Ac)
  MISC_FEATURE (13)..(13): Xaa is Sarc
XNTXKXFXKKNHX

SEQ ID NO: 32 - protein, 13 aa, Artificial sequence
  Synthetic construct
  MISC_FEATURE (1)..(1): Xaa is Pen
  MISC_FEATURE (4)..(4): Xaa is W(7-Et)
  MISC_FEATURE (5)..(5): Lys is Lys(Ac)
  MISC_FEATURE (6)..(6): Xaa is Pen
  MISC_FEATURE (7)..(7): Phe is Phe[4-(2-aminoethoxy)]
  MISC_FEATURE (8)..(8): Xaa is 2-Nal
  MISC_FEATURE (9)..(9): Xaa is THP
  MISC_FEATURE (13)..(13): Xaa is Sarc
XNTXKXFXXENHX

SEQ ID NO: 33 - protein, 13 aa, Artificial sequence
  Synthetic construct
  MISC_FEATURE (1)..(1): Xaa is Pen
  MISC_FEATURE (4)..(4): Xaa is W(7-Et)
  MISC_FEATURE (5)..(5): Lys is Lys(Ac)
  MISC_FEATURE (6)..(6): Xaa is Pen
  MISC_FEATURE (7)..(7): Phe is Phe[4-(2-aminoethoxy)]
  MISC_FEATURE (8)..(8): Xaa is 2-Nal
  MISC_FEATURE (9)..(9): Lys is a-MeLys
  MISC_FEATURE (10)..(10): Lys is Lys(Ac)
  MISC_FEATURE (13)..(13): Xaa is Sarc
XNTXKXFXKKNHX

SEQ ID NO: 34 - protein, 13 aa, Artificial sequence
  Synthetic construct
  MISC_FEATURE (1)..(1): Xaa is Pen
  MISC_FEATURE (4)..(4): Xaa is W(7-Me)
  MISC_FEATURE (5)..(5): Lys is Lys(Ac)
  MISC_FEATURE (6)..(6): Xaa is Pen
  MISC_FEATURE (7)..(7): Phe is Phe[4-(2-aminoethoxy)]
  MISC_FEATURE (8)..(8): Xaa is W(7-Et)]
  MISC_FEATURE (9)..(9): Lys is a-MeLys
  MISC_FEATURE (10)..(10): Lys is Lys(Ac)
  MISC_FEATURE (13)..(13): Xaa is Sarc
XNTXKXFXKKNHX

SEQ ID NO: 35 - protein, 13 aa, Artificial sequence
  Synthetic construct
  MISC_FEATURE (1)..(1): Xaa is Pen
  MISC_FEATURE (4)..(4): Xaa is W(7-Me)
  MISC_FEATURE (5)..(5): Lys is Lys(Ac)
  MISC_FEATURE (6)..(6): Xaa is Pen
  MISC_FEATURE (7)..(7): Phe is Phe[4-(2-aminoethoxy)]
  MISC_FEATURE (8)..(8): Xaa is W(4-Me)
  MISC_FEATURE (9)..(9): Lys is a-MeLys
  MISC_FEATURE (10)..(10): Lys is Lys(Ac)
  MISC_FEATURE (13)..(13): Xaa is Sarc
XNTXKXFXKKNHX

SEQ ID NO: 36 - protein, 13 aa, Artificial sequence
  Synthetic construct
  MISC_FEATURE (1)..(1): Xaa is Pen
  MISC_FEATURE (4)..(4): Xaa is W(7-Me)
  MISC_FEATURE (5)..(5): Lys is Lys(Ac)
  MISC_FEATURE (6)..(6): Xaa is Pen
  MISC_FEATURE (7)..(7): Phe is Phe[4-(2-aminoethoxy)]
  MISC_FEATURE (8)..(8): Xaa is W(6-Me)
  MISC_FEATURE (9)..(9): Lys is a-MeLys
  MISC_FEATURE (10)..(10): Lys is Lys(Ac)
  MISC_FEATURE (13)..(13): Xaa is Sarc
XNTXKXFXKKNHX

SEQ ID NO: 37 - protein, 13 aa, Artificial sequence
  Synthetic construct
  MISC_FEATURE (1)..(1): Xaa is Pen
  MISC_FEATURE (4)..(4): Xaa is W(7-Me)
  MISC_FEATURE (5)..(5): Lys is Lys(Ac)
  MISC_FEATURE (6)..(6): Xaa is Pen
  MISC_FEATURE (7)..(7): Phe is Phe[4-(2-aminoethoxy)]
  MISC_FEATURE (8)..(8): Xaa is W(4-OMe)
  MISC_FEATURE (9)..(9): Lys is a-MeLys
  MISC_FEATURE (10)..(10): Lys is Lys(Ac)
  MISC_FEATURE (13)..(13): Xaa is Sarc
XNTXKXFXKKNHX

SEQ ID NO: 38 - protein, 13 aa, Artificial sequence
  Synthetic construct
  MISC_FEATURE (1)..(1): Xaa is pen
  MISC_FEATURE (4)..(4): Xaa is W(7-Me)
  MISC_FEATURE (5)..(5): Lys is Lys(Ac)
  MISC_FEATURE (6)..(6): Xaa is Pen
  MISC_FEATURE (7)..(7): Phe is Phe[4-(2-aminoethoxy)]
  MISC_FEATURE (8)..(8): Xaa is W(7-i-Pr)
  MISC_FEATURE (9)..(9): Lys is a-MeLys
  MISC_FEATURE (10)..(10): Lys is Lys(Ac)
  MISC_FEATURE (13)..(13): Xaa is Sarc
XNTXKXFXKKNHX

SEQ ID NO: 39 - protein, 13 aa, Artificial sequence
  Synthetic construct
  MISC_FEATURE (1)..(1): Xaa is Pen
  MISC_FEATURE (4)..(4): Xaa is W(7-Me)
  MISC_FEATURE (5)..(5): Lys is Lys(Ac)
  MISC_FEATURE (6)..(6): Xaa is Pen
  MISC_FEATURE (7)..(7): Phe is Phe[4-(2-aminoethoxy)]
  MISC_FEATURE (8)..(8): Xaa is W(7-nPr)
  MISC_FEATURE (9)..(9): Lys is a-MeLys
  MISC_FEATURE (10)..(10): Lys is Lys(Ac)
  MISC_FEATURE (13)..(13): Xaa is Sarc
XNTXKXFXKKNHX

SEQ ID NO: 40 - protein, 13 aa, Artificial sequence
  Synthetic construct
  MISC_FEATURE (1)..(1): Xaa is Pen
  misc_feature (4)..(4): Xaa can be any naturally occurring amino acid
  MISC_FEATURE (5)..(5): Lys is Lys(Ac)
  MISC_FEATURE (6)..(6): Xaa is Pen
  MISC_FEATURE (7)..(7): Phe is Phe[4-(2-aminoethoxy)]
  MISC_FEATURE (8)..(8): Xaa is W(7-OMe)
  MISC_FEATURE (9)..(9): Lys is a-MeLys
  MISC_FEATURE (10)..(10): Lys is Lys(Ac)
  MISC_FEATURE (13)..(13): Xaa is Sarc
XNTXKXFXKKNHX

SEQ ID NO: 41 - protein, 13 aa, Artificial sequence
  Synthetic construct
  MISC_FEATURE (1)..(1): Xaa is Pen
  MISC_FEATURE (4)..(4): Xaa is W(7-Me)
  MISC_FEATURE (5)..(5): Lys is Lys(Ac)
  MISC_FEATURE (6)..(6): Xaa is Pen
  MISC_FEATURE (7)..(7): Phe is Phe[4-(2-aminoethoxy)]
  MISC_FEATURE (8)..(8): Xaa is W(6-Cl)
  MISC_FEATURE (9)..(9): Lys is a-MeLys
  MISC_FEATURE (10)..(10): Lys is Lys(Ac)
  MISC_FEATURE (13)..(13): Xaa is Sarc
XNTXKXFXKKNHX

SEQ ID NO: 42 - protein, 13 aa, Artificial sequence
  Synthetic construct
  MISC_FEATURE (1)..(1): Xaa is Pen
  MISC_FEATURE (4)..(4): Xaa is W(7-Me)
  MISC_FEATURE (5)..(5): Lys is Lys(Ac)
  MISC_FEATURE (6)..(6): Xaa is Pen
  MISC_FEATURE (7)..(7): Phe is Phe[4-(2-aminoethoxy)]
  MISC_FEATURE (8)..(8): Xaa is W(5-OMe)
  MISC_FEATURE (9)..(9): Lys is a-MeLys
  MISC_FEATURE (10)..(10): Lys is Lys(Ac)
  MISC_FEATURE (13)..(13): Xaa is Sarc
XNTXKXFXKKNHX

SEQ ID NO: 43 - protein, 13 aa, Artificial sequence
  Synthetic construct
  MISC_FEATURE (1)..(1): Xaa is Pen
  MISC_FEATURE (4)..(4): Xaa is W(7-Me)
  MISC_FEATURE (5)..(5): Lys is Lys(Ac)
  MISC_FEATURE (6)..(6): Xaa is Pen
  MISC_FEATURE (7)..(7): Phe is Phe[4-(2-aminoethoxy)]
  MISC_FEATURE (8)..(8): Xaa is W(3-MePh)
  MISC_FEATURE (9)..(9): Lys is a-MeLys
  MISC_FEATURE (10)..(10): Lys is Lys(Ac)
  MISC_FEATURE (13)..(13): Xaa is Sarc
XNTXKXFXKKNHX

SEQ ID NO: 44 - protein, 13 aa, Artificial sequence
  Synthetic construct
  MISC_FEATURE (1)..(1): Xaa is Pen
  MISC_FEATURE (4)..(4): Xaa is W(7-Me)
  MISC_FEATURE (5)..(5): Lys is Lys(Ac)
  MISC_FEATURE (6)..(6): Xaa is Pen
  MISC_FEATURE (7)..(7): Phe is Phe[4-(2-aminoethoxy)]
  MISC_FEATURE (8)..(8): Xaa is W(6-Ph)
  MISC_FEATURE (9)..(9): Lys is a-MeLys
  MISC_FEATURE (10)..(10): Lys is Lys(Ac)
  MISC_FEATURE (13)..(13): Xaa is Sarc
XNTXKXFXKKNHX

SEQ ID NO: 45 - protein, 13 aa, Artificial sequence
  Synthetic construct
  MISC_FEATURE (1)..(1): Xaa is Pen
  MISC_FEATURE (4)..(4): Xaa is W(7-Me)
  MISC_FEATURE (5)..(5): Lys is Lys(Ac)
  MISC_FEATURE (6)..(6): Xaa is Pen
  MISC_FEATURE (7)..(7): Phe is Phe[4-(2-aminoethoxy)]
  MISC_FEATURE (8)..(8): Xaa is W(6-Et)
  MISC_FEATURE (9)..(9): Lys is a-MeLys
  MISC_FEATURE (10)..(10): Lys is Lys(Ac)
  MISC_FEATURE (13)..(13): Xaa is Sarc
XNTXKXFXKKNHX

SEQ ID NO: 46 - protein, 13 aa, Artificial sequence
  Synthetic construct
  MISC_FEATURE (1)..(1): Xaa is Pen
  MISC_FEATURE (4)..(4): Xaa is W(7-(2-FPh)
  MISC_FEATURE (5)..(5): Lys is Lys(Ac)
  MISC_FEATURE (6)..(6): Xaa is Pen
  MISC_FEATURE (7)..(7): Phe is Phe[4-(2-aminoethoxy)]
  MISC_FEATURE (8)..(8): Xaa is 2-Nal
  MISC_FEATURE (9)..(9): Lys is a-MeLys
  MISC_FEATURE (10)..(10): Lys is Lys(Ac)
  MISC_FEATURE (13)..(13): Xaa is Sarc
XNTXKXFXKKNHX

SEQ ID NO: 47 - protein, 13 aa, Artificial sequence
  Synthetic construct
  MISC_FEATURE (1)..(1): Xaa is Pen
  MISC_FEATURE (4)..(4): Xaa is W(7-Me)
  MISC_FEATURE (5)..(5): Lys is Lys(Ac)
  MISC_FEATURE (6)..(6): Xaa is Pen
  MISC_FEATURE (7)..(7): Phe is Phe[4-(2-aminoethoxy)]
  MISC_FEATURE (8)..(8): Xaa is 2-Nal
  MISC_FEATURE (9)..(9): Lys is a-MeLys
  MISC_FEATURE (10)..(10): Lys is Lys(Ac)
  MISC_FEATURE (12)..(12): Leu is (D)Leu
  MISC_FEATURE (13)..(13): Tyr is (D)NMeTyr
XNTXKXFXKKNLY

SEQ ID NO: 48 - protein, 13 aa, Artificial sequence
  Synthetic construct
  MISC_FEATURE (1)..(1): Xaa is Pen
  MISC_FEATURE (4)..(4): Xaa is W(7-Me)
  MISC_FEATURE (5)..(5): Lys is Lys(Ac)
  MISC_FEATURE (6)..(6): Xaa is Pen
  MISC_FEATURE (7)..(7): Phe is Phe[4-(2-aminoethoxy)]
  MISC_FEATURE (8)..(8): Lys is a-MeLys
  MISC_FEATURE (9)..(9): Lys is a-MeLys
  MISC_FEATURE (10)..(10): Lys is Lys(Ac)
  MISC_FEATURE (12)..(12): Lys is (D)Lys
  MISC_FEATURE (13)..(13): Tyr is (D)NMeTyr
XNTXKXFXKKNKY

SEQ ID NO: 49 - protein, 13 aa, Artificial sequence
  Synthetic construct
  MISC_FEATURE (1)..(1): Xaa is Pen
  MISC_FEATURE (4)..(4): Xaa is W(7-(2-OMePh)
  MISC_FEATURE (5)..(5): Lys is Lys(Ac)
  MISC_FEATURE (6)..(6): Xaa is Pen
  MISC_FEATURE (7)..(7): Phe is Phe[4-(2-aminoethoxy)]
  MISC_FEATURE (8)..(8): Xaa is 2-Nal
  MISC_FEATURE (9)..(9): Lys is a-MeLys
  MISC_FEATURE (10)..(10): Lys is Lys(Ac)
  MISC_FEATURE (13)..(13): Xaa is Sarc
XNTXKXFXKKNHX

SEQ ID NO: 50 - protein, 13 aa, Artificial sequence
  Synthetic construct
  MISC_FEATURE (1)..(1): Xaa is Pen
  MISC_FEATURE (4)..(4): Xaa is W(7-Me)
  MISC_FEATURE (5)..(5): Lys is Lys(Ac)
  MISC_FEATURE (6)..(6): Xaa is Pen
  MISC_FEATURE (7)..(7): Phe is Phe[4-(2-aminoethoxy)]
  MISC_FEATURE (8)..(8): Xaa is W(7-Ph)
  MISC_FEATURE (9)..(9): Lys is a-MeLys
  MISC_FEATURE (10)..(10): Lys is Lys(Ac)
  MISC_FEATURE (13)..(13): Xaa is Sarc
XNTXKXFXKKNHX

SEQ ID NO: 51 - protein, 13 aa, Artificial sequence
  Synthetic construct
  MISC_FEATURE (1)..(1): Xaa is Pen
  MISC_FEATURE (4)..(4): Xaa is W(7-Ph)
  MISC_FEATURE (5)..(5): Lys is Lys(Ac)
  MISC_FEATURE (6)..(6): Xaa is Pen
  MISC_FEATURE (7)..(7): Phe is Phe[4-(2-aminoethoxy)]
  MISC_FEATURE (8)..(8): Xaa is 2-Nal
  MISC_FEATURE (9)..(9): Lys is a-MeLys
  MISC_FEATURE (10)..(10): Lys is Lys(Ac)
  MISC_FEATURE (13)..(13): Xaa is Sarc
XNTXKXFXKKNHX

SEQ ID NO: 52 - protein, 13 aa, Artificial sequence
  Synthetic construct
  MISC_FEATURE (1)..(1): Xaa is Pen
  MISC_FEATURE (4)..(4): Xaa is W(7-Ph)
  MISC_FEATURE (5)..(5): Lys is Lys(Ac)
  MISC_FEATURE (6)..(6): Xaa is Pen
  MISC_FEATURE (7)..(7): Phe is Phe[4-(2-aminoethoxy)]-
  MISC_FEATURE (7)..(7): Phe is Phe[4-(2-aminoethoxy)]
  MISC_FEATURE (8)..(8): Xaa is 2-Nal
  MISC_FEATURE (9)..(9): Xaa is THP
  MISC_FEATURE (13)..(13): Xaa is Sarc
XNTXKXFXXENHX

SEQ ID NO: 53 - protein, 13 aa, Artificial sequence
  Synthetic construct
  MISC_FEATURE (1)..(1): Xaa is Pen
  MISC_FEATURE (4)..(4): Xaa is W(7-Me)
  MISC_FEATURE (5)..(5): Lys is Lys(Ac)
  MISC_FEATURE (6)..(6): Xaa is Pen
  MISC_FEATURE (7)..(7): Phe is Phe[4-(2-aminoethoxy)]
  MISC_FEATURE (8)..(8): Xaa is 3-Quin
  MISC_FEATURE (9)..(9): Xaa is THP
  MISC_FEATURE (13)..(13): Xaa is Sarc
XNTXKXFXXENHX

SEQ ID NO: 54 - protein, 13 aa, Artificial sequence
  Synthetic construct
  MISC_FEATURE (1)..(1): Xaa is Pen
  MISC_FEATURE (4)..(4): Xaa is W(7-Me)
  MISC_FEATURE (5)..(5): Lys is Lys(Ac)
  MISC_FEATURE (6)..(6): Xaa is Pen
  MISC_FEATURE (7)..(7): Phe is Phe[4-(2-aminoethoxy)]
  MISC_FEATURE (8)..(8): Xaa is 2-Nal
  MISC_FEATURE (9)..(9): Xaa is THP
  MISC_FEATURE (13)..(13): Xaa is Sarc
XNTXKXFXXENHX

SEQ ID NO: 55 - protein, 13 aa, Artificial sequence
  Synthetic construct
  MISC_FEATURE (1)..(1): Xaa is Pen
  MISC_FEATURE (4)..(4): Xaa is W(7-Me)
  MISC_FEATURE (5)..(5): Lys is Lys(Ac)
  MISC_FEATURE (6)..(6): Xaa is Pen
  MISC_FEATURE (7)..(7): Phe is Phe[4-(2-aminoethoxy)]
  MISC_FEATURE (8)..(8): Xaa is 2-Nal
  MISC_FEATURE (9)..(9): Xaa is THP
  MISC_FEATURE (13)..(13): Xaa is Sarc
XNTXKXFXXENHX

SEQ ID NO: 56 - protein, 13 aa, Artificial sequence
  Synthetic construct
  MISC_FEATURE (1)..(1): Xaa is Pen
  MISC_FEATURE (4)..(4): Xaa is W(7-Me)
  MISC_FEATURE (5)..(5): Lys is Lys(Ac)
  MISC_FEATURE (6)..(6): Xaa is Pen
  MISC_FEATURE (7)..(7): Phe is Phe[4-(2-aminoethoxy)]
  MISC_FEATURE (8)..(8): Xaa is 2-Nal
  MISC_FEATURE (9)..(9): Xaa is THP
  MISC_FEATURE (13)..(13): Xaa is Sarc
XNTXKXFXXENHX

SEQ ID NO: 57 - protein, 13 aa, Artificial sequence
  Synthetic construct
  MISC_FEATURE (1)..(1): Xaa is Pen
  MISC_FEATURE (4)..(4): Xaa is W(7-Me)
  MISC_FEATURE (5)..(5): Lys is Lys(Ac)
  MISC_FEATURE (6)..(6): Xaa is Pen
  MISC_FEATURE (7)..(7): Phe is Phe[4-(2-aminoethoxy)]
  MISC_FEATURE (8)..(8): Xaa is 2-Nal
  MISC_FEATURE (9)..(9): Xaa is THP
  MISC_FEATURE (13)..(13): Tyr is (D)NMeTyr
XNTXKXFXXENHY

SEQ ID NO: 58 - protein, 13 aa, Artificial sequence
  Synthetic construct
  MISC_FEATURE (1)..(1): Xaa is Pen
  MISC_FEATURE (4)..(4): Xaa is W(7-Me)
  MISC_FEATURE (5)..(5): Lys is Lys(Ac)
  MISC_FEATURE (6)..(6): Xaa is Pen
  MISC_FEATURE (7)..(7): Phe is Phe[4-(2-aminoethoxy)]
  MISC_FEATURE (8)..(8): Xaa is 2-Nal
  MISC_FEATURE (9)..(9): Lys is a-MeLys
  MISC_FEATURE (10)..(10): Lys is Lys(Ac)
  MISC_FEATURE (13)..(13): Tyr is (D)NMeTyr
XNTXKXFXKKNFY

SEQ ID NO: 59 - protein, 13 aa, Artificial sequence
  Synthetic construct
  MISC_FEATURE (1)..(1): Xaa is Pen
  MISC_FEATURE (4)..(4): Xaa is W(7-Ph)
  MISC_FEATURE (5)..(5): Lys is Lys(Ac)
  MISC_FEATURE (6)..(6): Xaa is Pen
  MISC_FEATURE (7)..(7): Phe is Phe[4-(2-aminoethoxy)]
  MISC_FEATURE (8)..(8): Xaa is 2-Nal
  MISC_FEATURE (9)..(9): Xaa is THP
  MISC_FEATURE (13)..(13): Xaa is Sarc
XNTXKXFXXENHX

SEQ ID NO: 60 - protein, 13 aa, Artificial sequence
  Synthetic construct
  MISC_FEATURE (1)..(1): Xaa is Pen
  MISC_FEATURE (4)..(4): Xaa is W(7-Ph)
  MISC_FEATURE (5)..(5): Lys is Lys(Ac)
  MISC_FEATURE (6)..(6): Xaa is Pen
  MISC_FEATURE (7)..(7): Phe is Phe[4-(2-aminoethoxy)]
  MISC_FEATURE (8)..(8): Xaa is 2-Nal
  MISC_FEATURE (9)..(9): Xaa is THP
  MISC_FEATURE (13)..(13): Xaa is Sarc
XNTXKXFXXENHX

SEQ ID NO: 61 - protein, 13 aa, Artificial sequence
  Synthetic construct
  MISC_FEATURE (1)..(1): Xaa is Pen
  MISC_FEATURE (4)..(4): Xaa is W(7-Ph)
  MISC_FEATURE (5)..(5): Lys is Lys(Ac)
  MISC_FEATURE (6)..(6): Xaa is Pen
  MISC_FEATURE (7)..(7): Phe is Phe[4-(2-aminoethoxy)]
  MISC_FEATURE (8)..(8): Xaa is 2-Nal
  MISC_FEATURE (9)..(9): Xaa is THP
  MISC_FEATURE (13)..(13): Xaa is Sarc
XNTXKXFXXENHX

SEQ ID NO: 62 - protein, 13 aa, Artificial sequence
  Synthetic construct
  MISC_FEATURE (1)..(1): Xaa is Pen
  MISC_FEATURE (4)..(4): Xaa is W(7-Ph)
  MISC_FEATURE (5)..(5): Lys is Lys(Ac)
  MISC_FEATURE (6)..(6): Xaa is Pen
  MISC_FEATURE (7)..(7): Phe is Phe[4-(2-aminoethoxy)]
  MISC_FEATURE (8)..(8): Xaa is 2-Nal
  MISC_FEATURE (9)..(9): Xaa is THP
  MISC_FEATURE (13)..(13): Tyr is (D)NMeTyr
XNTXKXFXXENHY

SEQ ID NO: 63 - protein, 13 aa, Artificial sequence
  Synthetic construct
  MISC_FEATURE (1)..(1): Xaa is Pen
  MISC_FEATURE (4)..(4): Xaa is W(7-Me)
  MISC_FEATURE (5)..(5): Lys is Lys(Ac)
  MISC_FEATURE (6)..(6): Xaa is Pen
  MISC_FEATURE (7)..(7): Phe is Phe[4-(2-aminoethoxy)]
  MISC_FEATURE (8)..(8): Xaa is 2-Nal
  MISC_FEATURE (9)..(9): Xaa is THP
  MISC_FEATURE (11)..(11): Asn is (D)Asn
  MISC_FEATURE (13)..(13): Xaa is Sarc
XNTXKXFXXENHX

SEQ ID NO: 64 - protein, 13 aa, Artificial sequence
  Synthetic construct
  MISC_FEATURE (1)..(1): Xaa is Pen
  MISC_FEATURE (4)..(4): Xaa is W(7-Me)
  MISC_FEATURE (5)..(5): Lys is Lys(Ac)
  MISC_FEATURE (6)..(6): Xaa is Pen
  MISC_FEATURE (7)..(7): Phe is Phe[4-(2-aminoethoxy)]
  MISC_FEATURE (8)..(8): Xaa is 2-Nal
  MISC_FEATURE (9)..(9): Xaa is THP
  MISC_FEATURE (13)..(13): Xaa is Sarc
XNTXKXFXXEGHX

SEQ ID NO: 65 - protein, 13 aa, Artificial sequence
  Synthetic construct
  MISC_FEATURE (1)..(1): Xaa is Pen
  MISC_FEATURE (4)..(4): Xaa is [W(7-Me)
  MISC_FEATURE (5)..(5): Lys is Lys(Ac)
  MISC_FEATURE (6)..(6): Xaa is Pen
  MISC_FEATURE (7)..(7): Phe is Phe[4-(2-aminoethoxy)]
  MISC_FEATURE (8)..(8): Xaa is 2-Nal
  MISC_FEATURE (9)..(9): Xaa is THP
  MISC_FEATURE (11)..(11): Ser is h(Ser)
  MISC_FEATURE (13)..(13): Xaa is Sarc
XNTXKXFXXESHX

SEQ ID NO: 66 - protein, 13 aa, Artificial sequence
  Synthetic construct
  MISC_FEATURE (1)..(1): Xaa is Pen
  MISC_FEATURE (4)..(4): Xaa is W(7-Me)
  MISC_FEATURE (5)..(5): Lys is Lys(Ac)
  MISC_FEATURE (6)..(6): Xaa is Pen
  MISC_FEATURE (7)..(7): Phe is Phe[4-(2-aminoethoxy)]
  MISC_FEATURE (8)..(8): Xaa is 2-Nal
  MISC_FEATURE (9)..(9): Xaa is THP
XNTXKXFXXENHP

SEQ ID NO: 67 - protein, 13 aa, Artificial sequence
  Synthetic construct
  MISC_FEATURE (1)..(1): Xaa is Pen
  MISC_FEATURE (4)..(4): Xaa is W(7-(2-Nal))
  MISC_FEATURE (5)..(5): Lys is Lys(Ac)
  MISC_FEATURE (6)..(6): Xaa is Pen
  MISC_FEATURE (7)..(7): Phe is Phe[4-(2-aminoethoxy)]
  MISC_FEATURE (8)..(8): Xaa is 2-Nal
  MISC_FEATURE (9)..(9): Xaa is THP
  MISC_FEATURE (13)..(13): Xaa is Sarc
XNTXKXFXXENHX

SEQ ID NO: 68 - protein, 13 aa, Artificial sequence
  Synthetic construct
  MISC_FEATURE (1)..(1): Xaa is Pen
  MISC_FEATURE (4)..(4): Xaa is W(7-3BiPh)
  MISC_FEATURE (5)..(5): Lys is Lys(Ac)
  MISC_FEATURE (6)..(6): Xaa is Pen
  MISC_FEATURE (7)..(7): Phe is Phe[4-(2-aminoethoxy)]
  MISC_FEATURE (8)..(8): Xaa is 2-Nal
  MISC_FEATURE (9)..(9): Xaa is THP
  MISC_FEATURE (13)..(13): Xaa is Sarc
XNTXKXFXXENHX

SEQ ID NO: 69 - protein, 13 aa, Artificial sequence
  Synthetic construct
  MISC_FEATURE (1)..(1): Xaa is Pen
  MISC_FEATURE (4)..(4): Xaa is W(7-(Phenanthren-5-yl))
  MISC_FEATURE (5)..(5): Lys is Lys(Ac)
  MISC_FEATURE (6)..(6): Xaa is Pen
  MISC_FEATURE (7)..(7): Phe is Phe[4-(2-aminoethoxy)]
  MISC_FEATURE (8)..(8): Xaa is 2-Nal
  MISC_FEATURE (9)..(9): Xaa is THP
  MISC_FEATURE (13)..(13): Xaa is Sarc
XNTXKXFXXENHX

SEQ ID NO: 70 - protein, 13 aa, Artificial sequence
  Synthetic construct
  MISC_FEATURE (1)..(1): Xaa is Pen
  MISC_FEATURE (4)..(4): Xaa is W(7-(4-Anthracen-5-yl))
  MISC_FEATURE (5)..(5): Lys is Lys(Ac)
  MISC_FEATURE (6)..(6): Xaa is Pen
  MISC_FEATURE (7)..(7): Phe is Phe[4-(2-aminoethoxy)]
  MISC_FEATURE (8)..(8): Xaa is 2-Nal
  MISC_FEATURE (9)..(9): Xaa is THP
  MISC_FEATURE (13)..(13): Xaa is Sarc
XNTXKXFXXENHX

SEQ ID NO: 71 - protein, 13 aa, Artificial sequence
  Synthetic construct
  MISC_FEATURE (1)..(1): Xaa is Pen
  MISC_FEATURE (4)..(4): Xaa is W(7-(1-Nal))
  MISC_FEATURE (5)..(5): Lys is Lys(Ac)
  MISC_FEATURE (6)..(6): Xaa is Pen
  MISC_FEATURE (7)..(7): Phe is Phe[4-(2-aminoethoxy)]
  MISC_FEATURE (8)..(8): Xaa is 2-Nal
  MISC_FEATURE (9)..(9): Xaa is THP
  MISC_FEATURE (13)..(13): Xaa is Sarc
XNTXKXFXXENHX

SEQ ID NO: 72 - protein, 13 aa, Artificial sequence
  Synthetic construct
  MISC_FEATURE (1)..(1): Xaa is Pen
  MISC_FEATURE (4)..(4): Xaa is W(7-(4BiPh))
  MISC_FEATURE (5)..(5): Lys is Lys(Ac)
  MISC_FEATURE (6)..(6): Xaa is Pen
  MISC_FEATURE (7)..(7): Phe is Phe[4-(2-aminoethoxy)]
  MISC_FEATURE (8)..(8): Xaa is 2-Nal
  MISC_FEATURE (9)..(9): Xaa is THP
  MISC_FEATURE (13)..(13): Xaa is Sarc
XNTXKXFXXENHX

SEQ ID NO: 73 - protein, 13 aa, Artificial sequence
  Synthetic construct
  MISC_FEATURE (1)..(1): Xaa is Pen
  MISC_FEATURE (4)..(4): Xaa is W(7-(3,5-t-Bu-Ph))
  MISC_FEATURE (5)..(5): Lys is Lys(Ac)
  MISC_FEATURE (6)..(6): Xaa is Pen
  MISC_FEATURE (7)..(7): Phe is Phe[4-(2-aminoethoxy)]
  MISC_FEATURE (8)..(8): Xaa is 2-Nal
  MISC_FEATURE (9)..(9): Xaa is THP
  MISC_FEATURE (13)..(13): Xaa is Sarc
XNTXKXFXXENHX

SEQ ID NO: 74 - protein, 13 aa, Artificial sequence
  Synthetic construct
  MISC_FEATURE (1)..(1): Xaa is Pen
  MISC_FEATURE (4)..(4): Xaa is W(7-Me)
  MISC_FEATURE (5)..(5): Lys is Lys(Ac)
  MISC_FEATURE (6)..(6): Xaa is Pen
  MISC_FEATURE (7)..(7): Phe is Phe(4)
  MISC_FEATURE (8)..(8): Xaa is 2-Nal
  MISC_FEATURE (9)..(9): Xaa is THP
  MISC_FEATURE (13)..(13): Xaa is Sarc
XNTXKXFXXENHX

SEQ ID NO: 75 - protein, 13 aa, Artificial sequence
  Synthetic construct
  MISC_FEATURE (1)..(1): Xaa is Pen
  MISC_FEATURE (4)..(4): Xaa is W(7-Me)
  MISC_FEATURE (5)..(5): Lys is Lys(Ac)
  MISC_FEATURE (6)..(6): Xaa is Pen
  MISC_FEATURE (7)..(7): Phe is Phe(4-OMe)
  MISC_FEATURE (8)..(8): Xaa is 2-Nal
  MISC_FEATURE (9)..(9): Xaa is THP
  MISC_FEATURE (13)..(13): Xaa is Sarc
XNTXKXFXXENHX

SEQ ID NO: 76-77 - skipped (2 entries)

SEQ ID NO: 78 - protein, 12 aa, Artificial sequence
  Synthetic construct
  MISC_FEATURE (1)..(1): Xaa is Pen
  MISC_FEATURE (4)..(4): Xaa is W(7-Me)
  MISC_FEATURE (5)..(5): Lys is Lys(Ac)
  MISC_FEATURE (6)..(6): Xaa is Pen
  MISC_FEATURE (7)..(7): Phe is Phe[4-(2-aminoethoxy)]
  MISC_FEATURE (8)..(8): Xaa is 3-Quin
  MISC_FEATURE (9)..(9): Lys is a-MeLys
  MISC_FEATURE (10)..(10): Lys is Lys(Ac)
  MISC_FEATURE (12)..(12): Xaa is 2-Pal
XNTXKXFXKKNX

SEQ ID NO: 79 - protein, 12 aa, Artificial sequence
  Synthetic construct
  MISC_FEATURE (1)..(1): Xaa is Pen
  MISC_FEATURE (4)..(4): Xaa is W(7-Me)
  MISC_FEATURE (5)..(5): Lys is Lys(Ac)
  MISC_FEATURE (6)..(6): Xaa is Pen
  MISC_FEATURE (7)..(7): Phe is Phe[4-(2-aminoethoxy)]
  MISC_FEATURE (8)..(8): Xaa  is 2-Nal
  MISC_FEATURE (9)..(9): Lys is a-MeLys
  MISC_FEATURE (10)..(10): Lys is Lys(Ac)
  MISC_FEATURE (12)..(12): Xaa is 2-Pal
XNTXKXFXKKNX

SEQ ID NO: 80 - protein, 12 aa, Artificial sequence
  Synthetic construct
  MISC_FEATURE (1)..(1): Xaa is Pen
  MISC_FEATURE (4)..(4): Xaa is W(7-Me)
  MISC_FEATURE (5)..(5): Lys is Lys(Ac)
  MISC_FEATURE (6)..(6): Xaa is Pen
  MISC_FEATURE (7)..(7): Phe is Phe[4-(2-aminoethoxy)]
  MISC_FEATURE (8)..(8): Xaa is 2-Nal
  MISC_FEATURE (9)..(9): Lys is a-MeLys
  MISC_FEATURE (10)..(10): Lys is Lys(Ac)
  MISC_FEATURE (12)..(12): Xaa is 3-Pal
XNTXKXFXKKNX

SEQ ID NO: 81 - protein, 13 aa, Artificial sequence
  Synthetic construct
  MISC_FEATURE (1)..(1): Xaa is Pen
  MISC_FEATURE (4)..(4): Xaa is W(7-Me)
  MISC_FEATURE (5)..(5): Lys is Lys(Ac)
  MISC_FEATURE (6)..(6): Xaa is Pen
  MISC_FEATURE (7)..(7): Phe is Phe[4-(2-aminoethoxy)]
  MISC_FEATURE (8)..(8): Xaa is 2-Nal
  MISC_FEATURE (9)..(9): Xaa is THP
  MISC_FEATURE (10)..(10): Lys is Lys(Ac)
  MISC_FEATURE (13)..(13): Xaa is Sarc
XNTXKXFXXKNHX

SEQ ID NO: 82 - protein, 13 aa, Artificial sequence
  Synthetic construct
  MISC_FEATURE (1)..(1): Xaa is Pen
  MISC_FEATURE (4)..(4): Xaa is W(7-Me)
  MISC_FEATURE (5)..(5): Lys is Lys(Ac)
  MISC_FEATURE (6)..(6): Xaa is Pen
  MISC_FEATURE (7)..(7): Phe is Phe[4-(2-aminoethoxy)]
  MISC_FEATURE (8)..(8): Xaa is 2-Nal
  MISC_FEATURE (9)..(9): Lys is a-MeLys
  MISC_FEATURE (10)..(10): Lys is Lys(Ac)
  MISC_FEATURE (13)..(13): Tyr is (D)NMeTyr
XNTXKXFXKKNHY

SEQ ID NO: 83 - protein, 14 aa, Artificial sequence
  Synthetic construct
  MISC_FEATURE (1)..(1): Arg is (D)Arg
  MISC_FEATURE (2)..(2): Xaa is Pen
  MISC_FEATURE (5)..(5): Xaa is W(7-Me)
  MISC_FEATURE (6)..(6): Lys is Lys(Ac)
  MISC_FEATURE (7)..(7): Xaa is Pen
  MISC_FEATURE (8)..(8): Phe is Phe[4-(2-aminoethoxy)]
  MISC_FEATURE (9)..(9): Xaa is 2-Nal
  MISC_FEATURE (10)..(10): Lys is Lys(Ac)
  MISC_FEATURE (14)..(14): Tyr is (D)NMeTyr
RXNTXKXFXKENHY

SEQ ID NO: 84 - protein, 13 aa, Artificial sequence
  Synthetic construct
  MISC_FEATURE (1)..(1): xaa is Pen
  MISC_FEATURE (4)..(4): Xaa is W(7-Me)
  MISC_FEATURE (5)..(5): Lys is Lys(Ac)
  MISC_FEATURE (6)..(6): Xaa is Pen
  MISC_FEATURE (7)..(7): Phe is Phe[4-(2-aminoethoxy)]
  MISC_FEATURE (8)..(8): Xaa is 2-Nal
  MISC_FEATURE (9)..(9): Lys is a-MeLys
  MISC_FEATURE (10)..(10): Lys is Lys(Ac)
  MISC_FEATURE (12)..(12): Phe is Phe[4-aminomethyl]
  MISC_FEATURE (13)..(13): Tyr is (D)NMeTyr
XNTXKXFXKKNFY

SEQ ID NO: 85 - protein, 12 aa, Artificial sequence
  Synthetic construct
  MISC_FEATURE (1)..(1): Xaa is Pen
  MISC_FEATURE (4)..(4): Xaa is W(7-Me)
  MISC_FEATURE (5)..(5): Xaa is Cit
  MISC_FEATURE (6)..(6): Xaa is Pen
  MISC_FEATURE (7)..(7): Phe is Phe[4-(2-aminoethoxy)]
  MISC_FEATURE (8)..(8): Xaa is 2-Nal
  MISC_FEATURE (9)..(9): Leu is a-MeLeu
  MISC_FEATURE (10)..(10): Lys is Lys(Ac)
  MISC_FEATURE (12)..(12): His is (D)His
XNTXXXFXLKNH

SEQ ID NO: 86 - protein, 12 aa, Artificial sequence
  Synthetic construct
  MISC_FEATURE (1)..(1): Xaa is Pen
  MISC_FEATURE (4)..(4): Xaa is W(7-Me)
  MISC_FEATURE (5)..(5): Lys is Lys(Ac)
  MISC_FEATURE (6)..(6): Xaa is Pen
  MISC_FEATURE (7)..(7): Phe is Phe[4-(2-aminoethoxy)]
  MISC_FEATURE (8)..(8): Xaa is 2-Nal
  MISC_FEATURE (9)..(9): Lys is a-MeLys
  MISC_FEATURE (10)..(10): Lys is Lys(Ac)
  MISC_FEATURE (12)..(12): His is (D)His
XNTXKXFXKKNH

SEQ ID NO: 87 - protein, 14 aa, Artificial sequence
  Synthetic construct
  MISC_FEATURE (1)..(1): Arg is (D)Arg
  MISC_FEATURE (2)..(2): Xaa is Pen
  MISC_FEATURE (5)..(5): Xaa is W(7-Me)
  MISC_FEATURE (6)..(6): Lys is Lys(Ac)
  MISC_FEATURE (7)..(7): Xaa is Pen
  MISC_FEATURE (8)..(8): Xaa is Phe[4-(2-aminoethoxy)]
  MISC_FEATURE (9)..(9): Xaa is 2-Nal
  MISC_FEATURE (10)..(10): Xaa is THP
  MISC_FEATURE (13)..(13): His is (D)His
  MISC_FEATURE (14)..(14): His is (D)NMeTyr
RXNTXKXFXXENHY

SEQ ID NO: 88 - protein, 14 aa, Artificial sequence
  Synthetic construct
  MISC_FEATURE (1)..(1): Arg is (D)Arg
  MISC_FEATURE (2)..(2): Xaa is Pen
  MISC_FEATURE (5)..(5): Xaa is W(7-Me)
  MISC_FEATURE (6)..(6): Lys is Lys(Ac)
  MISC_FEATURE (7)..(7): Xaa is Pen
  MISC_FEATURE (8)..(8): Phe is Phe[4-(2-aminoethoxy)]
  MISC_FEATURE (9)..(9): Xaa is 2-Nal
  MISC_FEATURE (10)..(10): Xaa is THP
  MISC_FEATURE (13)..(13): Tyr is (D)NMeTyr
RXNTXKXFXXENNY

SEQ ID NO: 89 - protein, 13 aa, Artificial sequence
  Synthetic construct
  MISC_FEATURE (1)..(1): Xaa is Pen
  MISC_FEATURE (4)..(4): Xaa is W(7-Me)
  MISC_FEATURE (5)..(5): Lys is Lys(Ac)
  MISC_FEATURE (6)..(6): Xaa is Pen
  MISC_FEATURE (7)..(7): Phe is Phe[4-(2-aminoethoxy)]
  MISC_FEATURE (8)..(8): Xaa is 2-Nal
  MISC_FEATURE (9)..(9): Lys is a-MeLys
  MISC_FEATURE (10)..(10): Lys is Lys(Ac)
  MISC_FEATURE (13)..(13): Tyr is (D)NMeTyr
XNTXKXFXKKNNY

SEQ ID NO: 90 - protein, 13 aa, Artificial sequence
  Synthetic construct
  MISC_FEATURE (1)..(1): Xaa is Pen
  MISC_FEATURE (4)..(4): Xaa is W(7-Me)
  MISC_FEATURE (5)..(5): Lys is Lys(Ac)
  MISC_FEATURE (6)..(6): Xaa is Pen
  MISC_FEATURE (7)..(7): Phe is Phe[4-(2-aminoethoxy)]
  MISC_FEATURE (8)..(8): Xaa is 2-Nal
  MISC_FEATURE (9)..(9): Lys is a-MeLys
  MISC_FEATURE (10)..(10): Lys is Lys(Ac)
  MISC_FEATURE (12)..(12): Val is (D)Val
  MISC_FEATURE (13)..(13): Tyr is (D)NMeTyr
XNTXKXFXKKNVY

SEQ ID NO: 91 - protein, 13 aa, Artificial sequence
  Synthetic construct
  MISC_FEATURE (1)..(1): Xaa is Pen
  MISC_FEATURE (4)..(4): Xaa is W(7-Me)
  MISC_FEATURE (5)..(5): Lys is Lys(Ac)
  MISC_FEATURE (6)..(6): Xaa is Pen
  MISC_FEATURE (7)..(7): Phe is Phe[4-(2-aminoethoxy)
  MISC_FEATURE (8)..(8): Xaa is 2-Nal
  MISC_FEATURE (9)..(9): Lys is a-MeLys
  MISC_FEATURE (10)..(10): Lys is Lys(Ac)
  MISC_FEATURE (12)..(12): Thr is (D)Thr
  MISC_FEATURE (13)..(13): Tyr is (D)NMeTyr
XNTXKXFXKKNTY

SEQ ID NO: 92 - protein, 13 aa, Artificial sequence
  Synthetic construct
  MISC_FEATURE (1)..(1): Arg is (D)Arg
  MISC_FEATURE (2)..(2): Xaa is Pen
  MISC_FEATURE (5)..(5): Xaa is W(7-Me)
  MISC_FEATURE (6)..(6): Lys is Lys(Ac)
  MISC_FEATURE (7)..(7): Xaa is Pen
  MISC_FEATURE (8)..(8): Phe is Phe[4-(2-aminoethoxy)]
  MISC_FEATURE (9)..(9): Xaa is 2-Nal
  MISC_FEATURE (10)..(10): Xaa is THP
  MISC_FEATURE (13)..(13): His is (D)His
RXNTXKXFXXENH

SEQ ID NO: 93 - protein, 13 aa, Artificial sequence
  Synthetic construct
  MISC_FEATURE (1)..(1): Xaa is Abu
  MISC_FEATURE (4)..(4): Xaa is W(7-Ph)
  MISC_FEATURE (7)..(7): Phe is Phe[4-(2-aminoethoxy)]
  MISC_FEATURE (8)..(8): Xaa is 3-Quin
  MISC_FEATURE (9)..(9): Xaa is THP
  MISC_FEATURE (13)..(13): Xaa is Sarc
XNTXQCFXXENHX

SEQ ID NO: 94 - protein, 13 aa, Artificial sequence
  Synthetic construct
  MISC_FEATURE (1)..(1): Xaa is Abu
  MISC_FEATURE (4)..(4): Xaa is W(7-Me)
  MISC_FEATURE (7)..(7): Phe is Phe[4-(2-aminoethoxy)]
  MISC_FEATURE (8)..(8): Xaa is 3-Quin
  MISC_FEATURE (9)..(9): Xaa is THP
  MISC_FEATURE (13)..(13): Xaa is Sarc
XNTXQCFXXENHX

SEQ ID NO: 95 - protein, 13 aa, Artificial sequence
  Synthetic construct
  MISC_FEATURE (1)..(1): Xaa is Abu
  MISC_FEATURE (4)..(4): Xaa is W(7-Ph)
  MISC_FEATURE (7)..(7): Phe is Phe[4-(2-aminoethoxy)]
  MISC_FEATURE (8)..(8): Xaa is 2-Nal
  MISC_FEATURE (9)..(9): Lys is a-MeLys
  MISC_FEATURE (10)..(10): Lys is Lys(Ac)
  MISC_FEATURE (13)..(13): Xaa is Sarc
XNTXQCFXKKNHX

SEQ ID NO: 96 - protein, 13 aa, Artificial sequence
  Synthetic construct
  MISC_FEATURE (1)..(1): Xaa is Abu
  MISC_FEATURE (4)..(4): Xaa is W(7-Ph)
  MISC_FEATURE (7)..(7): Phe is Phe[4-(2-aminoethoxy)]
  MISC_FEATURE (8)..(8): Xaa is 2-Nal
  MISC_FEATURE (9)..(9): Xaa is THP
  MISC_FEATURE (13)..(13): Xaa is Sarc
XNTXQCFXXENHX

SEQ ID NO: 97 - protein, 13 aa, Artificial sequence
  Synthetic construct
  MISC_FEATURE (1)..(1): Xaa is Abu
  MISC_FEATURE (4)..(4): Xaa is W(7-Me)
  MISC_FEATURE (5)..(5): Lys is Lys(Ac)
  MISC_FEATURE (7)..(7): Phe is Phe[4-(2-aminoethoxy)]
  MISC_FEATURE (8)..(8): Xaa is 2-Nal
  MISC_FEATURE (9)..(9): Lys is a-MeLys
  MISC_FEATURE (10)..(10): Lys is Lys(Ac)
  MISC_FEATURE (13)..(13): Xaa is Sarc
XNTXKCFXKKNHX

SEQ ID NO: 98 - protein, 13 aa, Artificial sequence
  Synthetic construct
  MISC_FEATURE (1)..(1): Xaa is Abu
  MISC_FEATURE (4)..(4): Xaa is W(7-Ph)
  MISC_FEATURE (5)..(5): Lys is Lys(Ac)
  MISC_FEATURE (7)..(7): Phe is Phe[4-(2-aminoethoxy)]
  MISC_FEATURE (8)..(8): Xaa is 2-Nal
  MISC_FEATURE (9)..(9): Xaa is THP
  MISC_FEATURE (13)..(13): Xaa is Sarc
XNTXKCFXXENHX

SEQ ID NO: 99 - protein, 13 aa, Artificial sequence
  Synthetic construct
  MISC_FEATURE (1)..(1): Xaa is Abu
  MISC_FEATURE (4)..(4): Xaa is W(7-Me)
  MISC_FEATURE (5)..(5): Lys is Lys(Ac)
  MISC_FEATURE (7)..(7): Phe is Phe[4-(2-aminoethoxy)]
  MISC_FEATURE (8)..(8): Xaa is 2-Nal
  MISC_FEATURE (9)..(9): Xaa is THP
  MISC_FEATURE (13)..(13): Xaa is Sarc
XNTXKCFXXENHX

SEQ ID NO: 100 - protein, 14 aa, Artificial sequence
  Synthetic construct
  MISC_FEATURE (1)..(1): Arg is (D)Arg
  MISC_FEATURE (2)..(2): Xaa is Abu
  MISC_FEATURE (5)..(5): Xaa is W(7-Me)
  MISC_FEATURE (8)..(8): Phe is Phe[4-(2-aminoethoxy)]
  MISC_FEATURE (9)..(9): Xaa is 2-Nal
  MISC_FEATURE (10)..(10): Xaa is THP
  MISC_FEATURE (13)..(13): Xaa is Sarc
  misc_feature (14)..(14): Xaa can be any naturally occurring amino acid
RXNTXQCFXXENHX

SEQ ID NO: 101 - protein, 14 aa, Artificial sequence
  Synthetic construct
  MISC_FEATURE (1)..(1): Arg is (D)Arg
  MISC_FEATURE (2)..(2): Xaa is Abu
  MISC_FEATURE (5)..(5): Xaa is W(7-Me)
  MISC_FEATURE (8)..(8): Phe is Phe[4-(2-aminoethoxy)]
  MISC_FEATURE (9)..(9): Xaa is 2-Nal
  MISC_FEATURE (10)..(10): Xaa is THP
  MISC_FEATURE (13)..(13): Leu is (D)Leu
  MISC_FEATURE (14)..(14): Xaa is Sarc
RXNTXQCFXXENLX

SEQ ID NO: 102 - protein, 14 aa, Artificial sequence
  Synthetic construct
  MISC_FEATURE (1)..(1): Arg is (D)Arg
  MISC_FEATURE (2)..(2): Xaa is Abu
  MISC_FEATURE (5)..(5): Xaa is W(7-Me)
  MISC_FEATURE (6)..(6): Xaa isCit
  MISC_FEATURE (8)..(8): Phe is Phe[4-(2-aminoethoxy)]
  MISC_FEATURE (9)..(9): Xaa is 2-Nal
  MISC_FEATURE (10)..(10): Xaa is THP
  MISC_FEATURE (14)..(14): Xaa is Sarc
RXNTXXCFXXENHX

SEQ ID NO: 103 - protein, 13 aa, Artificial sequence
  Synthetic construct
  MISC_FEATURE (1)..(1): Xaa is Pen
  MISC_FEATURE (4)..(4): Xaa is W(7-Me)
  MISC_FEATURE (5)..(5): Lys is Lys(Ac)
  MISC_FEATURE (6)..(6): Xaa is Pen
  MISC_FEATURE (7)..(7): Phe is Phe[4-(2-aminoethoxy)]
  MISC_FEATURE (8)..(8): Xaa is 2-Nal
  MISC_FEATURE (9)..(9): Lys is a-MeLys
  MISC_FEATURE (10)..(10): Lys is Lys(Ac)
  MISC_FEATURE (12)..(12): Xaa is 3-Pal
  MISC_FEATURE (13)..(13): Xaa is Sarc
XNTXKXFXKKNXX

SEQ ID NO: 104 - protein, 13 aa, Artificial sequence
  Synthetic construct
  MISC_FEATURE (1)..(1): Xaa is Pen
  MISC_FEATURE (4)..(4): Xaa is W(7-Me)
  MISC_FEATURE (5)..(5): Xaa is Lys(Ac)
  MISC_FEATURE (6)..(6): Xaa is Pen
  MISC_FEATURE (7)..(7): Phe is Phe[4-(2-aminoethoxy)]
  MISC_FEATURE (8)..(8): Xaa is 2-Nal
  MISC_FEATURE (9)..(9): Xaa is THP
  MISC_FEATURE (12)..(12): Xaa is 3-Pal
  MISC_FEATURE (13)..(13): Xaa is Sarc
XNTXKXFXXENXX

SEQ ID NO: 105 - protein, 13 aa, Artificial sequence
  Synthetic construct
  MISC_FEATURE (1)..(1): Xaa is Pen
  MISC_FEATURE (4)..(4): Xaa is W(7-Ph)
  MISC_FEATURE (5)..(5): Lys is Lys(Ac)
  MISC_FEATURE (6)..(6): Xaa is Pen
  MISC_FEATURE (7)..(7): Phe is Phe[4-(2-aminoethoxy)]
  MISC_FEATURE (8)..(8): Xaa is 2-Nal
  MISC_FEATURE (9)..(9): Lys is a-MeLys
  MISC_FEATURE (10)..(10): Lys is Lys(Ac)
  MISC_FEATURE (12)..(12): Xaa is 3-Pal
  MISC_FEATURE (13)..(13): Xaa is Sarc
XNTXKXFXKKNXX

SEQ ID NO: 106 - protein, 13 aa, Artificial sequence
  Synthetic construct
  MISC_FEATURE (1)..(1): Xaa is Pen
  MISC_FEATURE (4)..(4): Xaa is W(7-Ph)
  MISC_FEATURE (5)..(5): Lys is Lys(Ac)
  MISC_FEATURE (6)..(6): Xaa is Pen
  MISC_FEATURE (7)..(7): Phe is Phe[4-(2-aminoethoxy)]
  MISC_FEATURE (8)..(8): Xaa is 2-Nal
  MISC_FEATURE (9)..(9): Xaa is THP
  MISC_FEATURE (12)..(12): Xaa is 3-Pal
  MISC_FEATURE (13)..(13): Xaa is Sarc
XNTXKXFXXENXX

SEQ ID NO: 107 - protein, 13 aa, Artificial sequence
  Synthetic construct
  MISC_FEATURE (1)..(1): Xaa is Pen
  MISC_FEATURE (4)..(4): Xaa is W(7-Me)
  MISC_FEATURE (5)..(5): Xaa is Cit
  MISC_FEATURE (6)..(6): Xaa is Pen
  MISC_FEATURE (7)..(7): Phe is Phe[4-(2-aminoethoxy)]
  MISC_FEATURE (8)..(8): Xaa is 2-Nal
  MISC_FEATURE (9)..(9): Xaa is THP
  MISC_FEATURE (12)..(12): Xaa is 3-Pal
  MISC_FEATURE (13)..(13): Xaa is Sarc
XNTXXXFXXENXX

SEQ ID NO: 108 - protein, 13 aa, Artificial sequence
  Synthetic construct
  MISC_FEATURE (1)..(1): Xaa is Pen
  MISC_FEATURE (4)..(4): Xaa is W(7-Me)
  MISC_FEATURE (6)..(6): Xaa is Pen
  MISC_FEATURE (7)..(7): Phe is Phe[4-(2-aminoethoxy)]
  MISC_FEATURE (8)..(8): Xaa is 2-Nal
  MISC_FEATURE (9)..(9): Xaa is THP
  MISC_FEATURE (12)..(12): Xaa is 3-Pal
  MISC_FEATURE (13)..(13): Xaa is Sarc
XNTXQXFXXENXX

SEQ ID NO: 109 - protein, 13 aa, Artificial sequence
  Synthetic construct
  MISC_FEATURE (1)..(1): Xaa is Pen
  MISC_FEATURE (4)..(4): Xaa is W(7-Me)
  MISC_FEATURE (7)..(7): Phe is Phe[4-(2-aminoethoxy)]
  MISC_FEATURE (8)..(8): Xaa is 2-Nal
  MISC_FEATURE (9)..(9): Xaa is THP
  MISC_FEATURE (12)..(12): Xaa is 3-Pal
  MISC_FEATURE (13)..(13): Xaa is Sarc
XQTXQCFXXENXX

SEQ ID NO: 110 - protein, 13 aa, Artificial sequence
  Synthetic construct
  MISC_FEATURE (1)..(1): Xaa is Abu
  MISC_FEATURE (4)..(4): Xaa is W(7-Me)
  MISC_FEATURE (7)..(7): Phe is Phe[4-(2-aminoethoxy)]
  MISC_FEATURE (8)..(8): Xaa is 2-Nal
  MISC_FEATURE (9)..(9): Lys is a-MeLys
  MISC_FEATURE (10)..(10): Lys is Lys(Ac)
  MISC_FEATURE (12)..(12): Xaa is 3-Pal
  MISC_FEATURE (13)..(13): Xaa is Sarc
XQTXQCFXKKNXX

SEQ ID NO: 111 - protein, 13 aa, Artificial sequence
  Synthetic construct
  MISC_FEATURE (1)..(1): Xaa is Abu
  MISC_FEATURE (4)..(4): Xaa is W(7-Me)
  MISC_FEATURE (5)..(5): Xaa is Cit
  MISC_FEATURE (7)..(7): Phe is Phe[4-(2-aminoethoxy)]
  MISC_FEATURE (8)..(8): Xaa is 2-Nal
  MISC_FEATURE (9)..(9): Xaa is THP
  MISC_FEATURE (12)..(12): Xaa is 3-Pal
  MISC_FEATURE (13)..(13): Xaa is Sarc
XQTXXCFXXENXX

SEQ ID NO: 112 - protein, 13 aa, Artificial sequence
  Synthetic construct
  MISC_FEATURE (1)..(1): Xaa is Abu
  MISC_FEATURE (4)..(4): Xaa is W(7-Me)
  MISC_FEATURE (5)..(5): Xaa is Cit
  MISC_FEATURE (7)..(7): Phe is Phe[4-(2-aminoethoxy)]
  MISC_FEATURE (8)..(8): Xaa is 2-Nal
  MISC_FEATURE (9)..(9): Lys is a-MeLys
  MISC_FEATURE (10)..(10): Lys is Lys(Ac)
  MISC_FEATURE (12)..(12): Xaa is 3-Pal
  MISC_FEATURE (13)..(13): Xaa is Sarc
XQTXXCFXKKNXX

SEQ ID NO: 113 - protein, 13 aa, Artificial sequence
  Synthetic construct
  MISC_FEATURE (1)..(1): Xaa is Abu
  MISC_FEATURE (4)..(4): Xaa is W(7-Me)
  MISC_FEATURE (7)..(7): Phe is Phe[4-(2-aminoethoxy)]
  MISC_FEATURE (8)..(8): Xaa is 2-Nal
  MISC_FEATURE (9)..(9): Xaa is THP
  MISC_FEATURE (12)..(12): Xaa is 3-Pal
  MISC_FEATURE (13)..(13): Xaa is beta-Alanine
XQTXQCFXXENXX

SEQ ID NO: 114 - protein, 13 aa, Artificial sequence
  Synthetic construct
  MISC_FEATURE (1)..(1): Xaa is Abu
  MISC_FEATURE (4)..(4): Xaa is W(7-Me)
  MISC_FEATURE (7)..(7): Phe is Phe[4-(2-aminoethoxy)]
  MISC_FEATURE (8)..(8): Xaa is 2-Nal
  MISC_FEATURE (9)..(9): Xaa is THP
  MISC_FEATURE (12)..(12): Xaa is 3-Pal
  MISC_FEATURE (13)..(13): Xaa is beta-Alanine
XQTXQCFXXENXX

SEQ ID NO: 115 - protein, 13 aa, Artificial sequence
  Synthetic construct
  MISC_FEATURE (1)..(1): Xaa is Pen
  MISC_FEATURE (4)..(4): Xaa is W(7-Me)
  MISC_FEATURE (5)..(5): Lys is Lys(Ac)
  MISC_FEATURE (6)..(6): Xaa is Pen
  MISC_FEATURE (7)..(7): Phe is Phe[4-(2-aminoethoxy)]
  MISC_FEATURE (8)..(8): Xaa is 2-Nal
  MISC_FEATURE (9)..(9): Xaa is THP
  MISC_FEATURE (12)..(12): Xaa is 4-Pal
  MISC_FEATURE (13)..(13): Xaa is Sarc
XNTXKXFXXENXX

SEQ ID NO: 116 - protein, 13 aa, Artificial sequence
  Synthetic construct
  MISC_FEATURE (1)..(1): Xaa is Pen
  MISC_FEATURE (4)..(4): Xaa is W(7-Ph)
  MISC_FEATURE (5)..(5): Lys is Lys(Ac)
  MISC_FEATURE (6)..(6): Xaa is Pen
  MISC_FEATURE (7)..(7): Phe is Phe[4-(2-aminoethoxy)]
  MISC_FEATURE (8)..(8): Xaa is 2-Nal
  MISC_FEATURE (9)..(9): Xaa is THP
  MISC_FEATURE (12)..(12): Xaa is 3-Pal
  MISC_FEATURE (13)..(13): Xaa is beta-Alanine
XNTXKXFXXENXX

SEQ ID NO: 117 - protein, 13 aa, Artificial sequence
  Synthetic construct
  MISC_FEATURE (1)..(1): Xaa is Pen
  MISC_FEATURE (4)..(4): Xaa is W(7-Ph)
  MISC_FEATURE (5)..(5): Lys is Lys(Ac)
  MISC_FEATURE (6)..(6): Xaa is Lys(Ac)
  MISC_FEATURE (7)..(7): Phe is Phe[4-(2-aminoethoxy)]
  MISC_FEATURE (8)..(8): Xaa is 2-Nal
  MISC_FEATURE (9)..(9): Xaa is THP
  MISC_FEATURE (10)..(10): Lys is Lys(Ac)
  MISC_FEATURE (12)..(12): Xaa is 3-Pal
  MISC_FEATURE (13)..(13): Xaa is Sarc
XNTXKXFXXKNXX

SEQ ID NO: 118 - protein, 13 aa, Artificial sequence
  Synthetic construct
  MISC_FEATURE (1)..(1): Xaa is Pen
  MISC_FEATURE (4)..(4): Xaa is W(7-Me)
  MISC_FEATURE (5)..(5): Lys is Lys(Ac)
  MISC_FEATURE (6)..(6): Xaa is Pen
  MISC_FEATURE (7)..(7): Phe is Phe[4-(2-aminoethoxy)]
  MISC_FEATURE (8)..(8): Xaa is 2-Nal
  MISC_FEATURE (9)..(9): Xaa is THP
  MISC_FEATURE (12)..(12): Xaa 3-Quin
  MISC_FEATURE (13)..(13): Xaa Sarc
XNTXKXFXXENXX

SEQ ID NO: 119 - protein, 13 aa, Artificial sequence
  Synthetic construct
  MISC_FEATURE (1)..(1): Xaa is Pen
  MISC_FEATURE (4)..(4): Xaa is W(7-Me)
  MISC_FEATURE (5)..(5): Lys is Lys(Ace)
  MISC_FEATURE (6)..(6): Xaa is Pen
  MISC_FEATURE (7)..(7): Phe is Phe[4-(2-aminoethoxy)]
  MISC_FEATURE (8)..(8): Xaa is 2-Nal
  MISC_FEATURE (9)..(9): Xaa is THP
  MISC_FEATURE (12)..(12): Xaa is 7-Aza-tryptophan
  MISC_FEATURE (13)..(13): Xaa is Sarc
XNTXKXFXXENXX

SEQ ID NO: 120 - protein, 13 aa, Artificial sequence
  Synthetic construct
  MISC_FEATURE (1)..(1): Xaa is Pen
  MISC_FEATURE (4)..(4): Xaa is W(7-Me)
  MISC_FEATURE (5)..(5): Lys is Lys(Ac)
  MISC_FEATURE (6)..(6): Xaa is Pen
  MISC_FEATURE (7)..(7): Phe is Phe[4-(2-aminoethoxy)]
  MISC_FEATURE (8)..(8): Xaa is 2-Nal
  MISC_FEATURE (9)..(9): Lys is a-MeLys
  MISC_FEATURE (10)..(10): Lys is Lys(Ac)
  MISC_FEATURE (12)..(12): Xaa is 3-Pal
  MISC_FEATURE (13)..(13): Tyr is NMeTyr
XNTXKXFXKKNXY

SEQ ID NO: 121 - protein, 13 aa, Artificial sequence
  Synthetic construct
  MISC_FEATURE (1)..(1): Xaa is Pen
  MISC_FEATURE (4)..(4): Xaa is W(7-Me)
  MISC_FEATURE (5)..(5): Lys is Lys(Ac)
  MISC_FEATURE (6)..(6): Xaa is Pen
  MISC_FEATURE (7)..(7): Phe is Phe[4-(2-aminoethoxy)]
  MISC_FEATURE (8)..(8): Xaa is 2-Nal
  MISC_FEATURE (9)..(9): Xaa is THP
  MISC_FEATURE (12)..(12): Xaa is 3-Pal
  MISC_FEATURE (13)..(13): Tyr is NMeTyr
XNTXKXFXXENXY

SEQ ID NO: 122 - protein, 13 aa, Artificial sequence
  Synthetic construct
  MISC_FEATURE (1)..(1): Xaa is Pen
  MISC_FEATURE (4)..(4): Xaa is W(7-Ph)
  MISC_FEATURE (5)..(5): Lys is Lys(Ac)
  MISC_FEATURE (6)..(6): Xaa is Pen
  MISC_FEATURE (7)..(7): Phe is Phe[4-(2-aminoethoxy)]
  MISC_FEATURE (8)..(8): Xaa is 2-Nal
  MISC_FEATURE (9)..(9): Lys is a-MeLys
  MISC_FEATURE (10)..(10): Lys is Lys(Ac)
  MISC_FEATURE (12)..(12): Xaa is 3-Pal
  MISC_FEATURE (13)..(13): Tyr is NMeTyr
XNTXKXFXKKNXY

SEQ ID NO: 123 - protein, 13 aa, Artificial sequence
  Synthetic construct
  MISC_FEATURE (1)..(1): Xaa is Pen
  MISC_FEATURE (4)..(4): Xaa is W(7-Me)
  MISC_FEATURE (5)..(5): Lys is Lys(Ac)
  MISC_FEATURE (6)..(6): Xaa is Pen
  MISC_FEATURE (7)..(7): Phe is Phe[4-(2-aminoethoxy)]
  MISC_FEATURE (8)..(8): Xaa is 2-Nal
  MISC_FEATURE (9)..(9): Xaa is THP
  MISC_FEATURE (12)..(12): Xaa is 3-Pal
  MISC_FEATURE (13)..(13): Tyr is NMeTyr
XNTXKXFXXENXY

SEQ ID NO: 124 - protein, 13 aa, Artificial sequence
  Synthetic construct
  MISC_FEATURE (1)..(1): Xaa is Pen
  MISC_FEATURE (4)..(4): Xaa is W(7-Me)
  MISC_FEATURE (5)..(5): Lys is Lys(Ac)
  MISC_FEATURE (6)..(6): Xaa is Pen
  MISC_FEATURE (7)..(7): Phe is Phe[4-(2-aminoethoxy)]
  MISC_FEATURE (8)..(8): Xaa is 2-Nal
  MISC_FEATURE (9)..(9): Xaa is THP
  MISC_FEATURE (12)..(12): Xaa is 3-Pal
  MISC_FEATURE (13)..(13): Xaa is Sarc
XNTXKXFXXENXX

SEQ ID NO: 125 - protein, 13 aa, Artificial sequence
  Synthetic construct
  MISC_FEATURE (1)..(1): Xaa is Pen
  MISC_FEATURE (4)..(4): Xaa is W(7-Me)
  MISC_FEATURE (5)..(5): Lys is Lys(Ac)
  MISC_FEATURE (6)..(6): Xaa is Pen
  MISC_FEATURE (7)..(7): Phe is Phe[4-(2-aminoethoxy)]
  MISC_FEATURE (8)..(8): Xaa is 2-Nal
  MISC_FEATURE (9)..(9): Xaa is THP
  MISC_FEATURE (12)..(12): Xaa is 3-Pal
  MISC_FEATURE (13)..(13): Xaa is Sarc
XNTXKXFXXENXX

SEQ ID NO: 126 - protein, 13 aa, Artificial sequence
  Synthetic construct
  MISC_FEATURE (1)..(1): Xaa is Pen
  MISC_FEATURE (4)..(4): Xaa is W(7-Ph)
  MISC_FEATURE (5)..(5): Xaa is Cit
  MISC_FEATURE (6)..(6): Xaa is Pen
  MISC_FEATURE (7)..(7): Phe is Phe[4-(2-aminoethoxy)]
  MISC_FEATURE (8)..(8): Xaa is 2-Nal
  MISC_FEATURE (9)..(9): Xaa is THP
  MISC_FEATURE (12)..(12): Xaa is 3-Pal
  MISC_FEATURE (13)..(13): Xaa is Sarc
XNTXXXFXXENXX

SEQ ID NO: 127 - protein, 13 aa, Artificial sequence
  Synthetic construct
  MISC_FEATURE (1)..(1): Xaa is Pen
  MISC_FEATURE (4)..(4): Xaa is W(7-Ph)
  MISC_FEATURE (6)..(6): Xaa is Pen
  MISC_FEATURE (7)..(7): Phe is Phe[4-(2-aminoethoxy)]
  MISC_FEATURE (8)..(8): Xaa is 2-Nal
  MISC_FEATURE (9)..(9): Xaa is THP
  MISC_FEATURE (12)..(12): Xaa is 3-Pal
  MISC_FEATURE (13)..(13): Xaa is Sarc
XNTXQXFXXENXX

SEQ ID NO: 128-129 - skipped (2 entries)

SEQ ID NO: 130 - protein, 13 aa, Artificial sequence
  Synthetic construct
  MISC_FEATURE (1)..(1): Xaa is Pen
  MISC_FEATURE (4)..(4): Xaa is W(7-Ph)
  MISC_FEATURE (5)..(5): Lys is Lys(Ac)
  MISC_FEATURE (6)..(6): Xaa is Pen
  MISC_FEATURE (7)..(7): Phe is Phe[4-(2-aminoethoxy)]
  MISC_FEATURE (8)..(8): Xaa is 2-Nal
  MISC_FEATURE (9)..(9): Lys is a-MeLys
  MISC_FEATURE (10)..(10): Lys is Lys(Ac)
  MISC_FEATURE (12)..(12): Xaa is 3-Pal
  MISC_FEATURE (13)..(13): Xaa is beta-Alanine
XNTXKXFXKKNXX

SEQ ID NO: 131 - protein, 13 aa, Artificial sequence
  Synthetic construct
  MISC_FEATURE (1)..(1): Xaa is Pen
  MISC_FEATURE (4)..(4): Xaa is W(7-Ph)
  MISC_FEATURE (5)..(5): Lys is Lys(Ac)
  MISC_FEATURE (6)..(6): Xaa is Pen
  MISC_FEATURE (7)..(7): Phe is Phe[4-(2-aminoethoxy)]
  MISC_FEATURE (8)..(8): Xaa is 2-Nal
  MISC_FEATURE (9)..(9): Xaa is THP
  MISC_FEATURE (12)..(12): Xaa is 3-Pal
  MISC_FEATURE (13)..(13): Xaa is beta-Alanine
XNTXKXFXXENXX

SEQ ID NO: 132 - protein, 13 aa, Artificial sequence
  Synthetic construct
  MISC_FEATURE (1)..(1): Xaa is Pen
  MISC_FEATURE (4)..(4): Xaa is W(7-Me)
  MISC_FEATURE (5)..(5): Lys is Lys(Ac)
  MISC_FEATURE (6)..(6): Xaa is Pen
  MISC_FEATURE (7)..(7): Phe is Phe[4-(2-aminoethoxy)]
  MISC_FEATURE (8)..(8): Xaa is 2-Nal
  MISC_FEATURE (9)..(9): Xaa is THP
  MISC_FEATURE (12)..(12): Xaa is 3-Pal
  MISC_FEATURE (13)..(13): Xaa is Sarc
XNTXKXFXXENXX

SEQ ID NO: 133 - protein, 13 aa, Artificial sequence
  Synthetic construct
  MISC_FEATURE (1)..(1): Xaa is Pen
  MISC_FEATURE (4)..(4): Xaa is W(7-Me)
  MISC_FEATURE (5)..(5): Lys is Lys(Ac)
  MISC_FEATURE (6)..(6): Xaa is Pen
  MISC_FEATURE (7)..(7): Phe is Phe[4-(2-aminoethoxy)]
  MISC_FEATURE (8)..(8): Xaa is 2-Nal
  MISC_FEATURE (9)..(9): Xaa is THP
  MISC_FEATURE (10)..(10): Lys is Lys(Ac)
  MISC_FEATURE (12)..(12): Xaa is 3-Pal
  MISC_FEATURE (13)..(13): Xaa is Sarc
XNTXKXFXXKNXX

SEQ ID NO: 134 - protein, 13 aa, Artificial sequence
  Synthetic construct
  MISC_FEATURE (1)..(1): Xaa is Abu
  MISC_FEATURE (4)..(4): Xaa is W(7-Ph)
  MISC_FEATURE (7)..(7): Phe is Phe[4-(2-aminoethoxy)]
  MISC_FEATURE (8)..(8): Xaa is 2-Nal
  MISC_FEATURE (9)..(9): Xaa is THP
  MISC_FEATURE (12)..(12): Xaa is 3-Pal
  MISC_FEATURE (13)..(13): Xaa is Sarc
XQTXQCFXXENXX

SEQ ID NO: 135 - protein, 13 aa, Artificial sequence
  Synthetic construct
  MISC_FEATURE (1)..(1): Xaa is Abu
  MISC_FEATURE (4)..(4): Xaa is W(7-Ph)
  MISC_FEATURE (7)..(7): Phe[4-(2-aminoethoxy)]
  MISC_FEATURE (8)..(8): Xaa is 2-Nal
  MISC_FEATURE (9)..(9): Lys is a-MeLys
  MISC_FEATURE (10)..(10): Lys is Lys(Ac)
  MISC_FEATURE (12)..(2): Xaa is 3-Pal
  misc_feature (12)..(12): Xaa can be any naturally occurring amino acid
  MISC_FEATURE (13)..(13): Xaa is Sarc
XQTXQCFXKKNXX

SEQ ID NO: 136 - protein, 13 aa, Artificial sequence
  Synthetic construct
  MISC_FEATURE (1)..(1): Xaa is Pen
  MISC_FEATURE (4)..(4): Xaa is W(7-Ph)
  MISC_FEATURE (5)..(5): Lys is Lys(Ac)
  MISC_FEATURE (6)..(6): Xaa is Pen
  MISC_FEATURE (7)..(7): Phe is Phe[4-(2-aminoethoxy)]
  MISC_FEATURE (8)..(8): Xaa is 2-Nal
  MISC_FEATURE (9)..(9): Xaa is THP
  MISC_FEATURE (10)..(10): Lys is Lys(Ac)
  MISC_FEATURE (12)..(12): Xaa is 3-Pal
  MISC_FEATURE (13)..(13): Xaa is Sarc
XNTXKXFXXKNXX

SEQ ID NO: 137 - protein, 13 aa, Artificial sequence
  Synthetic construct
  MISC_FEATURE (1)..(1): Xaa is Pen
  MISC_FEATURE (4)..(4): Xaa is W(7-Me)
  MISC_FEATURE (5)..(5): Lys is Lys(Ac)
  MISC_FEATURE (6)..(6): Xaa is Pen
  MISC_FEATURE (7)..(7): Phe is Phe[4-(2-aminoethoxy)]
  MISC_FEATURE (8)..(8): Xaa is 2-Nal
  MISC_FEATURE (9)..(9): Xaa is THP
  MISC_FEATURE (10)..(10): Lys is Lys(Ac)
  MISC_FEATURE (12)..(12): Xaa is 3-Pal
  MISC_FEATURE (13)..(13): Xaa is Sarc
XNTXKXFXXKNXX

SEQ ID NO: 138 - protein, 13 aa, Artificial sequence
  Synthetic construct
  MISC_FEATURE (1)..(1): Xaa is Pen
  MISC_FEATURE (4)..(4): Xaa is W(7-Me)
  MISC_FEATURE (5)..(5): Lys is Lys(Ac)
  MISC_FEATURE (6)..(6): Xaa is Pen
  MISC_FEATURE (7)..(7): Phe is Phe[4-(2-aminoethoxy)]
  MISC_FEATURE (8)..(8): Xaa is 2-Nal
  MISC_FEATURE (9)..(9): Xaa is THP
  MISC_FEATURE (10)..(10): Lys is Lys(Ac)
  MISC_FEATURE (12)..(12): Xaa is 3-Pal
  MISC_FEATURE (13)..(13): Xaa is Sarc
XETXKXFXXKNXX

SEQ ID NO: 139 - protein, 13 aa, Artificial sequence
  Synthetic construct
  MISC_FEATURE (1)..(1): Xaa is Pen
  MISC_FEATURE (4)..(4): Xaa is W(7-Ph)
  MISC_FEATURE (5)..(5): Lys is Lys(Ac)
  MISC_FEATURE (6)..(6): Xaa is Pen
  MISC_FEATURE (7)..(7): Phe is Phe[4-(2-aminoethoxy)]
  MISC_FEATURE (8)..(8): Xaa is 2-Nal
  MISC_FEATURE (9)..(9): Xaa is THP
  MISC_FEATURE (10)..(10): Lys is Lys(Ac)
  MISC_FEATURE (12)..(12): Xaa is 3-Pal
  MISC_FEATURE (13)..(13): Xaa is Sarc
XETXKXFXXKNXX

SEQ ID NO: 140 - protein, 13 aa, Artificial sequence
  Synthetic construct
  MISC_FEATURE (1)..(1): Xaa is Abu
  MISC_FEATURE (4)..(4): Xaa is W(7-Me)
  MISC_FEATURE (7)..(7): Phe is Phe[4-(2-aminoethoxy)]
  MISC_FEATURE (8)..(8): Xaa is 2-Nal
  MISC_FEATURE (9)..(9): Xaa is THP
  MISC_FEATURE (12)..(12): Xaa is 3-Pal
  MISC_FEATURE (13)..(13): Xaa is Sarc
XQTXQCFXXENXX

SEQ ID NO: 141 - protein, 13 aa, Artificial sequence
  Synthetic construct
  MISC_FEATURE (1)..(1): Xaa is Pen
  MISC_FEATURE (4)..(4): Xaa is W(7-Me)
  MISC_FEATURE (5)..(5): Lys is Lys(Ac)
  MISC_FEATURE (6)..(6): Xaa is Pen
  MISC_FEATURE (7)..(7): Phe is Phe[4-(2-aminoethoxy)]
  MISC_FEATURE (8)..(8): Xaa is 2-Nal
  MISC_FEATURE (9)..(9): Xaa is THP
  MISC_FEATURE (10)..(10): Lys is Lys(Ac)
  MISC_FEATURE (12)..(12): Xaa is 3-Pal
  MISC_FEATURE (13)..(13): Xaa is Sarc
XNTXKXFXXKNXX

SEQ ID NO: 142 - protein, 13 aa, Artificial sequence
  Synthetic construct
  MISC_FEATURE (1)..(1): Xaa is Pen
  MISC_FEATURE (4)..(4): Xaa is W(7-(3-carboxamidoPhenyl))
  MISC_FEATURE (5)..(5): Lys is Lys(Ac)
  MISC_FEATURE (6)..(6): Xaa is Pen
  MISC_FEATURE (7)..(7): Phe is Phe[4-(2-aminoethoxy)]
  MISC_FEATURE (8)..(8): Xaa is 2-Nal
  MISC_FEATURE (9)..(9): Xaa is THP
  MISC_FEATURE (12)..(12): Xaa is 3-Nal
  MISC_FEATURE (13)..(13): Xaa is Sarc
XNTXKXFXXENXX

SEQ ID NO: 143 - protein, 13 aa, Artificial sequence
  Synthetic construct
  MISC_FEATURE (1)..(1): Xaa is Pen
  MISC_FEATURE (4)..(4): Xaa is W(7-pyrimidin-5-yl)
  MISC_FEATURE (5)..(5): Lys is Lys(Ac)
  MISC_FEATURE (6)..(6): Xaa is Pen
  MISC_FEATURE (7)..(7): Phe is Phe[4-(2-aminoethoxy)]
  MISC_FEATURE (8)..(8): Xaa is 2-Nal
  MISC_FEATURE (9)..(9): Xaa is THP
  MISC_FEATURE (12)..(12): Xaa is 3-Pal
  MISC_FEATURE (13)..(13): Xaa is Sarc
XNTXKXFXXENXX

SEQ ID NO: 144 - protein, 13 aa, Artificial sequence
  Synthetic construct
  MISC_FEATURE (1)..(1): Xaa is Pen
  MISC_FEATURE (4)..(4): Xaa is W(7-imidazopyridinyl)
  MISC_FEATURE (5)..(5): Lys is Lys(Ac)
  MISC_FEATURE (6)..(6): Xaa is Pen
  MISC_FEATURE (7)..(7): Phe is Phe[4-(2-aminoethoxy)]
  MISC_FEATURE (8)..(8): Xaa is 2-Nal
  MISC_FEATURE (9)..(9): Xaa is THP
  MISC_FEATURE (12)..(12): Xaa is 3-Pal
  MISC_FEATURE (13)..(13): Xaa is Sarc
XNTXKXFXXENXX

SEQ ID NO: 145 - protein, 12 aa, Artificial sequence
  Synthetic construct
  MISC_FEATURE (1)..(1): Xaa is Pen
  MISC_FEATURE (4)..(4): Xaa is W(7-Me)
  MISC_FEATURE (5)..(5): Lys is Lys(Ac)
  MISC_FEATURE (6)..(6): Xaa is Pen
  MISC_FEATURE (7)..(7): Phe is Phe[4-(2-aminoethoxy)]
  MISC_FEATURE (8)..(8): Xaa is 2-Nal
  MISC_FEATURE (9)..(9): Lys is NMe(Lys)
  MISC_FEATURE (10)..(10): Lys is Lys(Ac)
  MISC_FEATURE (12)..(12): His is 3MeHis
XNTXKXFXKKNH

SEQ ID NO: 146 - protein, 13 aa, Artificial sequence
  Synthetic construct
  MISC_FEATURE (1)..(1): Arg is (D)Arg
  MISC_FEATURE (2)..(2): Xaa is Pen
  MISC_FEATURE (5)..(5): Xaa is W(7-Me)
  MISC_FEATURE (6)..(6): Lys is Lys(Ac)
  MISC_FEATURE (7)..(7): Xaa is Pen
  MISC_FEATURE (8)..(8): Phe is Phe[4-(2-aminoethoxy)]
  MISC_FEATURE (9)..(9): Xaa is 2-Nal
  MISC_FEATURE (10)..(10): Xaa is THP
  MISC_FEATURE (13)..(13): His is 3MeHis
RXNTXKXFXXENH

SEQ ID NO: 147 - protein, 13 aa, Artificial sequence
  Synthetic construct
  MISC_FEATURE (1)..(1): Xaa is Pen
  MISC_FEATURE (4)..(4): Xaa is W(7-(4Quin))
  MISC_FEATURE (5)..(5): Lys is Lys(Ac)
  MISC_FEATURE (6)..(6): Xaa is Pen
  MISC_FEATURE (7)..(7): Phe is Phe[4-(2-aminoethoxy)]
  MISC_FEATURE (8)..(8): Xaa is 2-Nal
  MISC_FEATURE (9)..(9): Xaa is THP
  MISC_FEATURE (12)..(12): Xaa is 3-Pal
  MISC_FEATURE (13)..(13): Xaa is Sarc
XNTXKXFXXENXX

SEQ ID NO: 148 - protein, 13 aa, Artificial sequence
  Synthetic construct
  MISC_FEATURE (1)..(1): Xaa is Pen
  MISC_FEATURE (4)..(4): Xaa is W(7-(3-pyrazol-1-yl))
  MISC_FEATURE (5)..(5): Lys is Lys(Ac)
  MISC_FEATURE (6)..(6): Xaa is Pen
  MISC_FEATURE (7)..(7): Phe is Phe[4-(2-aminoethoxy)]
  MISC_FEATURE (8)..(8): Xaa is 2-Nal
  MISC_FEATURE (9)..(9): Xaa is THP
  MISC_FEATURE (12)..(12): Xaa is 3-Pal
  MISC_FEATURE (13)..(13): Xaa is Sarc
XNTXKXFXXENXX

SEQ ID NO: 149 - protein, 13 aa, Artificial sequence
  Synthetic construct
  MISC_FEATURE (1)..(1): Xaa is Pen
  MISC_FEATURE (4)..(4): Xaa is W(7-(5-Et))
  MISC_FEATURE (5)..(5): Lys is Lys(Ac)
  MISC_FEATURE (6)..(6): Xaa is Pen
  MISC_FEATURE (7)..(7): Phe is Phe[4-(2-aminoethoxy)]
  MISC_FEATURE (8)..(8): Xaa is 2-Nal
  MISC_FEATURE (9)..(9): Xaa is THP
  MISC_FEATURE (12)..(12): Xaa is 3-Pal
  MISC_FEATURE (13)..(13): Xaa is Sarc
XNTXKXFXXENXX

SEQ ID NO: 150 - protein, 13 aa, Artificial sequence
  Synthetic construct
  MISC_FEATURE (1)..(1): Xaa is Pen
  MISC_FEATURE (4)..(4): Xaa is W(5-Ph)
  MISC_FEATURE (5)..(5): Lys is Lys(Ac)
  MISC_FEATURE (6)..(6): Xaa is Pen
  MISC_FEATURE (7)..(7): Phe is Phe[4-(2-aminoethoxy)]
  MISC_FEATURE (8)..(8): Xaa is 2-Nal
  MISC_FEATURE (9)..(9): Xaa is THP
  MISC_FEATURE (12)..(12): Xaa is 3-Pal
  MISC_FEATURE (13)..(13): Xaa is Sarc
XNTXKXFXXENXX

SEQ ID NO: 151 - protein, 13 aa, Artificial sequence
  Synthetic construct
  MISC_FEATURE (1)..(1): Xaa is Pen
  MISC_FEATURE (4)..(4): Xaa is W(7-(3-pyrazol-1-yl))
  MISC_FEATURE (5)..(5): Lys is Lys(Ac)
  MISC_FEATURE (6)..(6): Xaa is Pen
  MISC_FEATURE (7)..(7): Phe is Phe[4-(2-aminoethoxy)]
  MISC_FEATURE (8)..(8): Xaa is 2-Nal
  MISC_FEATURE (9)..(9): Xaa is THP
  MISC_FEATURE (12)..(12): Xaa is 3-Pal
  MISC_FEATURE (13)..(13): Xaa is Sarc
XNTXKXFXXENXX

SEQ ID NO: 152 - protein, 13 aa, Artificial sequence
  Synthetic construct
  MISC_FEATURE (1)..(1): Xaa is Pen
  MISC_FEATURE (4)..(4): Xaa is W(7-indazol-5-yl)
  MISC_FEATURE (5)..(5): Lys is Lys(Ac)
  MISC_FEATURE (6)..(6): Xaa is Pen
  MISC_FEATURE (7)..(7): Phe is Phe[4-(2-aminoethoxy)]
  MISC_FEATURE (8)..(8): Xaa is 2-Nal
  MISC_FEATURE (9)..(9): Xaa is THP
  MISC_FEATURE (12)..(12): Xaa is 3-Pal
  MISC_FEATURE (13)..(13): Xaa is Sarc
XNTXKXFXXENXX

SEQ ID NO: 153 - protein, 13 aa, Artificial sequence
  Synthetic construct
  MISC_FEATURE (1)..(1): Xaa is Pen
  MISC_FEATURE (4)..(4): Xaa is W(4-F)
  MISC_FEATURE (5)..(5): Lys is Lys(Ac)
  MISC_FEATURE (6)..(6): Xaa is Pen
  MISC_FEATURE (7)..(7): Phe is Phe[4-(2-aminoethoxy)]
  MISC_FEATURE (8)..(8): Xaa is 2-Nal
  MISC_FEATURE (9)..(9): Xaa is THP
  MISC_FEATURE (12)..(12): Xaa is 3-Pal
  MISC_FEATURE (13)..(13): Xaa is Sarc
XNTXKXFXXENXX

SEQ ID NO: 154 - protein, 13 aa, Artificial sequence
  Synthetic construct
  MISC_FEATURE (1)..(1): Xaa is Pen
  MISC_FEATURE (4)..(4): Xaa is W(5-CN)
  MISC_FEATURE (5)..(5): Lys is Lys(Ac)
  MISC_FEATURE (6)..(6): Xaa is Pen
  MISC_FEATURE (7)..(7): Phe is Phe[4-(2-aminoethoxy)]
  MISC_FEATURE (8)..(8): Xaa is 2-Nal
  MISC_FEATURE (9)..(9): Xaa is THP
  MISC_FEATURE (12)..(12): Xaa is 3-Pal
  MISC_FEATURE (13)..(13): Xaa is Sarc
XNTXKXFXXENXX

SEQ ID NO: 155 - protein, 13 aa, Artificial sequence
  Synthetic construct
  MISC_FEATURE (1)..(1): Xaa is Pen
  MISC_FEATURE (4)..(4): Xaa is W(7-CN)
  MISC_FEATURE (5)..(5): Lys is Lys(Ac)
  MISC_FEATURE (6)..(6): Xaa is Pen
  MISC_FEATURE (7)..(7): Phe is Phe[4-(2-aminoethoxy)]
  MISC_FEATURE (8)..(8): Xaa is 2-Nal
  MISC_FEATURE (9)..(9): Xaa is THP
  MISC_FEATURE (12)..(12): Xaa is 3-Pal
  MISC_FEATURE (13)..(13): Xaa is Sarc
XNTXKXFXXENXX

SEQ ID NO: 156 - protein, 13 aa, Artificial sequence
  Synthetic construct
  MISC_FEATURE (1)..(1): Xaa is Pen
  MISC_FEATURE (4)..(4): Xaa is W(4-OMe)
  MISC_FEATURE (5)..(5): Lys is Lys(Ac)
  MISC_FEATURE (6)..(6): Xaa is Pen
  MISC_FEATURE (7)..(7): Phe is Phe[4-(2-aminoethoxy)]
  MISC_FEATURE (8)..(8): Xaa is 2-Nal
  MISC_FEATURE (9)..(9): Xaa is THP
  MISC_FEATURE (12)..(12): Xaa is 3-Pal
  MISC_FEATURE (13)..(13): Xaa is Sarc
XNTXKXFXXENXX

SEQ ID NO: 157 - protein, 13 aa, Artificial sequence
  Synthetic construct
  MISC_FEATURE (1)..(1): Xaa is Pen
  MISC_FEATURE (4)..(4): Xaa is W(4-Me)
  MISC_FEATURE (5)..(5): Lys is Lys(Ac)
  MISC_FEATURE (6)..(6): Xaa is Pen
  MISC_FEATURE (7)..(7): Phe is Phe[4-(2-aminoethoxy)]
  MISC_FEATURE (8)..(8): Xaa is 2-Nal
  MISC_FEATURE (9)..(9): Xaa is THP
  MISC_FEATURE (12)..(12): Xaa is 3-Pal
  MISC_FEATURE (13)..(13): Xaa is Sarc
XNTXKXFXXENXX

SEQ ID NO: 158 - protein, 13 aa, Artificial sequence
  Synthetic construct
  MISC_FEATURE (1)..(1): Xaa is Pen
  MISC_FEATURE (5)..(5): Lys is Lys(Ac)
  MISC_FEATURE (6)..(6): Xaa is Pen
  MISC_FEATURE (7)..(7): Phe is Phe[4-(2-aminoethoxy)]
  MISC_FEATURE (8)..(8): Xaa is 2-Nal
  MISC_FEATURE (9)..(9): Xaa is THP
  MISC_FEATURE (12)..(12): Xaa is 3-Pal
  MISC_FEATURE (13)..(13): Xaa is Sarc
XNTWKXFXXENXX

SEQ ID NO: 159 - protein, 13 aa, Artificial sequence
  Synthetic construct
  MISC_FEATURE (1)..(1): Xaa is Pen
  MISC_FEATURE (5)..(5): Lys is Lys(Ac)
  MISC_FEATURE (6)..(6): Xaa is Pen
  MISC_FEATURE (7)..(7): Phe is Phe[4-(2-aminoethoxy)]
  MISC_FEATURE (8)..(8): Xaa is 2-Nal
  MISC_FEATURE (9)..(9): Xaa is 1-aminocyclopentanecarboxylic acid
  MISC_FEATURE (12)..(12): Xaa is 3-Pal
  MISC_FEATURE (13)..(13): Xaa is Sarc
XNTWKXFXXENXX

SEQ ID NO: 160 - protein, 13 aa, Artificial sequence
  Synthetic construct
  MISC_FEATURE (1)..(1): Xaa is Pen
  MISC_FEATURE (4)..(4): Xaa is W(5-Ca)
  MISC_FEATURE (5)..(5): Lys is Lys(Ac)
  MISC_FEATURE (6)..(6): Xaa is Pen
  MISC_FEATURE (7)..(7): Phe is Phe[4-(2-aminoethoxy)]
  MISC_FEATURE (8)..(8): Xaa is 2-Nal
  MISC_FEATURE (9)..(9): Xaa is THP
  MISC_FEATURE (12)..(12): Xaa is 3-Pal
  MISC_FEATURE (13)..(13): Xaa is Sarc
XNTXKXFXXENXX

SEQ ID NO: 161 - protein, 13 aa, Artificial sequence
  Synthetic construct
  MISC_FEATURE (1)..(1): Xaa is Pen
  MISC_FEATURE (4)..(4): Xaa is Trp_4Aza
  MISC_FEATURE (5)..(5): Lys is Lys(Ac)
  MISC_FEATURE (6)..(6): Xaa is Pen
  MISC_FEATURE (7)..(7): Phe is Phe[4-(2-aminoethoxy)]
  MISC_FEATURE (8)..(8): Xaa is 2-Nal
  MISC_FEATURE (9)..(9): Xaa is THP
  MISC_FEATURE (12)..(12): Xaa is 3-Pal
  MISC_FEATURE (13)..(13): Xaa is Sarc
XNTWKXFXXENXX

SEQ ID NO: 162 - protein, 13 aa, Artificial sequence
  Synthetic construct
  MISC_FEATURE (1)..(1): Xaa is Pen
  MISC_FEATURE (5)..(5): Lys is Lys(Ac)
  MISC_FEATURE (6)..(6): Xaa is Pen
  MISC_FEATURE (7)..(7): Phe is Phe[4-(2-aminoethoxy)]
  MISC_FEATURE (8)..(8): Xaa is 2-Nal
  MISC_FEATURE (9)..(9): Xaa is THP
  MISC_FEATURE (12)..(12): Xaa is 3-Pal
  MISC_FEATURE (13)..(13): Xaa is Sarc
XNTWKXFXXENXX

SEQ ID NO: 163 - protein, 13 aa, Artificial sequence
  Synthetic construct
  MISC_FEATURE (1)..(1): Xaa is Pen
  MISC_FEATURE (5)..(5): Lys is Lys(Ac)
  MISC_FEATURE (6)..(6): Xaa is Pen
  MISC_FEATURE (7)..(7): Phe is Phe[4-(2-aminoethoxy)]
  MISC_FEATURE (8)..(8): Xaa is 2-Nal
  MISC_FEATURE (9)..(9): Xaa is THP
  MISC_FEATURE (10)..(10): Lys is Lys(Ac)
  MISC_FEATURE (12)..(12): Xaa is 3-Pal
  MISC_FEATURE (13)..(13): Xaa is Sarc
XNTWKXFXXKNXX

SEQ ID NO: 164 - protein, 13 aa, Artificial sequence
  Synthetic construct
  MISC_FEATURE (1)..(1): Arg is (D)Arg
  MISC_FEATURE (2)..(2): Xaa is Pen
  MISC_FEATURE (5)..(5): Xaa is W(7-Me)
  MISC_FEATURE (6)..(6): Lys is Lys(Ac)
  MISC_FEATURE (7)..(7): Xaa is Pen
  MISC_FEATURE (8)..(8): Phe is Phe[4-(2-aminoethoxy)]
  MISC_FEATURE (9)..(9): Xaa is 2-Nal
  MISC_FEATURE (10)..(10): Xaa is THP
  MISC_FEATURE (13)..(13): Xaa is 5Pyal
RXNTXKXFXXENX

SEQ ID NO: 165 - protein, 12 aa, Artificial sequence
  Synthetic construct
  MISC_FEATURE (1)..(1): Xaa is Pen
  MISC_FEATURE (4)..(4): Xaa is W(7-Me)
  MISC_FEATURE (5)..(5): Lys is Lys(Ac)
  MISC_FEATURE (6)..(6): Xaa is Pen
  MISC_FEATURE (7)..(7): Phe is Phe[4-(2-aminoethoxy)]
  MISC_FEATURE (8)..(8): Xaa is 2-Nal
  MISC_FEATURE (9)..(9): Lys is a-Me-Lys
  MISC_FEATURE (10)..(10): Lys is Lys(Ac)
  MISC_FEATURE (12)..(12): Xaa is 5Pyal
XNTXKXFXKKNX

SEQ ID NO: 166 - protein, 13 aa, Artificial sequence
  Synthetic construct
  MISC_FEATURE (1)..(1): Arg is (D)Arg
  MISC_FEATURE (2)..(2): Xaa is Pen
  MISC_FEATURE (5)..(5): Xaa is W(7-Me)
  MISC_FEATURE (6)..(6): Lys is Lys(Ac)
  MISC_FEATURE (7)..(7): Xaa is Pen
  MISC_FEATURE (8)..(8): Phe is Phe[4-(2-aminoethoxy)]
  MISC_FEATURE (9)..(9): Xaa is 2-Nal
  MISC_FEATURE (10)..(10): Xaa is THP
  MISC_FEATURE (13)..(13): His is (1-Me)His
RXNTXKXFXXENH

SEQ ID NO: 167 - protein, 12 aa, Artificial sequence
  Synthetic construct
  MISC_FEATURE (1)..(1): Xaa is Pen
  MISC_FEATURE (4)..(4): Xaa is W(7-Me)]
  MISC_FEATURE (5)..(5): Lys is Lys(Ac)
  MISC_FEATURE (6)..(6): Xaa is Pen
  MISC_FEATURE (7)..(7): Phe is Phe[4-(2-aminoethoxy)]
  MISC_FEATURE (8)..(8): Xaa is 2-Nal
  MISC_FEATURE (9)..(9): Lys is aMeLys
  MISC_FEATURE (10)..(10): Lys is Lys(Ac)
  MISC_FEATURE (12)..(12): His is (1-Me)His
XNTXKXFXKKNH

SEQ ID NO: 168 - protein, 13 aa, Artificial sequence
  Synthetic construct
  MISC_FEATURE (1)..(1): Xaa is Pen
  MISC_FEATURE (4)..(4): Xaa is W(7-Me)
  MISC_FEATURE (5)..(5): Lys is Lys(Ac)
  MISC_FEATURE (6)..(6): Xaa is Pen
  MISC_FEATURE (7)..(7): Phe is Phe[4-(2-aminoethoxy)]
  MISC_FEATURE (8)..(8): Xaa is 2-Nal
  MISC_FEATURE (9)..(9): Lys is a-Me-Lys
  MISC_FEATURE (10)..(10): Lys is Lys(Ac)
  MISC_FEATURE (12)..(12): Xaa is 3-Pal
  MISC_FEATURE (13)..(13): Tyr is (D)NMeTyr
XNTXKXFXKKNXY

SEQ ID NO: 169 - protein, 13 aa, Artificial sequence
  Synthetic construct
  MISC_FEATURE (1)..(1): Xaa is Pen
  MISC_FEATURE (4)..(4): Xaa is W(7-Me)
  MISC_FEATURE (5)..(5): Lys is Lys(Ac)
  MISC_FEATURE (6)..(6): Xaa is Pen
  MISC_FEATURE (7)..(7): Phe is Phe[4-(2-aminoethoxy)]
  MISC_FEATURE (8)..(8): Xaa is 2-Nal
  MISC_FEATURE (9)..(9): Lys is a-MeLys
  MISC_FEATURE (10)..(10): Lys is Lys(Ac)
  MISC_FEATURE (12)..(12): Xaa is Aib
  MISC_FEATURE (13)..(13): Xaa is (D)Thr
XNTXKXFXKKNXT

SEQ ID NO: 170 - protein, 13 aa, Artificial sequence
  Synthetic construct
  MISC_FEATURE (1)..(1): Xaa is Pen
  MISC_FEATURE (4)..(4): Xaa is W(7-Me)
  MISC_FEATURE (5)..(5): Lys is Lys(Ac)
  MISC_FEATURE (6)..(6): Xaa is Pen
  MISC_FEATURE (7)..(7): Phe is Phe[4-(2-aminoethoxy)]
  MISC_FEATURE (8)..(8): Xaa is 2-Nal
  MISC_FEATURE (9)..(9): Xaa is THP
  MISC_FEATURE (13)..(13): Pro is (D)Pro
XNTXKXFXXENHP

SEQ ID NO: 171-200 - skipped (30 entries)

SEQ ID NO: 201 - protein, 14 aa, Artificial sequence
  Synthetic construct
  MISC_FEATURE (1)..(1): Arg is (D)Arg
  MISC_FEATURE (2)..(2): Xaa is Pen
  MISC_FEATURE (5)..(5): Xaa is W(7-Me)
  MISC_FEATURE (6)..(6): Xaa is Cit
  MISC_FEATURE (7)..(7): Xaa is Pen
  MISC_FEATURE (8)..(8): Phe is Phe[4-(2-aminoethoxy)]
  MISC_FEATURE (9)..(9): Xaa is 2-Nal
  MISC_FEATURE (10)..(10): Leu is aMeLeu
  MISC_FEATURE (13)..(13): Lys is (D)Lys
  MISC_FEATURE (14)..(14): Tyr is (D)NMeTyr
RXNTXXXFXLENKY

SEQ ID NO: 202 - protein, 14 aa, Artificial sequence
  Synthetic construct
  MISC_FEATURE (1)..(1): Arg is (D)Arg
  MISC_FEATURE (2)..(2): Xaa is Pen
  MISC_FEATURE (5)..(5): Xaa is W(7 Me)
  MISC_FEATURE (6)..(6): Xaa is Cit
  MISC_FEATURE (7)..(7): Xaa is Pen
  MISC_FEATURE (8)..(8): Phe is Phe[4 (2 aminoethoxy)]
  MISC_FEATURE (9)..(9): Xaa is 2-Nal
  MISC_FEATURE (10)..(10): Leu is aMeLeu
  MISC_FEATURE (13)..(13): His is (D)His
  MISC_FEATURE (14)..(14): Tyr is (D)NMeTyr
RXNTXXXFXLENHY

SEQ ID NO: 203 - protein, 13 aa, Artificial sequence
  Synthetic construct
  MISC_FEATURE (1)..(1): Xaa is Pen
  MISC_FEATURE (4)..(4): Xaa is W(7 Me)
  MISC_FEATURE (5)..(5): Lys is Lys(Ac)
  MISC_FEATURE (6)..(6): Xaa is Pen
  MISC_FEATURE (7)..(7): Phe is Phe[4 (2 aminoethoxy)]
  MISC_FEATURE (8)..(8): Xaa is 2-Nal
  MISC_FEATURE (9)..(9): Lys is a MeLys
  MISC_FEATURE (10)..(10): Lys is a Lys(Ac)
  MISC_FEATURE (12)..(12): Xaa is (D)Orn
  MISC_FEATURE (13)..(13): Tyr is (D)NMeTyr
XNTXKXFXKKNXY

SEQ ID NO: 204 - protein, 13 aa, Artificial sequence
  Synthetic construct
  MISC_FEATURE (1)..(1): Xaa is Pen
  MISC_FEATURE (4)..(4): Xaa is W(7 Me)
  MISC_FEATURE (5)..(5): Lys is Lys(Ac)
  MISC_FEATURE (6)..(6): Xaa is Pen
  MISC_FEATURE (7)..(7): Phe is Phe[4 (2 aminoethoxy)]
  MISC_FEATURE (8)..(8): Xaa is 2-Nal
  MISC_FEATURE (9)..(9): Lys is a MeLys
  MISC_FEATURE (10)..(10): Lys is Lys(Ac)
  MISC_FEATURE (12)..(12): Ser is (D)Ser
  MISC_FEATURE (13)..(13): Tyr is (D)NMeTyr
XNTXKXFXKKNSY

SEQ ID NO: 205 - protein, 13 aa, Artificial sequence
  Synthetic construct
  MISC_FEATURE (1)..(1): Xaa is Pen
  MISC_FEATURE (4)..(4): Xaa is W(7 Me)
  MISC_FEATURE (5)..(5): Lys is Lys(Ac)
  MISC_FEATURE (6)..(6): Xaa is Pen
  MISC_FEATURE (7)..(7): Phe is Phe[4 (2 aminoethoxy)]
  MISC_FEATURE (8)..(8): Xaa is 2-Nal
  MISC_FEATURE (9)..(9): Lys is a MeLys
  MISC_FEATURE (10)..(10): Lys is Lys(Ac)
  MISC_FEATURE (12)..(12): Phe is (D)Phe
  MISC_FEATURE (13)..(13): Tyr is (D)NMeTyr
XNTXKXFXKKNFY

SEQ ID NO: 206 - protein, 14 aa, Artificial sequence
  Synthetic construct
  MISC_FEATURE (1)..(1): Arg is (D)Arg
  MISC_FEATURE (2)..(2): Xaa is Pen
  MISC_FEATURE (5)..(5): Xaa is W(7 Me)
  MISC_FEATURE (6)..(6): Lys is Lys(Ac)
  MISC_FEATURE (7)..(7): Xaa is Pen
  MISC_FEATURE (8)..(8): Phe is Phe[4 (2 aminoethoxy)]
  MISC_FEATURE (9)..(9): Xaa is 2-Nal
  MISC_FEATURE (10)..(10): Xaa is THP
  MISC_FEATURE (14)..(14): Tyr is (D)Tyr
RXNTXKXFXXENHY

SEQ ID NO: 207 - protein, 13 aa, Artificial sequence
  Synthetic construct
  MISC_FEATURE (1)..(1): Xaa is Pen
  MISC_FEATURE (4)..(4): Xaa is W(7 Me)
  MISC_FEATURE (5)..(5): Tyr is (D)Tyr
  MISC_FEATURE (6)..(6): Xaa is Pen
  MISC_FEATURE (7)..(7): Phe is Phe[4 (2 aminoethoxy)]
  MISC_FEATURE (8)..(8): Xaa is 2-Nal
  MISC_FEATURE (9)..(9): Lys is a-MeLys
  MISC_FEATURE (10)..(10): Lys is Lys(Ac)
  MISC_FEATURE (12)..(12): Lys is (D)Lys
  MISC_FEATURE (13)..(13): Tyr is (D)NMeTyr
XNTXYXFXKKNKY

SEQ ID NO: 208 - protein, 14 aa, Artificial sequence
  Synthetic construct
  MISC_FEATURE (1)..(1): Arg is (D)Arg
  MISC_FEATURE (2)..(2): Xaa is Pen
  MISC_FEATURE (5)..(5): Xaa is W(7-Me)
  MISC_FEATURE (6)..(6): Lys is Lys(Ac)
  MISC_FEATURE (7)..(7): Phe is Phe[4-(2-aminoethoxy)]
  MISC_FEATURE (8)..(8): Xaa is 2-Nal
  MISC_FEATURE (9)..(9): Xaa is THP
  misc_feature (10)..(10): Xaa can be any naturally occurring amino acid
RXNTXKXFXXENHP

SEQ ID NO: 209 - protein, 14 aa, Artificial sequence
  Synthetic construct
  MISC_FEATURE (1)..(1): Arg is (D)Arg
  MISC_FEATURE (2)..(2): Xaa is Pen
  MISC_FEATURE (5)..(5): Xaa is W(7-Me)
  MISC_FEATURE (6)..(6): Lys is Lys(Ac)
  MISC_FEATURE (7)..(7): Xaa is Pen
  MISC_FEATURE (8)..(8): Phe is Phe[4-(2-aminoethoxy)]
  MISC_FEATURE (9)..(9): Xaa is 2-Nal
  MISC_FEATURE (10)..(10): Xaa is THP
  MISC_FEATURE (14)..(14): Pro is (D)Pro
RXNTXKXFXXENHP

SEQ ID NO: 210 - protein, 13 aa, Artificial sequence
  Synthetic construct
  MISC_FEATURE (1)..(1): Xaa is Pen
  MISC_FEATURE (4)..(4): Xaa is W(7-Me)
  MISC_FEATURE (5)..(5): Phe is Phe(4)
  MISC_FEATURE (6)..(6): Xaa is Pen
  MISC_FEATURE (7)..(7): Phe is Phe[4-(2-aminoethoxy)]
  MISC_FEATURE (8)..(8): Xaa is 2-Nal
  MISC_FEATURE (9)..(9): Lys is a-MeLys
  MISC_FEATURE (10)..(10): Lys is Lys(Ac)
  MISC_FEATURE (12)..(12): Lys is (D)Lys
  MISC_FEATURE (13)..(13): Tyr is (D)NMeTyr
XNTXFXFXKKNKY

SEQ ID NO: 211 - protein, 13 aa, Artificial sequence
  Synthetic construct
  MISC_FEATURE (1)..(1): Xaa is Pen
  MISC_FEATURE (4)..(4): Xaa is W(7-Me)
  MISC_FEATURE (5)..(5): Lys is Lys(Ac)
  MISC_FEATURE (6)..(6): Xaa is Pen
  MISC_FEATURE (7)..(7): Phe is Phe[4-(2-aminoethoxy)]
  MISC_FEATURE (8)..(8): Xaa is 2-Nal
  MISC_FEATURE (9)..(9): Xaa is 1-aminocyclopentanecarboxylic acid
  MISC_FEATURE (13)..(13): Xaa is Sarc
XNTXKXFXXENFX

SEQ ID NO: 212 - protein, 13 aa, Artificial sequence
  Synthetic construct
  MISC_FEATURE (1)..(1): Arg is (D)Arg
  MISC_FEATURE (2)..(2): Xaa is Pen
  MISC_FEATURE (5)..(5): Xaa is W(7-Me)
  MISC_FEATURE (6)..(6): Lys is Lys(Ac)
  MISC_FEATURE (7)..(7): Xaa is Pen
  MISC_FEATURE (8)..(8): Phe is Phe[4-(2-aminoethoxy)]
  MISC_FEATURE (9)..(9): Xaa is 2-Nal
  MISC_FEATURE (10)..(10): Xaa is THP
RXNTXKXFXXENH

SEQ ID NO: 213 - protein, 13 aa, Artificial sequence
  Synthetic construct
  MISC_FEATURE (1)..(1): Xaa is Pen
  MISC_FEATURE (4)..(4): Xaa is W(7-Me)
  MISC_FEATURE (5)..(5): Lys is Lys(Ac)
  MISC_FEATURE (6)..(6): Xaa is Pen
  MISC_FEATURE (7)..(7): Phe is Phe[4-(2-aminoethoxy)]
  MISC_FEATURE (8)..(8): Xaa is 2-Nal
  MISC_FEATURE (9)..(9): Lys is a-MeLys
  MISC_FEATURE (10)..(10): Lys is Lys(Ac)
  MISC_FEATURE (13)..(13): Xaa is N(H)Me
XNTXKXFXKKNHX

SEQ ID NO: 214 - protein, 13 aa, Artificial sequence
  Synthetic construct
  MISC_FEATURE (1)..(1): Xaa is Pen
  MISC_FEATURE (4)..(4): Xaa is W(7-Me)
  MISC_FEATURE (5)..(5): Phe is Phe(4-NH(Ac))
  MISC_FEATURE (6)..(6): Xaa is Pen
  MISC_FEATURE (7)..(7): Phe is Phe[4-(2-aminoethoxy)]
  MISC_FEATURE (8)..(8): Xaa is 2-Nal
  MISC_FEATURE (9)..(9): Lys is a-MeLys
  MISC_FEATURE (10)..(10): Lys is Lys(Ac)
  MISC_FEATURE (12)..(12): Lys is (D)Lys
  MISC_FEATURE (13)..(13): Tyr is (D)NMeTyr
XNTXFXFXKKNKY

SEQ ID NO: 215 - protein, 13 aa, Artificial sequence
  Synthetic construct
  MISC_FEATURE (1)..(1): Xaa is Pen
  MISC_FEATURE (4)..(4): Xaa is W(7-Me)
  MISC_FEATURE (5)..(5): Lys is Lys(Ac)
  MISC_FEATURE (6)..(6): Xaa is Pen
  MISC_FEATURE (7)..(7): Phe is Phe[4-(2-aminoethoxy)]
  MISC_FEATURE (8)..(8): Xaa is 2-Nal
  MISC_FEATURE (9)..(9): Lys is a-MeLys
  MISC_FEATURE (10)..(10): Lys is aLys(Ac)
  MISC_FEATURE (13)..(13): Tyr is (D)NMeTyr
XNTXKXFXKKNYY

SEQ ID NO: 216 - protein, 13 aa, Artificial sequence
  Synthetic construct
  MISC_FEATURE (1)..(1): Xaa is Pen
  MISC_FEATURE (4)..(4): Xaa is W(7-Me)
  MISC_FEATURE (5)..(5): Xaa is Cit
  MISC_FEATURE (6)..(6): Xaa is Pen
  MISC_FEATURE (7)..(7): Phe is Phe[4-(2-aminoethoxy)]
  MISC_FEATURE (8)..(8): Xaa is 2-Nal
  MISC_FEATURE (9)..(9): Leu is a-MeLeu
  MISC_FEATURE (10)..(10): Lys is Lys(Ac)
  MISC_FEATURE (12)..(12): Lys is (D)Lys
  MISC_FEATURE (13)..(13): Tyr is (D)NMeTyr]
XNTXXXFXLKNKY

SEQ ID NO: 217 - protein, 13 aa, Artificial sequence
  Synthetic construct
  MISC_FEATURE (1)..(1): Xaa is Pen
  MISC_FEATURE (4)..(4): Xaa is W(7-Me)
  MISC_FEATURE (5)..(5): Lys is Lys(Ac)
  MISC_FEATURE (6)..(6): Xaa is Pen
  MISC_FEATURE (7)..(7): Phe is Phe[4-(2-aminoethoxy)]
  MISC_FEATURE (8)..(8): Xaa is 2-Nal
  MISC_FEATURE (9)..(9): Lys is [a-MeLys]
  MISC_FEATURE (10)..(10): Lys is Lys(Ac)
  MISC_FEATURE (11)..(11): Lys is (D)Lys
  MISC_FEATURE (12)..(12): His is (D)His
  MISC_FEATURE (13)..(13): Tyr is (D)NMeTyr
XNTXKXFXKKNHY

SEQ ID NO: 218 - protein, 13 aa, Artificial sequence
  Synthetic construct
  MISC_FEATURE (1)..(1): Xaa is Pen
  MISC_FEATURE (4)..(4): Xaa is W(7-Me)
  MISC_FEATURE (5)..(5): Lys is Lys(Ac)
  MISC_FEATURE (6)..(6): Xaa is Pen
  MISC_FEATURE (7)..(7): Phe is Phe[4-(2-aminoethoxy)]
  MISC_FEATURE (8)..(8): Xaa is 2-Nal
  MISC_FEATURE (9)..(9): Lys is a-MeLys
  MISC_FEATURE (10)..(10): Lys is Lys(Ac)
  MISC_FEATURE (12)..(12): Ala is beta Alanine
  MISC_FEATURE (13)..(13): Tyr is (D)NMeTyr
XNTXKXFXKKNAY

SEQ ID NO: 219 - protein, 13 aa, Artificial sequence
  Synthetic construct
  MISC_FEATURE (1)..(1): Xaa is Pen
  MISC_FEATURE (4)..(4): Xaa is W(7-Me)
  MISC_FEATURE (5)..(5): Lys is Lys(Ac)
  MISC_FEATURE (6)..(6): Xaa is Pen
  MISC_FEATURE (7)..(7): Phe is Phe[4-(2-aminoethoxy)]
  MISC_FEATURE (8)..(8): Xaa is 2-Nal
  MISC_FEATURE (9)..(9): Lys is a-MeLys
  MISC_FEATURE (10)..(10): Lys is Lys(Ac)
  MISC_FEATURE (12)..(12): Ala is beta Alanine
  MISC_FEATURE (13)..(13): Tyr is (D)NMeTyr
XNTXKXFXKKNAY

SEQ ID NO: 220 - protein, 13 aa, Artificial sequence
  Synthetic construct
  MISC_FEATURE (1)..(1): Xaa is Pen
  MISC_FEATURE (4)..(4): Xaa is W(7-Me)
  MISC_FEATURE (5)..(5): Lys is Lys(Ac)
  MISC_FEATURE (6)..(6): Xaa is Pen
  MISC_FEATURE (7)..(7): Phe is Phe[4-(2-aminoethoxy)]
  MISC_FEATURE (8)..(8): Xaa is 2-Nal
  MISC_FEATURE (9)..(9): Lys is a-MeLys
  MISC_FEATURE (10)..(10): Lys is Lys(Ac)
  MISC_FEATURE (12)..(12): Ala is beta Alanine
  MISC_FEATURE (13)..(13): Tyr is (D)NMeTyr
XNTXKXFXKKNAY

SEQ ID NO: 221 - protein, 14 aa, Artificial sequence
  Synthetic construct
  MISC_FEATURE (1)..(1): Arg is (D)Arg
  MISC_FEATURE (2)..(2): Xaa is Pen
  MISC_FEATURE (5)..(5): Xaa is W(7-Me)
  MISC_FEATURE (6)..(6): Lys is Lys(Ac)
  MISC_FEATURE (7)..(7): Xaa is Pen
  MISC_FEATURE (8)..(8): Phe is Phe[4-(2-aminoethoxy)]
  MISC_FEATURE (9)..(9): Xaa is 2-Nal
  MISC_FEATURE (10)..(10): Lys is a-MeLys
  MISC_FEATURE (14)..(14): Xaa is N(H)Me
RXNTXKXFXKENHX

SEQ ID NO: 222 - protein, 14 aa, Artificial sequence
  Synthetic construct
  MISC_FEATURE (1)..(1): Arg is (D)Arg
  MISC_FEATURE (2)..(2): Xaa is Pen
  MISC_FEATURE (5)..(5): Xaa is W(7-Me)
  MISC_FEATURE (6)..(6): Lys is Lys(Ac)
  MISC_FEATURE (7)..(7): Xaa is Pen
  MISC_FEATURE (8)..(8): Phe is Phe[4-(2-aminoethoxy)]
  MISC_FEATURE (9)..(9): Xaa is 2-Nal
  MISC_FEATURE (10)..(10): Xaa is THP
  MISC_FEATURE (13)..(13): Xaa is THP
RXNTXKXFXXENXP

SEQ ID NO: 223 - protein, 14 aa, Artificial sequence
  Synthetic construct
  MISC_FEATURE (1)..(1): Arg is (D)Arg
  MISC_FEATURE (2)..(2): Xaa is Pen
  MISC_FEATURE (5)..(5): Xaa is W(7-Me)
  MISC_FEATURE (6)..(6): Lys is Lys(Ac)
  MISC_FEATURE (7)..(7): Xaa is Pen
  MISC_FEATURE (8)..(8): Phe is Phe[4-(2-aminoethoxy)]
  MISC_FEATURE (9)..(9): Xaa is 2-Nal
  MISC_FEATURE (10)..(10): Xaa is THP
  MISC_FEATURE (13)..(13): Xaa is THP
  MISC_FEATURE (14)..(14): Pro is (D)Pro
RXNTXKXFXXENXP

SEQ ID NO: 224 - protein, 14 aa, Artificial sequence
  Synthetic construct
  MISC_FEATURE (1)..(1): Arg is (D)Arg
  MISC_FEATURE (2)..(2): Xaa is Pen
  MISC_FEATURE (5)..(5): Xaa is W(7-Me)
  MISC_FEATURE (6)..(6): Lys is Lys(Ac)
  MISC_FEATURE (7)..(7): Xaa is Pen
  MISC_FEATURE (8)..(8): Phe is Phe[4-(2-aminoethoxy)]
  MISC_FEATURE (9)..(9): Xaa is 2-Nal
  MISC_FEATURE (10)..(10): Xaa is 1-aminocyclopentanecarboxylic acid
  MISC_FEATURE (13)..(13): Ala is beta Alanine
  MISC_FEATURE (14)..(14): Xaa is Sarc
RXNTXKXFXXENAX

SEQ ID NO: 225 - protein, 14 aa, Artificial sequence
  Synthetic construct
  MISC_FEATURE (1)..(1): Arg is (D)Arg
  MISC_FEATURE (2)..(2): Xaa is Pen
  MISC_FEATURE (5)..(5): Xaa is W(7-Me)
  MISC_FEATURE (6)..(6): Lys is Lys(Ac)
  MISC_FEATURE (7)..(7): Xaa is Pen
  MISC_FEATURE (8)..(8): Phe is Phe[4-(2-aminoethoxy)]
  MISC_FEATURE (9)..(9): Xaa is 2-Nal
  MISC_FEATURE (10)..(10): Xaa is 1-aminocyclopentanecarboxylic acid
  MISC_FEATURE (13)..(13): Val is (D)Val
  MISC_FEATURE (14)..(14): Xaa is Sarc
RXNTXKXFXXENVX

SEQ ID NO: 226 - protein, 14 aa, Artificial sequence
  Synthetic construct
  MISC_FEATURE (1)..(1): Arg is (D)Arg
  MISC_FEATURE (2)..(2): Xaa is Pen
  MISC_FEATURE (5)..(5): Xaa is W(7-Me)
  MISC_FEATURE (6)..(6): Lys is Lys(Ac)
  MISC_FEATURE (7)..(7): Xaa is Pen
  MISC_FEATURE (8)..(8): Phe is Phe[4-(2-aminoethoxy)]
  MISC_FEATURE (9)..(9): Xaa is 2-Nal
  MISC_FEATURE (10)..(10): Xaa is 1-aminocyclopentanecarboxylic acid
  MISC_FEATURE (13)..(13): Arg is (D)Arg
  MISC_FEATURE (14)..(14): Xaa is Sarc
RXNTXKXFXXENRX

SEQ ID NO: 227 - protein, 14 aa, Artificial sequence
  Synthetic construct
  MISC_FEATURE (1)..(1): Arg is (D)Arg
  MISC_FEATURE (2)..(2): Xaa is Pen
  MISC_FEATURE (5)..(5): Xaa is W(7-Me)
  MISC_FEATURE (6)..(6): Lys is Lys(Ac)
  MISC_FEATURE (7)..(7): Xaa is Pen
  MISC_FEATURE (8)..(8): Phe is Phe[4-(2-aminoethoxy)]
  MISC_FEATURE (9)..(9): Xaa is 2-Nal
  MISC_FEATURE (10)..(10): Xaa is 1-aminocyclopentanecarboxylic acid
  MISC_FEATURE (13)..(3): Xaa is 3,4-dimethoxy-L-homophenylalanine
  misc_feature (13)..(13): Xaa can be any naturally occurring amino acid
  MISC_FEATURE (14)..(14): Xaa is Sarc
RXNTXKXFXXENXX

SEQ ID NO: 228 - protein, 13 aa, Artificial sequence
  Synthetic construct
  MISC_FEATURE (1)..(1): Xaa is Pen
  MISC_FEATURE (4)..(4): Xaa is W(7-Me)
  MISC_FEATURE (5)..(5): Lys is Lys(Ac)
  MISC_FEATURE (6)..(6): Xaa is Pen
  MISC_FEATURE (7)..(7): Phe is Phe[4-(2-aminoethoxy)]
  MISC_FEATURE (8)..(8): Xaa is 2-Nal
  MISC_FEATURE (9)..(9): Xaa is 1-aminocyclopentanecarboxylic acid
  MISC_FEATURE (12)..(12): Phe is Phe[4-NH2]
  MISC_FEATURE (13)..(13): Xaa is Sarc
XNTXKXFXXENFX

SEQ ID NO: 229 - protein, 14 aa, Artificial sequence
  Synthetic construct
  MISC_FEATURE (1)..(1): Arg is (D)Arg
  MISC_FEATURE (2)..(2): Xaa is Pen
  MISC_FEATURE (5)..(5): Xaa is W(7-Me)
  MISC_FEATURE (6)..(6): Lys is Lys(Ac)
  MISC_FEATURE (7)..(7): Xaa is Pen
  MISC_FEATURE (8)..(8): Phe is Phe[4-(2-aminoethoxy)]
  MISC_FEATURE (9)..(9): Xaa is 2-Nal
  MISC_FEATURE (10)..(10): Xaa is 1-aminocyclopentanecarboxylic acid
  MISC_FEATURE (13)..(13): Xaa is Phe[4-NH2]
  MISC_FEATURE (14)..(14): Xaa is Sarc
RXNTXKXFXXENFX

SEQ ID NO: 230 - protein, 14 aa, Artificial sequence
  Synthetic construct
  MISC_FEATURE (1)..(1): Arg is (D)Arg
  MISC_FEATURE (2)..(2): Xaa is Pen
  MISC_FEATURE (5)..(5): Xaa is W(7-Me)
  MISC_FEATURE (6)..(6): Lys is Lys(Ac)
  MISC_FEATURE (7)..(7): Xaa is Pen
  MISC_FEATURE (8)..(8): Phe is Phe[4-(2-aminoethoxy)]
  MISC_FEATURE (9)..(9): Xaa is 2-Nal
  MISC_FEATURE (10)..(10): Xaa is 1-aminocyclopentanecarboxylic acid
  MISC_FEATURE (14)..(14): Xaa is Sarc
RXNTXKXFXXENFX

SEQ ID NO: 231 - protein, 14 aa, Artificial sequence
  Synthetic construct
  MISC_FEATURE (1)..(1): Arg is (D)Arg
  MISC_FEATURE (2)..(2): Xaa is Pen
  MISC_FEATURE (5)..(5): Xaa is W(7-Me)
  MISC_FEATURE (6)..(6): Lys is Lys(Ac)
  MISC_FEATURE (7)..(7): Xaa is Pen
  MISC_FEATURE (8)..(8): Phe is Phe[4-(2-aminoethoxy)]
  MISC_FEATURE (9)..(9): Xaa is 2-Nal
  MISC_FEATURE (10)..(10): Xaa is 1-aminocyclopentanecarboxylic acid
  MISC_FEATURE (13)..(13): Xaa is THP
  MISC_FEATURE (14)..(14): Xaa is Sarc
RXNTXKXFXXENXX

SEQ ID NO: 232 - protein, 14 aa, Artificial sequence
  Synthetic construct
  MISC_FEATURE (1)..(1): Arg is (D)Arg
  MISC_FEATURE (2)..(2): Xaa is Pen
  MISC_FEATURE (5)..(5): Xaa is W(7-Me)
  MISC_FEATURE (6)..(6): Lys is Lys(Ac)
  MISC_FEATURE (7)..(7): Xaa is Pen
  MISC_FEATURE (8)..(8): Phe is Phe[4-(2-aminoethoxy)]
  MISC_FEATURE (9)..(9): Xaa is 2-Nal
  MISC_FEATURE (10)..(10): Xaa is 1-aminocyclopentanecarboxylic acid
  MISC_FEATURE (13)..(13): Leu is (D)Leu
  MISC_FEATURE (14)..(14): Xaa is Sarc
RXNTXKXFXXENLX

SEQ ID NO: 233 - protein, 14 aa, Artificial sequence
  Synthetic construct
  MISC_FEATURE (1)..(1): Arg is (D)Arg
  MISC_FEATURE (5)..(5): Xaa is W(7-Me)
  MISC_FEATURE (6)..(6): Lys is Lys(Ac)
  MISC_FEATURE (7)..(7): Cys is a-MeCys
  MISC_FEATURE (8)..(8): Phe is Phe[4-(2-aminoethoxy)]
  MISC_FEATURE (9)..(9): Xaa is 2-Nal
  MISC_FEATURE (10)..(10): Xaa is 1-aminocyclopentanecarboxylic acid
  MISC_FEATURE (14)..(14): Xaa is Sarc
RCNTXKCFXXENHX

SEQ ID NO: 234 - protein, 14 aa, Artificial sequence
  Synthetic construct
  MISC_FEATURE (1)..(1): Arg is (D)Arg
  MISC_FEATURE (5)..(5): Xaa is W(7-Me)
  MISC_FEATURE (6)..(6): Lys is Lys(Ac)
  MISC_FEATURE (7)..(7): Cys is a-MeCys
  MISC_FEATURE (8)..(8): Phe is Phe[4-(2-aminoethoxy)]
  MISC_FEATURE (9)..(9): Xaa is 2-Nal
  MISC_FEATURE (10)..(10): Xaa is 1-aminocyclopentanecarboxylic acid
  MISC_FEATURE (13)..(13): Leu is (D)Leu
  MISC_FEATURE (14)..(14): Xaa is Sarc
RCNTXKCFXXENLX

SEQ ID NO: 235 - protein, 14 aa, Artificial sequence
  Synthetic construct
  MISC_FEATURE (1)..(1): Arg is (D)Arg
  MISC_FEATURE (2)..(2): Xaa is Pen
  MISC_FEATURE (5)..(5): Xaa is W(7-Me)
  MISC_FEATURE (6)..(6): Lys is Lys(Ac)
  MISC_FEATURE (7)..(7): Xaa is Pen
  MISC_FEATURE (8)..(8): Phe is Phe[4-(2-aminoethoxy)]
  MISC_FEATURE (9)..(9): Xaa is 2-Nal
  MISC_FEATURE (10)..(10): Xaa is 1-aminocyclopentanecarboxylic acid
  MISC_FEATURE (13)..(13): Xaa is 3-Pal
  MISC_FEATURE (14)..(14): Xaa is Sarc
RXNTXKXFXXENXX

SEQ ID NO: 236 - protein, 13 aa, Artificial sequence
  Synthetic construct
  MISC_FEATURE (1)..(1): Xaa is Pen
  MISC_FEATURE (4)..(4): Xaa is W(7-Me)
  MISC_FEATURE (5)..(5): Lys is Lys(Ac)
  MISC_FEATURE (6)..(6): Xaa is Pen
  MISC_FEATURE (7)..(7): Phe is Phe[4-(2-aminoethoxy)]
  MISC_FEATURE (8)..(8): Xaa is 2-Nal
  MISC_FEATURE (9)..(9): Lys is a-MeLys
  MISC_FEATURE (10)..(10): Lys is Lys(Ac)
  MISC_FEATURE (12)..(12): Ala is beta Alanine
  MISC_FEATURE (13)..(13): Xaa is Sarc
XNTXKXFXKKNAX

SEQ ID NO: 237 - protein, 13 aa, Artificial sequence
  Synthetic construct
  MISC_FEATURE (1)..(1): Xaa is Pen
  MISC_FEATURE (4)..(4): Xaa is W(7-Me)
  MISC_FEATURE (5)..(5): Lys is Lys(Ac)
  MISC_FEATURE (6)..(6): Xaa is Pen
  MISC_FEATURE (7)..(7): Phe is [4-(2-aminoethoxy)]
  MISC_FEATURE (8)..(8): Xaa is 2-Nal
  MISC_FEATURE (9)..(9): Lys is a-MeLys
  MISC_FEATURE (10)..(10): Lys is Lys(Ac)
  MISC_FEATURE (12)..(12): Val is (D)Val
  MISC_FEATURE (13)..(13): Xaa is Sarc
XNTXKXFXKKNVX

SEQ ID NO: 238 - protein, 13 aa, Artificial sequence
  Synthetic construct
  MISC_FEATURE (1)..(1): Xaa is Pen
  MISC_FEATURE (4)..(4): Xaa is W(7-Me)
  MISC_FEATURE (5)..(5): Lys is Lys(Ac)
  MISC_FEATURE (6)..(6): Xaa is Pen
  MISC_FEATURE (7)..(7): Phe is Phe[4-(2-aminoethoxy)]
  MISC_FEATURE (8)..(8): Xaa is 2-Nal
  MISC_FEATURE (9)..(9): Lys is a-MeLys
  MISC_FEATURE (10)..(10): Lys is Lys(Ac)
  MISC_FEATURE (12)..(12): Arg is (D)Arg
  MISC_FEATURE (13)..(13): Xaa is Sarc
XNTXKXFXKKNRX

SEQ ID NO: 239 - protein, 13 aa, Artificial sequence
  Synthetic construct
  MISC_FEATURE (1)..(1): Xaa is Pen
  MISC_FEATURE (4)..(4): Xaa is W(7-Me)
  MISC_FEATURE (5)..(5): Lys is Lys(Ac)
  MISC_FEATURE (6)..(6): Xaa is Pen
  MISC_FEATURE (7)..(7): Phe is Phe[4-(2-aminoethoxy)]
  MISC_FEATURE (8)..(8): Xaa is 2-Nal
  MISC_FEATURE (9)..(9): Lys is a-MeLys
  MISC_FEATURE (10)..(10): Lys is Lys(Ac)
  MISC_FEATURE (12)..(12): Xaa is Hph
  MISC_FEATURE (13)..(13): Xaa is Sarc
XNTXKXFXKKNXX

SEQ ID NO: 240 - protein, 13 aa, Artificial sequence
  Synthetic construct
  MISC_FEATURE (1)..(1): Xaa is Pen
  MISC_FEATURE (4)..(4): Xaa is W(7-Me)
  MISC_FEATURE (5)..(5): Lys is Lys(Ac)
  MISC_FEATURE (6)..(6): Xaa is Pen
  MISC_FEATURE (7)..(7): Phe is Phe[4-(2-aminoethoxy)]
  MISC_FEATURE (8)..(8): Xaa is 2-Nal
  MISC_FEATURE (9)..(9): Lys is a-MeLys
  MISC_FEATURE (10)..(10): Lys is Lys(Ac)
  MISC_FEATURE (13)..(13): Xaa is Sarc
XNTXKXFXKKNYX

SEQ ID NO: 241 - protein, 13 aa, Artificial sequence
  Synthetic construct
  MISC_FEATURE (1)..(1): Xaa is Pen
  MISC_FEATURE (4)..(4): Xaa is W(7-Me)
  MISC_FEATURE (5)..(5): Lys is Lys(Ac)
  MISC_FEATURE (6)..(6): Xaa is Pen
  MISC_FEATURE (7)..(7): Phe is Phe[4-(2-aminoethoxy)]
  MISC_FEATURE (8)..(8): Xaa is 2-Nal
  MISC_FEATURE (9)..(9): Lys is a-MeLys
  MISC_FEATURE (10)..(10): Lys is Lys(Ac)
  MISC_FEATURE (13)..(13): Xaa is Sarc
XNTXKXFXKKNYX

SEQ ID NO: 242 - protein, 13 aa, Artificial sequence
  Synthetic construct
  MISC_FEATURE (1)..(1): Arg is (D)Arg
  MISC_FEATURE (2)..(2): Xaa is Pen
  MISC_FEATURE (5)..(5): Xaa is W(7-Me)
  MISC_FEATURE (6)..(6): Lys is Lys(Ac)
  MISC_FEATURE (7)..(7): Xaa is Pen
  MISC_FEATURE (8)..(8): Phe is Phe[4-(2-aminoethoxy)]
  MISC_FEATURE (9)..(9): Xaa is 2-Nal
  MISC_FEATURE (10)..(10): Xaa isTHP
  MISC_FEATURE (13)..(13): Xaa is 4-Pal
RXNTXKXFXXENX

SEQ ID NO: 243 - protein, 13 aa, Artificial sequence
  Synthetic construct
  MISC_FEATURE (1)..(1): Xaa is Pen
  MISC_FEATURE (4)..(4): Xaa is W(7-Me)
  MISC_FEATURE (5)..(5): Lys is Lys(Ac)
  MISC_FEATURE (6)..(6): Xaa is Pen
  MISC_FEATURE (7)..(7): Phe is Phe[4-(2-aminoethoxy)]
  MISC_FEATURE (8)..(8): Xaa is 2-Nal
  MISC_FEATURE (9)..(9): Lys is a-MeLys
  MISC_FEATURE (10)..(10): Lys is Lys(Ac)
  MISC_FEATURE (12)..(12): Phe is Phe(4-CF3)
  MISC_FEATURE (13)..(13): Xaa is Sarc
XNTXKXFXKKNFX

SEQ ID NO: 244 - protein, 13 aa, Artificial sequence
  Synthetic construct
  MISC_FEATURE (1)..(1): Xaa is Pen
  MISC_FEATURE (4)..(4): Xaa is W(7-Me)
  MISC_FEATURE (5)..(5): Lys is Lys(Ac)
  MISC_FEATURE (6)..(6): Xaa is Pen
  MISC_FEATURE (7)..(7): Phe is Phe[4-(2-aminoethoxy)]
  MISC_FEATURE (8)..(8): Xaa is 2-Nal
  MISC_FEATURE (9)..(9): Lys is a-MeLys
  MISC_FEATURE (10)..(10): Lys is Lys(Ac)
  MISC_FEATURE (12)..(12): Tyr is Tyr_CHF2
  MISC_FEATURE (13)..(13): Xaa is Sarc
XNTXKXFXKKNYX

SEQ ID NO: 245 - protein, 13 aa, Artificial sequence
  Synthetic construct
  MISC_FEATURE (1)..(1): Xaa is Pen
  MISC_FEATURE (4)..(4): Xaa is W(7-Me)
  MISC_FEATURE (5)..(5): Lys is Lys(Ac)
  MISC_FEATURE (6)..(6): Xaa is Pen
  MISC_FEATURE (7)..(7): Phe is Phe[4-(2-aminoethoxy)]
  MISC_FEATURE (8)..(8): Xaa is 2-Nal
  MISC_FEATURE (9)..(9): Lys is a-MeLys
  MISC_FEATURE (10)..(10): Lys is Lys(Ac)
  MISC_FEATURE (12)..(12): Xaa is THP
XNTXKXFXKKNXP

SEQ ID NO: 246 - protein, 13 aa, Artificial sequence
  Synthetic construct
  MISC_FEATURE (1)..(1): Xaa is Pen
  MISC_FEATURE (4)..(4): Xaa is W(7-Me)
  MISC_FEATURE (5)..(5): Lys is Lys(Ac)
  MISC_FEATURE (6)..(6): Xaa is Pen
  MISC_FEATURE (7)..(7): Phe is Phe[4-(2-aminoethoxy)]
  MISC_FEATURE (8)..(8): Xaa is 2-Nal
  MISC_FEATURE (9)..(9): Lys is a-MeLys
  MISC_FEATURE (10)..(10): Lys is Lys(Ac)
  MISC_FEATURE (12)..(12): Xaa is 3-Pal
  MISC_FEATURE (13)..(13): Tyr is (D)NMeTyr
XNTXKXFXKKNXY

SEQ ID NO: 247 - protein, 14 aa, Artificial sequence
  Synthetic construct
  MISC_FEATURE (1)..(1): Arg is (D)Arg
  MISC_FEATURE (2)..(2): Xaa is Pen
  MISC_FEATURE (5)..(5): Xaa is W(7-Me)
  MISC_FEATURE (6)..(6): Lys is Lys(Ac)
  MISC_FEATURE (7)..(7): Xaa is Pen
  MISC_FEATURE (8)..(8): Phe is Phe[4-(2-aminoethoxy)]
  MISC_FEATURE (9)..(9): Xaa is 2-Nal
  MISC_FEATURE (10)..(10): Xaa is THP
  MISC_FEATURE (13)..(13): Xaa is 3-Pal
  MISC_FEATURE (14)..(14): Xaa is Sarc
RXNTXKXFXXENXX

SEQ ID NO: 248 - protein, 14 aa, Artificial sequence
  Synthetic construct
  MISC_FEATURE (1)..(1): Arg is (D)Arg
  MISC_FEATURE (2)..(2): Xaa is Pen
  MISC_FEATURE (5)..(5): Xaa is W(7-Me)
  MISC_FEATURE (6)..(6): Lys is Lys(Ac)
  MISC_FEATURE (7)..(7): Xaa is Pen
  MISC_FEATURE (8)..(8): Phe is Phe[4-(2-aminoethoxy)]
  MISC_FEATURE (9)..(9): Xaa is 2-Nal
  MISC_FEATURE (10)..(10): Xaa is THP
  MISC_FEATURE (13)..(13): Xaa is 4-Pal
  MISC_FEATURE (14)..(14): Xaa is Sarc
RXNTXKXFXXENXX

SEQ ID NO: 249 - protein, 14 aa, Artificial sequence
  Synthetic construct
  MISC_FEATURE (1)..(1): Arg is (D)Arg
  MISC_FEATURE (2)..(2): Xaa is Pen
  MISC_FEATURE (5)..(5): Xaa is W(7-Me)
  MISC_FEATURE (6)..(6): Lys is Lys(Ac)
  MISC_FEATURE (7)..(7): Xaa is Pen
  MISC_FEATURE (8)..(8): Phe is Phe[4-(2-aminoethoxy)]
  MISC_FEATURE (9)..(9): Xaa is 2-Nal
  MISC_FEATURE (10)..(10): Xaa is THP
  MISC_FEATURE (13)..(13): Phe is Phe(2-aminomethyl)
  MISC_FEATURE (14)..(14): Xaa is Sarc
RXNTXKXFXXENFX

SEQ ID NO: 250 - protein, 14 aa, Artificial sequence
  Synthetic construct
  MISC_FEATURE (1)..(1): Arg is (D)Arg
  MISC_FEATURE (2)..(2): Xaa is Pen
  MISC_FEATURE (5)..(5): Xaa is W(7-Me)
  MISC_FEATURE (6)..(6): Lys is Lys(Ac)
  MISC_FEATURE (7)..(7): Xaa is Pen
  MISC_FEATURE (8)..(8): Phe is Phe[4-(2-aminoethoxy)]
  MISC_FEATURE (9)..(9): Xaa is 2-Nal
  MISC_FEATURE (10)..(10): Xaa is THP
  MISC_FEATURE (13)..(13): Xaa is 3-Pal
  MISC_FEATURE (14)..(14): Pro is Pro(4,4diF)
RXNTXKXFXXENXP

SEQ ID NO: 251 - protein, 14 aa, Artificial sequence
  Synthetic construct
  MISC_FEATURE (1)..(1): Arg is (D)Arg
  MISC_FEATURE (2)..(2): Xaa is Pen
  MISC_FEATURE (5)..(5): Xaa is W(7-Me)
  MISC_FEATURE (6)..(6): Lys is Lys(Ac)
  MISC_FEATURE (7)..(7): Xaa is Pen
  MISC_FEATURE (8)..(8): Phe is Phe[4-(2-aminoethoxy)]
  MISC_FEATURE (9)..(9): Xaa is 2-Nal
  MISC_FEATURE (10)..(10): Xaa is THP
  MISC_FEATURE (13)..(13): Xaa is 3-Pal
  MISC_FEATURE (14)..(14): Pro is a-MePro
RXNTXKXFXXENXP

SEQ ID NO: 252 - protein, 14 aa, Artificial sequence
  Synthetic construct
  MISC_FEATURE (1)..(1): Arg is (D)Arg
  MISC_FEATURE (2)..(2): Xaa is Pen
  MISC_FEATURE (5)..(5): Xaa is W(7-Me)
  MISC_FEATURE (6)..(6): Lys is Lys(Ac)
  MISC_FEATURE (7)..(7): Xaa is Pen
  MISC_FEATURE (8)..(8): Phe is Phe[4-(2-aminoethoxy)]
  MISC_FEATURE (9)..(9): Xaa is 2-Nal
  MISC_FEATURE (10)..(10): Xaa is THP
  MISC_FEATURE (13)..(13): Xaa is 3-Pal
  MISC_FEATURE (14)..(14): Pro is Aib
RXNTXKXFXXENXX

SEQ ID NO: 253 - protein, 13 aa, Artificial sequence
  Synthetic construct
  MISC_FEATURE (1)..(1): Xaa is Pen
  MISC_FEATURE (4)..(4): Xaa is W(7-Me)
  MISC_FEATURE (5)..(5): Lys is Lys(Ac)
  MISC_FEATURE (6)..(6): Xaa is Pen
  MISC_FEATURE (7)..(7): Phe is Phe[4-(2-aminoethoxy)]
  MISC_FEATURE (8)..(8): Xaa is 2-Nal
  MISC_FEATURE (9)..(9): Lys is a-MeLys
  MISC_FEATURE (10)..(10): Lys is Lys(Ac)
  MISC_FEATURE (12)..(12): His is His(3-Me)
  MISC_FEATURE (13)..(13): Xaa is Sarc
XNTXKXFXKKNHX

SEQ ID NO: 254-260 - skipped (7 entries)

SEQ ID NO: 261 - protein, 14 aa, Artificial sequence
  Synthetic construct
  MISC_FEATURE (1)..(1): Arg is (D)Arg
  MISC_FEATURE (2)..(2): Xaa is Pen
  MISC_FEATURE (5)..(5): Xaa is W(7-Me)
  MISC_FEATURE (6)..(6): Lys is Lys(Ac)
  MISC_FEATURE (7)..(7): Xaa is Pen
  MISC_FEATURE (8)..(8): Phe is Phe[4-(2-aminoethoxy)]
  MISC_FEATURE (9)..(9): Xaa is 2-Nal
  MISC_FEATURE (10)..(10): Xaa is THP
  MISC_FEATURE (13)..(13): Xaa is His(3-Me)
  MISC_FEATURE (14)..(14): Xaa is Sarc
RXNTXKXFXXENHX

SEQ ID NO: 262 - protein, 14 aa, Artificial sequence
  Synthetic construct
  MISC_FEATURE (1)..(1): Arg is (D)Arg
  MISC_FEATURE (2)..(2): Xaa is Pen
  MISC_FEATURE (6)..(6): Lys is Lys(Ac)
  MISC_FEATURE (7)..(7): Xaa is Pen
  MISC_FEATURE (8)..(8): Phe is Phe[4-(2-aminoethoxy)]
  MISC_FEATURE (9)..(9): Xaa is 2-Nal
  MISC_FEATURE (10)..(10): Xaa is THP
  MISC_FEATURE (13)..(13): His is His(3-Me)
  MISC_FEATURE (14)..(14): Xaa is Sarc
RXNTWKXFXXENHX

SEQ ID NO: 263-265 - skipped (3 entries)

SEQ ID NO: 266 - protein, 14 aa, Artificial sequence
  Synthetic construct
  MISC_FEATURE (1)..(1): Arg is (D)Arg
  MISC_FEATURE (2)..(2): Xaa is Pen
  MISC_FEATURE (5)..(5): Xaa is W(7-Me)
  MISC_FEATURE (6)..(6): Lys is Lys(Ac)
  MISC_FEATURE (7)..(7): Xaa is Pen
  MISC_FEATURE (8)..(8): Phe is Phe[4-(2-aminoethoxy)]
  MISC_FEATURE (9)..(9): Xaa is 2-Nal
  MISC_FEATURE (10)..(10): Xaa is THP
  MISC_FEATURE (13)..(13): Xaa is 3-Pal
  MISC_FEATURE (14)..(14): Xaa is Sarc
RXNTXKXFXXENXX

SEQ ID NO: 267 - protein, 14 aa, Artificial sequence
  Synthetic construct
  MISC_FEATURE (1)..(1): Arg is (D)Arg
  MISC_FEATURE (2)..(2): Xaa is Pen
  MISC_FEATURE (5)..(5): Xaa is W(7-Me)
  MISC_FEATURE (6)..(6): Lys is Lys(Ac)
  MISC_FEATURE (7)..(7): Xaa is Pen
  MISC_FEATURE (8)..(8): Phe is Phe[4-(2-aminoethoxy)]
  MISC_FEATURE (9)..(9): Xaa is 2-Nal
  MISC_FEATURE (10)..(10): Xaa is THP
  MISC_FEATURE (13)..(13): Xaa is 3-Pal
  MISC_FEATURE (14)..(14): Xaa is N(H)Me
RXNTXKXFXXENXX

SEQ ID NO: 268-269 - skipped (2 entries)

SEQ ID NO: 270 - protein, 14 aa, Artificial sequence
  Synthetic construct
  MISC_FEATURE (1)..(1): Arg is (D)Arg
  MISC_FEATURE (2)..(1): Xaa is Pen
  misc_feature (2)..(2): Xaa can be any naturally occurring amino acid
  MISC_FEATURE (5)..(5): Xaa is W(7-Me)
  MISC_FEATURE (6)..(6): Lys is Lys(Ac)
  MISC_FEATURE (7)..(7): Xaa is Pen
  MISC_FEATURE (8)..(8): Phe is Phe[4-(2-aminoethoxy)]
  MISC_FEATURE (9)..(9): Xaa is 2-Nal
  MISC_FEATURE (10)..(10): Xaa is THP
  MISC_FEATURE (13)..(13): Xaa is 3-Pal
  MISC_FEATURE (14)..(14): Xaa is Sarc
RXNTXKXFXXENXX

SEQ ID NO: 271 - protein, 14 aa, Artificial sequence
  Synthetic construct
  MISC_FEATURE (1)..(1): Arg is (D)Arg
  MISC_FEATURE (2)..(2): Xaa is Pen
  MISC_FEATURE (6)..(6): Lys is Lys(Ac)
  MISC_FEATURE (7)..(7): Xaa is Pen
  MISC_FEATURE (8)..(8): Phe is Phe[4-(2-aminoethoxy)]
  MISC_FEATURE (9)..(9): Xaa is 2-Nal
  MISC_FEATURE (10)..(10): Xaa is THP
  MISC_FEATURE (13)..(13): Xaa is 3-Pal
  MISC_FEATURE (14)..(14): Xaa is Sarc
RXNTWKXFXXENXX

SEQ ID NO: 272 - protein, 15 aa, Artificial sequence
  Synthetic construct
  MISC_FEATURE (1)..(1): Xaa is Propyl
  MISC_FEATURE (2)..(2): Arg is (D)Arg
  MISC_FEATURE (3)..(3): Xaa is Pen
  MISC_FEATURE (6)..(6): Xaa is W(7-Me)
  MISC_FEATURE (7)..(7): Lys is Lys(Ac)
  MISC_FEATURE (8)..(8): Xaa is Pen
  MISC_FEATURE (9)..(9): Phe is Phe[4-(2-(N-propionylamino)ethoxy)]
  MISC_FEATURE (10)..(10): Xaa is 2-Nal
  MISC_FEATURE (11)..(11): Xaa is THP
  MISC_FEATURE (14)..(14): Xaa is 3-Pal
  MISC_FEATURE (15)..(15): Xaa is Sarc
XRXNTXKXFXXENXX

SEQ ID NO: 273 - protein, 14 aa, Artificial sequence
  Synthetic construct
  MISC_FEATURE (1)..(1): Arg is (D)Arg
  MISC_FEATURE (2)..(2): Xaa is Pen
  MISC_FEATURE (5)..(5): Xaa is W(7-Me)
  MISC_FEATURE (6)..(6): Lys is Lys(Ac)
  MISC_FEATURE (7)..(7): Xaa is Pen
  MISC_FEATURE (8)..(8): Phe is Phe[4-(2-(N-(4-hydroxy-3-methylPhenyl)-propionylamino)
  MISC_FEATURE (9)..(9): Xaa is 2-Nal
  MISC_FEATURE (10)..(10): Xaa is THP
  MISC_FEATURE (13)..(13): Xaa is 3-Pal
  MISC_FEATURE (14)..(14): Xaa is Sarc
RXNTXKXFXXENXX

SEQ ID NO: 274 - protein, 15 aa, Artificial sequence
  Synthetic construct
  MISC_FEATURE (1)..(1): Xaa is N3_Acid
  MISC_FEATURE (2)..(2): Arg is (D)Arg
  MISC_FEATURE (3)..(3): Xaa is Pen
  MISC_FEATURE (6)..(6): Xaa is W(7-Me)
  MISC_FEATURE (7)..(7): Lys is Lys(Ac)
  MISC_FEATURE (8)..(8): Xaa is Pen
  MISC_FEATURE (9)..(9): Phe is Phe[4-(2-aminoethoxy)]
  MISC_FEATURE (10)..(10): Xaa is 2-Nal
  MISC_FEATURE (11)..(11): Xaa is THP
  MISC_FEATURE (13)..(13): Xaa is 3-Pal
  MISC_FEATURE (14)..(14): Xaa is Sarc
  misc_feature (15)..(15): Xaa can be any naturally occurring amino acid
XRXNTXKXFXXENXX

SEQ ID NO: 275 - protein, 15 aa, Artificial sequence
  Synthetic construct
  MISC_FEATURE (1)..(1): Xaa is FPrpTriazoleMe_Acid
  MISC_FEATURE (2)..(2): Arg is (D)Arg
  MISC_FEATURE (3)..(3): Xaa is Pen
  MISC_FEATURE (6)..(6): Xaa is W(7-Me)
  MISC_FEATURE (7)..(7): Lys is Lys(Ac)
  MISC_FEATURE (8)..(8): Xaa is Pen
  MISC_FEATURE (9)..(9): Phe is Phe[4-(2-aminoethoxy)]
  MISC_FEATURE (10)..(10): Xaa is 2-Nal
  MISC_FEATURE (11)..(11): Xaa is THP
  MISC_FEATURE (14)..(14): Xaa is 3-Pal
  MISC_FEATURE (15)..(15): Xaa is Sarc
XRXNTXKXFXXENXX

SEQ ID NO: 276 - protein, 14 aa, Artificial sequence
  Synthetic construct
  MISC_FEATURE (1)..(1): Arg is (D)Arg
  MISC_FEATURE (2)..(2): Xaa is Pen
  MISC_FEATURE (5)..(5): Xaa is W(7-Me)
  MISC_FEATURE (6)..(6): Lys is Lys(Ac)
  MISC_FEATURE (7)..(7): Xaa is Pen
  MISC_FEATURE (8)..(8): Phe is Phe[4-(2-aminoethoxy)]
  MISC_FEATURE (9)..(9): Xaa is 2-Nal
  MISC_FEATURE (10)..(10): Xaa is THP
  MISC_FEATURE (13)..(13): Xaa is 3Pal(5-Me)
  MISC_FEATURE (14)..(14): Xaa is Sarc
RXNTXKXFXXENXX

SEQ ID NO: 277 - protein, 14 aa, Artificial sequence
  Synthetic construct
  MISC_FEATURE (1)..(1): Arg is (D)Arg
  MISC_FEATURE (2)..(2): Xaa is Pen
  MISC_FEATURE (5)..(5): Xaa is W(7-Me)
  MISC_FEATURE (6)..(6): Lys is Lys(Ac)
  MISC_FEATURE (7)..(7): Xaa is Pen
  MISC_FEATURE (8)..(8): Phe is Phe[4-(2-aminoethoxy)]
  MISC_FEATURE (9)..(9): Xaa is 2-Nal
  MISC_FEATURE (10)..(10): Xaa is THP
  MISC_FEATURE (13)..(13): Xaa is 3Pal(5)
  MISC_FEATURE (14)..(14): Xaa is Sarc
RXNTXKXFXXENXX

SEQ ID NO: 278 - protein, 13 aa, Artificial sequence
  Synthetic construct
  MISC_FEATURE (1)..(1): Xaa is Pen
  MISC_FEATURE (4)..(4): Xaa is W(7-Me)
  MISC_FEATURE (5)..(5): Lys is Lys(Ac)
  MISC_FEATURE (6)..(6): Xaa is Pen
  MISC_FEATURE (7)..(7): Phe is Phe[4-(2-aminoethoxy)]
  MISC_FEATURE (8)..(8): Xaa is 2-Nal
  MISC_FEATURE (9)..(9): Xaa is THP
  MISC_FEATURE (12)..(12): His is His(3-Me)
  MISC_FEATURE (13)..(13): Xaa is N(H)Me
XNTXKXFXXENHX

SEQ ID NO: 279 - protein, 14 aa, Artificial sequence
  Synthetic construct
  MISC_FEATURE (1)..(1): Arg is (D)Arg
  MISC_FEATURE (2)..(2): Xaa is Pen
  MISC_FEATURE (5)..(5): Xaa is W(7-Me)
  MISC_FEATURE (6)..(6): Lys is Lys(Ac)
  MISC_FEATURE (7)..(7): Xaa is Pen
  MISC_FEATURE (8)..(8): Phe is Phe[4-(2-aminoethoxy)]
  MISC_FEATURE (9)..(9): Xaa is 2-Nal
  MISC_FEATURE (10)..(10): Xaa is THP
  MISC_FEATURE (13)..(13): Xaa is 3-Pal
  MISC_FEATURE (14)..(14): Tyr is (D)NMeTyr
RXNTXKXFXXENXY

SEQ ID NO: 280 - protein, 14 aa, Artificial sequence
  Synthetic construct
  MISC_FEATURE (1)..(1): Arg is (D)Arg
  MISC_FEATURE (2)..(2): Xaa is Pen
  MISC_FEATURE (5)..(5): Xaa is W(7-Me)
  MISC_FEATURE (6)..(6): Lys is Lys(Ac)
  MISC_FEATURE (7)..(7): Xaa is Pen
  MISC_FEATURE (8)..(8): Phe is Phe[4-(2-aminoethoxy)]
  MISC_FEATURE (9)..(9): Xaa is 2-Nal
  MISC_FEATURE (10)..(10): Xaa is THP
  MISC_FEATURE (13)..(13): Xaa is 3-Pal
  MISC_FEATURE (14)..(14): Xaa is Gly(N cyclohexylmethyl)
RXNTXKXFXXENXG

SEQ ID NO: 281 - protein, 14 aa, Artificial sequence
  Synthetic construct
  MISC_FEATURE (1)..(1): Arg is (D)Arg
  MISC_FEATURE (2)..(2): Xaa is Pen
  MISC_FEATURE (5)..(5): Xaa is W(7-Me)
  MISC_FEATURE (6)..(6): Lys is Lys(Ac)
  MISC_FEATURE (7)..(7): Xaa is Pen
  MISC_FEATURE (8)..(8): Phe is Phe[4-(2-aminoethoxy)]
  MISC_FEATURE (9)..(9): Xaa is 2-Nal
  MISC_FEATURE (10)..(10): Xaa is THP
  MISC_FEATURE (13)..(13): Xaa is 3-Pal
  MISC_FEATURE (14)..(14): Gly is Gly(N isobutyl)
RXNTXKXFXXENXG

SEQ ID NO: 282 - protein, 13 aa, Artificial sequence
  Synthetic construct
  MISC_FEATURE (1)..(1): Arg is (D)Arg
  MISC_FEATURE (2)..(2): Xaa is Pen
  MISC_FEATURE (5)..(5): Xaa is W(7-Me)
  MISC_FEATURE (6)..(6): Lys is Lys(Ac)
  MISC_FEATURE (7)..(7): Xaa is Pen
  MISC_FEATURE (8)..(8): Phe is Phe[4-(2-aminoethoxy)]
  MISC_FEATURE (9)..(9): Xaa is 2-Nal
  MISC_FEATURE (10)..(10): Xaa is THP
  MISC_FEATURE (13)..(13): Xaa is 3Pal(3-Me)
RXNTXKXFXXENX

SEQ ID NO: 283 - protein, 14 aa, Artificial sequence
  Synthetic construct
  MISC_FEATURE (1)..(1): Arg is (D)Arg
  MISC_FEATURE (2)..(2): Xaa is a-MeCys
  MISC_FEATURE (5)..(5): Xaa is W(7-Me)
  MISC_FEATURE (6)..(6): Lys is Lys(Ac)
  MISC_FEATURE (7)..(7): Xaa is Pen
  MISC_FEATURE (8)..(8): Phe is Phe[4-(2-aminoethoxy)]
  MISC_FEATURE (9)..(9): Xaa is 2-Nal
  MISC_FEATURE (10)..(10): Xaa is THP
  MISC_FEATURE (13)..(13): Xaa is 3-Pal
  MISC_FEATURE (14)..(14): Xaa is Sarc
RCNTXKCFXXENXX

SEQ ID NO: 284 - protein, 13 aa, Artificial sequence
  Synthetic construct
  MISC_FEATURE (1)..(1): Xaa is Pen
  MISC_FEATURE (5)..(5): Lys is Lys(Ac)
  MISC_FEATURE (6)..(6): Xaa is Pen
  MISC_FEATURE (7)..(7): Phe is Phe[4-(2-aminoethoxy)]
  MISC_FEATURE (8)..(8): Xaa is 2-Nal
  MISC_FEATURE (9)..(9): Xaa is THP
  MISC_FEATURE (12)..(12): Xaa is 3-Pal
  MISC_FEATURE (13)..(13): Xaa is Sarc
XNTWKXFXXENXX

SEQ ID NO: 285 - protein, 13 aa, Artificial sequence
  Synthetic construct
  MISC_FEATURE (1)..(1): Xaa is Pen
  MISC_FEATURE (5)..(5): Lys is Lys(Ac)
  MISC_FEATURE (6)..(6): Xaa is Pen
  MISC_FEATURE (7)..(7): Phe is Phe[4-(2-aminoethoxy)]
  MISC_FEATURE (8)..(8): Xaa is 2-Nal
  MISC_FEATURE (9)..(9): Xaa is 1-aminocyclopentanecarboxylic acid
  MISC_FEATURE (12)..(12): Xaa is 3-Pal
  MISC_FEATURE (13)..(13): Xaa is Sarc
XNTWKXFXXENXX

SEQ ID NO: 286 - protein, 13 aa, Artificial sequence
  Synthetic construct
  MISC_FEATURE (1)..(1): Xaa is Pen
  MISC_FEATURE (4)..(4): Xaa is W(7-Me)
  MISC_FEATURE (5)..(5): Lys is Lys(Ac)
  MISC_FEATURE (6)..(6): Xaa is Pen
  MISC_FEATURE (7)..(7): Phe is Phe(4)
  MISC_FEATURE (8)..(8): Xaa is 2-Nal
  MISC_FEATURE (9)..(9): Xaa is THP
  MISC_FEATURE (12)..(12): Xaa is 3-Pal
  MISC_FEATURE (13)..(13): Xaa is Sarc
XNTXKXFXXENXX

SEQ ID NO: 287 - protein, 13 aa, Artificial sequence
  Synthetic construct
  MISC_FEATURE (1)..(1): Xaa is Pen
  MISC_FEATURE (2)..(2): Gly is Gly(Allyl)
  MISC_FEATURE (4)..(4): Xaa is W(7-Me)
  MISC_FEATURE (5)..(5): Lys is Lys(Ac)
  MISC_FEATURE (6)..(6): Xaa is Pen
  MISC_FEATURE (7)..(7): Tyr is Tyr(O-Allyl)
  MISC_FEATURE (8)..(8): Xaa is 2-Nal
  MISC_FEATURE (9)..(9): Xaa is THP
  MISC_FEATURE (10)..(10): Lys is Lys(Ac)
  MISC_FEATURE (12)..(12): Xaa is 3-Pal
  MISC_FEATURE (13)..(13): Xaa is Sarc
XGTXKXYXXKNXX

SEQ ID NO: 288 - protein, 13 aa, Artificial sequence
  Synthetic construct
  MISC_FEATURE (1)..(1): Xaa is Pen
  MISC_FEATURE (2)..(2): Glys is Gly(Allyl)
  MISC_FEATURE (4)..(4): Xaa is W(7-Me)
  MISC_FEATURE (5)..(5): Lys is Lys(Ac)
  MISC_FEATURE (6)..(6): Xaa is Pen
  MISC_FEATURE (7)..(7): Tyr is Tyr(O-Allyl)
  MISC_FEATURE (8)..(8): Xaa is 2-Nal
  MISC_FEATURE (9)..(9): Xaa is THP
  MISC_FEATURE (10)..(10): Lys is Lys(Ac)
  MISC_FEATURE (12)..(12): Xaa  is 3-Pal
  MISC_FEATURE (13)..(13): Xaa  is Sarc
XGDXKXYXXKNXX

SEQ ID NO: 289 - protein, 13 aa, Artificial sequence
  Synthetic construct
  MISC_FEATURE (1)..(1): Xaa is Pen
  MISC_FEATURE (2)..(2): Glys is Gly(Allyl)
  MISC_FEATURE (4)..(4): Xaa is W(4-F)
  MISC_FEATURE (5)..(5): Lys is Lys(Ac)
  MISC_FEATURE (6)..(6): Xaa is Pen
  MISC_FEATURE (7)..(7): Tyr is Tyr(O-Allyl)
  MISC_FEATURE (8)..(8): Xaa is 2-Nal
  MISC_FEATURE (9)..(9): Xaa is THP
  MISC_FEATURE (10)..(10): Lys is Lys(Ac)
  MISC_FEATURE (12)..(12): Xaa is 3-Pal
  MISC_FEATURE (13)..(13): Xaa is Sarc
XGTXKXYXXKNXX

SEQ ID NO: 290 - protein, 13 aa, Artificial sequence
  Synthetic construct
  MISC_FEATURE (1)..(1): Xaa is Pen
  MISC_FEATURE (4)..(4): Xaa is W(7-Me)
  MISC_FEATURE (5)..(5): Lys is Lys(Ac)
  MISC_FEATURE (6)..(6): Xaa is Pen
  MISC_FEATURE (7)..(7): Xaa is Phe[4-(2-aminoethoxy)]
  MISC_FEATURE (8)..(8): Xaa is 2-Nal
  MISC_FEATURE (9)..(9): Xaa is THP
  MISC_FEATURE (12)..(12): Xaa is 3-Pal
  MISC_FEATURE (13)..(13): Xaa is Sarc
XNDXKXFXXENXX

SEQ ID NO: 291 - protein, 13 aa, Artificial sequence
  Synthetic construct
  MISC_FEATURE (1)..(1): Xaa is Pen
  MISC_FEATURE (4)..(4): Xaa is W(7-Me)
  MISC_FEATURE (5)..(5): Lys is Lys(Ac)
  MISC_FEATURE (6)..(6): Xaa is Pen
  MISC_FEATURE (7)..(7): Phe is Phe[4-(2-aminoethoxy)]
  MISC_FEATURE (8)..(8): Xaa is 2-Nal
  MISC_FEATURE (9)..(9): Xaa is THP
  MISC_FEATURE (12)..(12): Xaa is 3-Pal
  MISC_FEATURE (13)..(13): Xaa is Sarc
XLTXKXFXXENXX

SEQ ID NO: 292-298 - skipped (7 entries)

SEQ ID NO: 299 - protein, 13 aa, Artificial sequence
  Synthetic construct
  MISC_FEATURE (1)..(1): Xaa is Pen
  MISC_FEATURE (4)..(4): Xaa is W(7-Me)
  MISC_FEATURE (5)..(5): Lys is Lys(Ac)
  MISC_FEATURE (6)..(6): Xaa is Pen
  MISC_FEATURE (7)..(7): Phe is Phe(4)
  MISC_FEATURE (8)..(8): Xaa is 2-Nal
  MISC_FEATURE (9)..(9): Lys is a-MeLys
  MISC_FEATURE (10)..(10): Lys is Lys(Ac)
  MISC_FEATURE (12)..(12): Xaa is 3-Pal
  MISC_FEATURE (13)..(13): Xaa is Sarc
XNTXKXFXKKNXX

SEQ ID NO: 300-307 - skipped (8 entries)

SEQ ID NO: 308 - protein, 13 aa, Artificial sequence
  Synthetic construct
  MISC_FEATURE (1)..(1): Xaa is Pen
  MISC_FEATURE (4)..(4): Xaa is W(7-Me)
  MISC_FEATURE (5)..(5): Lys is Lys(Ac)
  MISC_FEATURE (6)..(6): Xaa is Pen
  MISC_FEATURE (8)..(8): Xaa is 2-Nal
  MISC_FEATURE (9)..(9): Xaa is THP
  MISC_FEATURE (10)..(10): Lys is Lys(Ac)
  MISC_FEATURE (12)..(12): Xaa is 3-Pal
  MISC_FEATURE (13)..(13): Xaa is Sarc
XNTXKXFXXKNXX

SEQ ID NO: 309 - protein, 13 aa, Artificial sequence
  Synthetic construct
  MISC_FEATURE (1)..(1): Xaa is Pen
  MISC_FEATURE (4)..(4): Xaa is W(7-Me)
  MISC_FEATURE (5)..(5): Lys is Lys(Ac)
  MISC_FEATURE (6)..(6): Xaa is Pen
  MISC_FEATURE (8)..(8): Xaa is 2-Nal
  MISC_FEATURE (9)..(9): Xaa is THP
  MISC_FEATURE (10)..(10): Lys is Lys(Ac)
  MISC_FEATURE (12)..(12): Xaa is 3-Pal
  MISC_FEATURE (13)..(13): Xaa is Sarc
XNTXKXYXXKNXX

SEQ ID NO: 310 - protein, 13 aa, Artificial sequence
  Synthetic construct
  MISC_FEATURE (1)..(1): Xaa is Pen
  MISC_FEATURE (4)..(4): Xaa is W(7-Me)]
  MISC_FEATURE (5)..(5): Lys is Lys(Ac)
  MISC_FEATURE (6)..(6): Xaa is Pen
  MISC_FEATURE (7)..(7): Phe is Phe(4-OMe)
  MISC_FEATURE (8)..(8): Xaa is 2-Nal
  MISC_FEATURE (9)..(9): Xaa is THP
  MISC_FEATURE (10)..(10): Lys is Lys(Ac)
  MISC_FEATURE (12)..(12): Xaa is 3-Pal
  MISC_FEATURE (13)..(13): Xaa is Sarc
XNTXKXFXXKNXX

SEQ ID NO: 311 - protein, 13 aa, Artificial sequence
  Synthetic construct
  MISC_FEATURE (1)..(1): Xaa is Pen
  MISC_FEATURE (4)..(4): Xaa is W(7-Me)
  MISC_FEATURE (5)..(5): Lys is Lys(Ac)
  MISC_FEATURE (6)..(6): Xaa is Pen
  MISC_FEATURE (7)..(7): Phe is Phe(4)
  MISC_FEATURE (8)..(8): Xaa is 2-Nal
  MISC_FEATURE (9)..(9): Xaa is THP
  MISC_FEATURE (10)..(10): Lys is Lys(Ac)
  MISC_FEATURE (12)..(12): Xaa is 3-Pal
  MISC_FEATURE (13)..(13): Xaa is Sarc
XNTXKXFXXKNXX

SEQ ID NO: 312-331 - skipped (20 entries)

SEQ ID NO: 332 - protein, 13 aa, Artificial sequence
  Synthetic construct
  MISC_FEATURE (1)..(1)
  MISC_FEATURE (1)..(1): Xaa is Pen
  MISC_FEATURE (4)..(4): Xaa is W(7-Me)
  MISC_FEATURE (5)..(5): Lys is Lys(N-acetyl-N-propyl)
  MISC_FEATURE (6)..(6): Xaa is Pen
  MISC_FEATURE (7)..(7): Phe is Phe[4-(2-aminoethoxy)
  MISC_FEATURE (8)..(8): Xaa is 2-Nal
  MISC_FEATURE (9)..(9): Xaa is THP
  MISC_FEATURE (12)..(12): Xaa is 3-Pal
  MISC_FEATURE (13)..(13): Xaa is Sarc
XNTXKXFXXENXX

SEQ ID NO: 333 - protein, 13 aa, Artificial sequence
  Synthetic construct
  MISC_FEATURE (1)..(1): Xaa is Pen
  MISC_FEATURE (4)..(4): Xaa is W(7-Me)
  MISC_FEATURE (5)..(5): Lys is Lys(N-acetyl-N-butyl)
  MISC_FEATURE (6)..(6): Xaa is Pen
  MISC_FEATURE (7)..(7): Phe is Phe[4-(2-aminoethoxy)]
  MISC_FEATURE (8)..(8): Xaa is 2-Nal
  MISC_FEATURE (9)..(9): Xaa is THP
  MISC_FEATURE (12)..(12): Xaa is 3-Pal
  MISC_FEATURE (13)..(13): Xaa is Sarc
XNTXKXFXXENXX

SEQ ID NO: 334 - protein, 13 aa, Artificial sequence
  Synthetic construct
  MISC_FEATURE (1)..(1): Xaa is Pen
  MISC_FEATURE (4)..(4): Xaa is W(7-Me)
  MISC_FEATURE (5)..(5): Lys is Lys(N-acetyl-N-isobutyl)
  MISC_FEATURE (6)..(6): Xaa is Pen
  MISC_FEATURE (7)..(7): Phe is Phe[4-(2-aminoethoxy)]
  MISC_FEATURE (8)..(8): Xaa is 2-Nal
  MISC_FEATURE (9)..(9): Xaa is THP
  MISC_FEATURE (12)..(12): Xaa is 3-Pal
  MISC_FEATURE (13)..(13): Xaa is Sarc
XNTXKXFXXENXX

SEQ ID NO: 335 - protein, 13 aa, Artificial sequence
  Synthetic construct
  MISC_FEATURE (1)..(1): Xaa is Pen
  MISC_FEATURE (4)..(4): Xaa is W(7-Me)
  MISC_FEATURE (5)..(5): Lys is Lys(N-acetyl-N-benzyl)
  MISC_FEATURE (6)..(6): Xaa is Pen
  MISC_FEATURE (7)..(7): Phe is Phe[4-(2-aminoethoxy)]
  MISC_FEATURE (8)..(8): Xaa is 2-Nal
  MISC_FEATURE (9)..(9): Xaa is THP
  MISC_FEATURE (12)..(12): Xaa is 3-Pal
  MISC_FEATURE (13)..(13): Xaa is Sarc
XNTXKXFXXENXX

SEQ ID NO: 336-338 - skipped (3 entries)

SEQ ID NO: 339 - protein, 13 aa, Artificial sequence
  Synthetic construct
  MISC_FEATURE (1)..(1): Xaa is Pen
  MISC_FEATURE (4)..(4): Xaa is W(7-Me)
  MISC_FEATURE (5)..(5): Lys is Lys(Ac)
  MISC_FEATURE (6)..(6): Xaa is Pen
  MISC_FEATURE (7)..(7): Phe is Phe(4)
  MISC_FEATURE (8)..(8): Xaa is 2-Nal
  MISC_FEATURE (9)..(9): Leu is a-MeLeu
  MISC_FEATURE (12)..(12): Xaa is 3-Pal
  MISC_FEATURE (13)..(13): Xaa is Sarc
XLTXKXFXLENXX

SEQ ID NO: 340-346 - skipped (7 entries)

SEQ ID NO: 347 - protein, 13 aa, Artificial sequence
  Synthetic construct
  MISC_FEATURE (1)..(1): Xaa is Pen
  MISC_FEATURE (4)..(4): Xaa is W(7-Me)
  MISC_FEATURE (5)..(5): Lys is Lys(Ac)
  MISC_FEATURE (6)..(6): Xaa is Pen
  MISC_FEATURE (7)..(7): Phe is Phe(4-OMe)
  MISC_FEATURE (8)..(8): Xaa is 2-Nal
  MISC_FEATURE (9)..(9): Leu is a-MeLeu
  MISC_FEATURE (12)..(12): Xaa is 3-Pal
  MISC_FEATURE (13)..(13): Xaa is Sarc
XLTXKXFXLENXX

SEQ ID NO: 348-372 - skipped (25 entries)

SEQ ID NO: 373 - protein, 13 aa, Artificial sequence
  Synthetic construct
  MISC_FEATURE (1)..(1): Xaa is Abu
  MISC_FEATURE (4)..(4): Xaa is W(7-Me)
  MISC_FEATURE (5)..(5): Lys is Lys(Ac)
  MISC_FEATURE (6)..(6): Xaa is Pen
  MISC_FEATURE (7)..(7): Phe is Phe[4-(2-aminoethoxy)]
  MISC_FEATURE (8)..(8): Xaa is 2-Nal
  MISC_FEATURE (9)..(9): Xaa is THP
  MISC_FEATURE (12)..(12): Xaa is 3-Pal
  MISC_FEATURE (13)..(13): Xaa is Sarc
XNTXKXFXXENXX

SEQ ID NO: 374-377 - skipped (4 entries)

SEQ ID NO: 378 - protein, 13 aa, Artificial sequence
  Synthetic construct
  MISC_FEATURE (1)..(1): Xaa is Pen
  MISC_FEATURE (4)..(4): Xaa is W(7-Me)
  MISC_FEATURE (5)..(5): Lys is Lys(Ac)
  MISC_FEATURE (6)..(6): Xaa is Pen
  MISC_FEATURE (7)..(7): Phe is Phe(4)
  MISC_FEATURE (8)..(8): Xaa is 2-Nal
  MISC_FEATURE (9)..(9): Xaa is THP
  MISC_FEATURE (10)..(10): Lys is Lys(Ac)
  MISC_FEATURE (12)..(12): Xaa is 3-Pal
  MISC_FEATURE (13)..(13): Xaa is Sarc
XNTXKXFXXKIXX

SEQ ID NO: 379 - protein, 13 aa, Artificial sequence
  Synthetic construct
  MISC_FEATURE (1)..(1): Xaa is Pen
  MISC_FEATURE (4)..(4): Xaa is W(7-Me)
  MISC_FEATURE (5)..(5): Lys is Lys(Ac)
  MISC_FEATURE (6)..(6): Xaa is Pen
  MISC_FEATURE (7)..(7): Phe is Phe(4)
  MISC_FEATURE (8)..(8): Xaa is 2-Nal
  MISC_FEATURE (9)..(9): Xaa is THP
  MISC_FEATURE (10)..(10): Lys is Lys(Ac)
  MISC_FEATURE (12)..(12): Xaa is 3-Pal
  MISC_FEATURE (13)..(13): Leu is (D)Leu
XNTXKXFXXKIXL

SEQ ID NO: 380 - protein, 13 aa, Artificial sequence
  Synthetic construct
  MISC_FEATURE (1)..(1): Xaa is Pen
  MISC_FEATURE (4)..(4): Xaa is W(7-Me)
  MISC_FEATURE (5)..(5): Lys is Lys(Ac)
  MISC_FEATURE (6)..(6): Xaa is Pen
  MISC_FEATURE (7)..(7): Phe is Phe(4)
  MISC_FEATURE (8)..(8): Xaa is 2-Nal
  MISC_FEATURE (9)..(9): Xaa is THP
  MISC_FEATURE (10)..(10): Lys is Lys(Ac)
  MISC_FEATURE (12)..(12): Xaa is 3-Pal
  MISC_FEATURE (13)..(13): Leu is a-MeLeu
XNTXKXFXXKIXL

SEQ ID NO: 381 - protein, 13 aa, Artificial sequence
  Synthetic construct
  MISC_FEATURE (1)..(1): Xaa is Pen
  MISC_FEATURE (4)..(4): Xaa is W(7-Me)
  MISC_FEATURE (5)..(5): Lys is Lys(Ac)
  MISC_FEATURE (6)..(6): Xaa is Pen
  MISC_FEATURE (7)..(7): Phe is Phe(4)
  MISC_FEATURE (8)..(8): Xaa is 2-Nal
  MISC_FEATURE (9)..(9): Xaa is THP
  MISC_FEATURE (10)..(10): Lys is Lys(Ac)
  MISC_FEATURE (12)..(12): Xaa is 3-Pal
  MISC_FEATURE (13)..(13): Xaa is aMe-Nle
XNTXKXFXXKIXX

SEQ ID NO: 382 - protein, 13 aa, Artificial sequence
  Synthetic construct
  MISC_FEATURE (1)..(1): Xaa is Pen
  MISC_FEATURE (4)..(4): Xaa is W(7-Me)
  MISC_FEATURE (5)..(5): Lys is Lys(Ac)
  MISC_FEATURE (6)..(6): Xaa is Pen
  MISC_FEATURE (7)..(7): Phe is Phe(4)
  MISC_FEATURE (8)..(8): Xaa is 2-Nal
  MISC_FEATURE (9)..(9): Xaa is THP
  MISC_FEATURE (10)..(10): Lys is Lys(Ac)
  MISC_FEATURE (12)..(12): Xaa is 3-Pal
  MISC_FEATURE (13)..(13): Xaa is Sarc
XITXKXFXXKIXX

SEQ ID NO: 383 - protein, 13 aa, Artificial sequence
  Synthetic construct
  MISC_FEATURE (1)..(1): Xaa is Pen
  MISC_FEATURE (4)..(4): Xaa is W(7-Me)
  MISC_FEATURE (5)..(5): Lys is Lys(Ac)
  MISC_FEATURE (6)..(6): Xaa is Pen
  MISC_FEATURE (7)..(7): Phe is Phe(4)
  MISC_FEATURE (8)..(8): Xaa is 2-Nal
  MISC_FEATURE (9)..(9): Xaa is THP
  MISC_FEATURE (10)..(10): Lys is Lys(Ac)
  MISC_FEATURE (12)..(12): Xaa is 3-Pal
  MISC_FEATURE (13)..(13): Leu is (D)Leu
XITXKXFXXKIXL

SEQ ID NO: 384 - protein, 13 aa, Artificial sequence
  Synthetic construct
  MISC_FEATURE (1)..(1): Xaa is Pen
  MISC_FEATURE (4)..(4): Xaa is W(7-Me)
  MISC_FEATURE (5)..(5): Lys is Lys(Ac)
  MISC_FEATURE (6)..(6): Xaa is Pen
  MISC_FEATURE (7)..(7): Phe is Phe(4)
  MISC_FEATURE (8)..(8): Xaa is 2-Nal
  MISC_FEATURE (9)..(9): Xaa is THP
  MISC_FEATURE (10)..(10): Lys is Lys(Ac)
  MISC_FEATURE (12)..(12): Xaa is 3-Pal
  MISC_FEATURE (13)..(13): Leu is a-Me-Leu
XITXKXFXXKIXL

SEQ ID NO: 385-444 - skipped (60 entries)

SEQ ID NO: 445 - protein, 13 aa, Artificial sequence
  Synthetic construct
  MISC_FEATURE (1)..(1): Xaa is Pen
  MISC_FEATURE (4)..(4): Xaa is W(7-Me)
  MISC_FEATURE (5)..(5): Lys is Lys(Ac)
  MISC_FEATURE (6)..(6): Xaa is Pen
  MISC_FEATURE (7)..(7): Phe is Phe(4-OMe)
  MISC_FEATURE (8)..(8): Xaa is 2-Nal
  MISC_FEATURE (9)..(9): Lys is a-MeLys
  MISC_FEATURE (10)..(10): Lys is Lys(Ac)
  MISC_FEATURE (12)..(12): Xaa is 3-Pal
  MISC_FEATURE (13)..(13): Xaa is Sarc
XNTXKXFXKKAXX

SEQ ID NO: 446 - protein, 13 aa, Artificial sequence
  Synthetic construct
  MISC_FEATURE (1)..(1): Xaa is Pen
  MISC_FEATURE (4)..(4): Xaa is W(7-Me)
  MISC_FEATURE (5)..(5): Lys is Lys(Ac)
  MISC_FEATURE (6)..(6): Xaa is Pen
  MISC_FEATURE (7)..(7): Phe is Phe(4-OMe)
  MISC_FEATURE (8)..(8): Xaa is 2-Nal
  MISC_FEATURE (9)..(9): Lys is a-MeLys
  MISC_FEATURE (10)..(10): Lys is Lys(Ac)
  MISC_FEATURE (12)..(12): Xaa is 3-Pal
  MISC_FEATURE (13)..(13): Xaa is Sarc
XATXKXFXKKAXX

SEQ ID NO: 447 - protein, 20 aa, Artificial sequence
  Synthetic construct
NWQPWSSPFVHQTSQETGKR

SEQ ID NO: 448 - protein, 13 aa, Artificial sequence
  Synthetic construct
  MISC_FEATURE (1)..(1): Xaa is Abu
  MISC_FEATURE (4)..(4): Xaa is is unsubstituted Trp, or Trp substituted with cyano, halo, alkyl, haloalkyl, hydroxy, alkoxy, substituted or unsubstituted aryl, or substituted or unsubstituted heteroaryl
  MISC_FEATURE (7)..(7): Xaa is Tyr, or substituted Tyr, unsubstituted Phe, or Phe substituted with halo, alkyl, haloalkyl, hydroxy, alkoxy, cyano, cycloalkyl, carboxy, carboxamido, 2-aminoethoxy, or 2-acetylaminoethoxy
  MISC_FEATURE (8)..(8): Xaa is 2-Nal, Phe(2-Me), Phe(3-Me), Phe(4-Me), Phe(3,4-dimethoxy), 2Quin, 3Quin, 1-Nal, unsubstituted Trp, or Trp substituted with cyano, halo, alkyl, haloalkyl, hydroxy, or alkoxy
  MISC_FEATURE (9)..(9): Xaa is 4-amino-4-carboxy-tetrahydropyran (THP), Acvc, alpha-MeLys, alpha-MeLeu, alpha-MeArg, alpha-MePhe, alpha-MeLeu, alpha-MeLys, alpha-MeAsn, alpha-MeTyr, Ala, cyclohexylAla, Lys, or Aib
  MISC_FEATURE (10)..(11): Xaa is any amino acid
  MISC_FEATURE (12)..(12): Xaa is Pal
  MISC_FEATURE (13)..(13): Xaa is any amino acid
XNTXQCXXXXXXX

SEQ ID NO: 449 - protein, 13 aa, Artificial sequence
  Synthetic construct
  MISC_FEATURE (1)..(1): Xaa is Abu
  MISC_FEATURE (4)..(4): Xaa is is unsubstituted Trp, or Trp substituted with cyano, halo, alkyl, haloalkyl, hydroxy, alkoxy, substituted or unsubstituted aryl, or substituted or unsubstituted heteroaryl
  MISC_FEATURE (7)..(7): Tyr, or substituted Tyr, unsubstituted Phe, or Phe substituted with halo, alkyl, haloalkyl, hydroxy, alkoxy, cyano, cycloalkyl, carboxy, carboxamido, 2-aminoethoxy, or 2-acetylaminoethoxy
  MISC_FEATURE (8)..(8): Xaa is 2-Nal, Phe(2-Me), Phe(3-Me), Phe(4-Me), Phe(3,4-dimethoxy), 2Quin, 3Quin, 1-Nal, unsubstituted Trp, or Trp substituted with cyano, halo, alkyl, haloalkyl, hydroxy, or alkoxy
  MISC_FEATURE (9)..(9): Xaa is 4-amino-4-carboxy-tetrahydropyran (THP), Acvc, alpha-MeLys, alpha-MeLeu, alpha-MeArg, alpha-MePhe, alpha-MeLeu, alpha-MeLys, alpha-MeAsn, alpha-MeTyr, Ala, cyclohexylAla, Lys, or Aib
  MISC_FEATURE (10)..(11): Xaa is any amino acid
  MISC_FEATURE (12)..(12): Xaa is any amino acid
  MISC_FEATURE (13)..(13): Xaa is Sarc
XNTXQCXXXXXXX

SEQ ID NO: 450 - protein, 13 aa, Artificial sequence
  Synthetic construct
  MISC_FEATURE (1)..(1): Xaa is Pen
  MISC_FEATURE (4)..(4): Xaa is is unsubstituted Trp, or Trp substituted with cyano, halo, alkyl, haloalkyl, hydroxy, alkoxy, substituted or unsubstituted aryl, or substituted or unsubstituted heteroaryl
  MISC_FEATURE (6)..(6): Xaa is Pen
  MISC_FEATURE (7)..(7): Tyr, or substituted Tyr, unsubstituted Phe, or Phe substituted with halo, alkyl, haloalkyl, hydroxy, alkoxy, cyano, cycloalkyl, carboxy, carboxamido, 2-aminoethoxy, or 2-acetylaminoethoxy
  MISC_FEATURE (8)..(8): Xaa is 2-Nal, Phe(2-Me), Phe(3-Me), Phe(4-Me), Phe(3,4-dimethoxy), 2Quin, 3Quin, 1-Nal, unsubstituted Trp, or Trp substituted with cyano, halo, alkyl, haloalkyl, hydroxy, or alkoxy
  MISC_FEATURE (9)..(9): Xaa is 4-amino-4-carboxy-tetrahydropyran (THP), Acvc, alpha-MeLys, alpha-MeLeu, alpha-MeArg, alpha-MePhe, alpha-MeLeu, alpha-MeLys, alpha-MeAsn, alpha-MeTyr, Ala, cyclohexylAla, Lys, or Aib
  MISC_FEATURE (10)..(11): Xaa is any amino acid
  MISC_FEATURE (12)..(12): Xaa is any amino acid
  MISC_FEATURE (13)..(13): Tyr is (D)NMeTyr
XNTXQXXXXXXXY

SEQ ID NO: 451 - protein, 13 aa, Artificial sequence
  Synthetic construct
  MISC_FEATURE (1)..(1): Xaa is Pen
  MISC_FEATURE (4)..(4): Xaa is is unsubstituted Trp, or Trp substituted with cyano, halo, alkyl, haloalkyl, hydroxy, alkoxy, substituted or unsubstituted aryl, or substituted or unsubstituted heteroaryl
  MISC_FEATURE (6)..(6): Xaa is Pen
  MISC_FEATURE (7)..(7): Tyr, or substituted Tyr, unsubstituted Phe, or Phe substituted with halo, alkyl, haloalkyl, hydroxy, alkoxy, cyano, cycloalkyl, carboxy, carboxamido, 2-aminoethoxy, or 2-acetylaminoethoxy
  MISC_FEATURE (8)..(8): Xaa is 2-Nal, Phe(2-Me), Phe(3-Me), Phe(4-Me), Phe(3,4-dimethoxy), 2Quin, 3Quin, 1-Nal, unsubstituted Trp, or Trp substituted with cyano, halo, alkyl, haloalkyl, hydroxy, or alkoxy
  MISC_FEATURE (9)..(9): Xaa is 4-amino-4-carboxy-tetrahydropyran (THP), Acvc, alpha-MeLys, alpha-MeLeu, alpha-MeArg, alpha-MePhe, alpha-MeLeu, alpha-MeLys, alpha-MeAsn, alpha-MeTyr, Ala, cyclohexylAla, Lys, or Aib
  MISC_FEATURE (10)..(11): Xaa is any amino acid
  MISC_FEATURE (12)..(12): Xaa is any amino acid
  MISC_FEATURE (13)..(13): Tyr is (D)NMeTyr
XQTXQXXXXXXXY

SEQ ID NO: 452 - protein, 13 aa, Artificial sequence
  Synthetic construct
  MISC_FEATURE (1)..(1): Xaa is Abu
  MISC_FEATURE (4)..(4): Xaa is is unsubstituted Trp, or Trp substituted with cyano, halo, alkyl, haloalkyl, hydroxy, alkoxy, substituted or unsubstituted aryl, or substituted or unsubstituted heteroaryl
  MISC_FEATURE (7)..(7): Tyr, or substituted Tyr, unsubstituted Phe, or Phe substituted with halo, alkyl, haloalkyl, hydroxy, alkoxy, cyano, cycloalkyl, carboxy, carboxamido, 2-aminoethoxy, or 2-acetylaminoethoxy
  MISC_FEATURE (8)..(8): Xaa is 2-Nal, Phe(2-Me), Phe(3-Me), Phe(4-Me), Phe(3,4-dimethoxy), 2Quin, 3Quin, 1-Nal, unsubstituted Trp, or Trp substituted with cyano, halo, alkyl, haloalkyl, hydroxy, or alkoxy
  MISC_FEATURE (9)..(9): Xaa is 4-amino-4-carboxy-tetrahydropyran (THP), Acvc, alpha-MeLys, alpha-MeLeu, alpha-MeArg, alpha-MePhe, alpha-MeLeu, alpha-MeLys, alpha-MeAsn, alpha-MeTyr, Ala, cyclohexylAla, Lys, or Aib
  MISC_FEATURE (10)..(11): Xaa is any amino acid
  MISC_FEATURE (12)..(12): Xaa is any amino acid
  MISC_FEATURE (13)..(13): Tyr is (D)NMeTyr
XNTXQCXXXXXXY

SEQ ID NO: 453 - protein, 13 aa, Artificial sequence
  Synthetic construct
  MISC_FEATURE (1)..(1): Xaa is Abu
  MISC_FEATURE (4)..(4): Xaa is is unsubstituted Trp, or Trp substituted with cyano, halo, alkyl, haloalkyl, hydroxy, alkoxy, substituted or unsubstituted aryl, or substituted or unsubstituted heteroaryl
  MISC_FEATURE (6)..(6): Xaa is Pen
  MISC_FEATURE (7)..(7): Tyr, or substituted Tyr, unsubstituted Phe, or Phe substituted with halo, alkyl, haloalkyl, hydroxy, alkoxy, cyano, cycloalkyl, carboxy, carboxamido, 2-aminoethoxy, or 2-acetylaminoethoxy
  MISC_FEATURE (8)..(8): Xaa is 2-Nal, Phe(2-Me), Phe(3-Me), Phe(4-Me), Phe(3,4-dimethoxy), 2Quin, 3Quin, 1-Nal, unsubstituted Trp, or Trp substituted with cyano, halo, alkyl, haloalkyl, hydroxy, or alkoxy
  MISC_FEATURE (9)..(9): Xaa is 4-amino-4-carboxy-tetrahydropyran (THP), Acvc, alpha-MeLys, alpha-MeLeu, alpha-MeArg, alpha-MePhe, alpha-MeLeu, alpha-MeLys, alpha-MeAsn, alpha-MeTyr, Ala, cyclohexylAla, Lys, or Aib
  MISC_FEATURE (10)..(11): Xaa is any amino acid
  MISC_FEATURE (12)..(12): Xaa is any amino acid
  MISC_FEATURE (13)..(13): Tyr is (D)NMeTyr
XQTXQXXXXXXXY

SEQ ID NO: 454 - protein, 13 aa, Artificial sequence
  Synthetic construct
  MISC_FEATURE (1)..(1): Xaa is Pen
  MISC_FEATURE (4)..(4): Xaa is is unsubstituted Trp, or Trp substituted with cyano, halo, alkyl, haloalkyl, hydroxy, alkoxy, substituted or unsubstituted aryl, or substituted or unsubstituted heteroaryl
  MISC_FEATURE (6)..(6): Xaa is Pen
  MISC_FEATURE (7)..(7): Phe is Phe[4-(2-aminoethoxy)
  MISC_FEATURE (8)..(8): Xaa is 2-Nal, Phe(2-Me), Phe(3-Me), Phe(4-Me), Phe(3,4-dimethoxy), 2Quin, 3Quin, 1-Nal, unsubstituted Trp, or Trp substituted with cyano, halo, alkyl, haloalkyl, hydroxy, or alkoxy
  MISC_FEATURE (9)..(9): Xaa is 4-amino-4-carboxy-tetrahydropyran (THP), Acvc, alpha-MeLys, alpha-MeLeu, alpha-MeArg, alpha-MePhe, alpha-MeLeu, alpha-MeLys, alpha-MeAsn, alpha-MeTyr, Ala, cyclohexylAla, Lys, or Aib
  MISC_FEATURE (10)..(11): Xaa is any amino acid
  MISC_FEATURE (12)..(12): Xaa is 2-Pal, 3-Pal, or 4-Pal
  MISC_FEATURE (13)..(13): Xaa is any amino acid
XNTXQXFXXXXXX

SEQ ID NO: 455 - protein, 13 aa, Artificial sequence
  Synthetic construct
  MISC_FEATURE (1)..(1): Xaa is Pen
  MISC_FEATURE (4)..(4): Xaa is is unsubstituted Trp, or Trp substituted with cyano, halo, alkyl, haloalkyl, hydroxy, alkoxy, substituted or unsubstituted aryl, or substituted or unsubstituted heteroaryl
  MISC_FEATURE (6)..(6): Xaa is Pen
  MISC_FEATURE (7)..(7): Phe is Phe[4-(2-aminoethoxy)
  MISC_FEATURE (8)..(8): Xaa is 2-Nal, Phe(2-Me), Phe(3-Me), Phe(4-Me), Phe(3,4-dimethoxy), 2Quin, 3Quin, 1-Nal, unsubstituted Trp, or Trp substituted with cyano, halo, alkyl, haloalkyl, hydroxy, or alkoxy
  MISC_FEATURE (9)..(9): Xaa is 4-amino-4-carboxy-tetrahydropyran (THP), Acvc, alpha-MeLys, alpha-MeLeu, alpha-MeArg, alpha-MePhe, alpha-MeLeu, alpha-MeLys, alpha-MeAsn, alpha-MeTyr, Ala, cyclohexylAla, Lys, or Aib
  MISC_FEATURE (10)..(11): Xaa is 4-amino-4-carboxy-tetrahydropyran (THP), Acvc, alpha-MeLys, alpha-MeLeu, alpha-MeArg, alpha-MePhe, alpha-MeLeu, alpha-MeLys, alpha-MeAsn, alpha-MeTyr, Ala, cyclohexylAla, Lys, or Aib
  MISC_FEATURE (12)..(12): Xaa is 2Pal, 3Pal, or 4Pal
  MISC_FEATURE (13)..(13): Xaa is any amino acid
XQTXQXFXXXXXX

SEQ ID NO: 456 - protein, 13 aa, Artificial sequence
  Synthetic construct
  MISC_FEATURE (1)..(1): Xaa is Abu
  MISC_FEATURE (4)..(4): Xaa is is unsubstituted Trp, or Trp substituted with cyano, halo, alkyl, haloalkyl, hydroxy, alkoxy, substituted or unsubstituted aryl, or substituted or unsubstituted heteroaryl
  MISC_FEATURE (7)..(7): Phe is Phe[4-(2-aminoethoxy)
  MISC_FEATURE (8)..(8): Xaa is 2-Nal, Phe(2-Me), Phe(3-Me), Phe(4-Me), Phe(3,4-dimethoxy), 2Quin, 3Quin, 1-Nal, unsubstituted Trp, or Trp substituted with cyano, halo, alkyl, haloalkyl, hydroxy, or alkoxy
  MISC_FEATURE (9)..(9): Xaa is 4-amino-4-carboxy-tetrahydropyran (THP), Acvc, alpha-MeLys, alpha-MeLeu, alpha-MeArg, alpha-MePhe, alpha-MeLeu, alpha-MeLys, alpha-MeAsn, alpha-MeTyr, Ala, cyclohexylAla, Lys, or Aib
  MISC_FEATURE (10)..(11): Xaa is any amino acid
  MISC_FEATURE (12)..(12): Xaa is 2Pal, 3Pal, or 4Pal
  MISC_FEATURE (13)..(13): Xaa is any amino acid
XNTXQCFXXXXXX

SEQ ID NO: 457 - protein, 13 aa, Artificial sequence
  Synthetic construct
  MISC_FEATURE (1)..(1): Xaa is Abu
  MISC_FEATURE (4)..(4): Xaa is is unsubstituted Trp, or Trp substituted with cyano, halo, alkyl, haloalkyl, hydroxy, alkoxy, substituted or unsubstituted aryl, or substituted or unsubstituted heteroaryl
  MISC_FEATURE (6)..(6): Xaa is Pen
  MISC_FEATURE (7)..(7): Phe is Phe[4-(2-aminoethoxy)
  MISC_FEATURE (8)..(8): Xaa is 2-Nal, Phe(2-Me), Phe(3-Me), Phe(4-Me), Phe(3,4-dimethoxy), 2Quin, 3Quin, 1-Nal, unsubstituted Trp, or Trp substituted with cyano, halo, alkyl, haloalkyl, hydroxy, or alkoxy
  MISC_FEATURE (9)..(9): Xaa is 4-amino-4-carboxy-tetrahydropyran (THP), Acvc, alpha-MeLys, alpha-MeLeu, alpha-MeArg, alpha-MePhe, alpha-MeLeu, alpha-MeLys, alpha-MeAsn, alpha-MeTyr, Ala, cyclohexylAla, Lys, or Aib
  MISC_FEATURE (10)..(11): Xaa is any amino acid
  MISC_FEATURE (12)..(12): Xaa is 2Pal, 3Pal, or 4Pal
  MISC_FEATURE (13)..(13): Xaa is any amino acid
XQTXQXFXXXXXX

SEQ ID NO: 458 - protein, 13 aa, Artificial sequence
  Synthetic construct
  MISC_FEATURE (1)..(1): Xaa is Abu
  MISC_FEATURE (4)..(4): Xaa is is unsubstituted Trp, or Trp substituted with cyano, halo, alkyl, haloalkyl, hydroxy, alkoxy, substituted or unsubstituted aryl, or substituted or unsubstituted heteroaryl
  MISC_FEATURE (6)..(6): Xaa is Pen
  MISC_FEATURE (7)..(7): Phe is Phe[4-(2-aminoethoxy)
  MISC_FEATURE (8)..(8): Xaa is 2-Nal, Phe(2-Me), Phe(3-Me), Phe(4-Me), Phe(3,4-dimethoxy), 2Quin, 3Quin, 1-Nal, unsubstituted Trp, or Trp substituted with cyano, halo, alkyl, haloalkyl, hydroxy, or alkoxy
  MISC_FEATURE (9)..(9): Xaa is 4-amino-4-carboxy-tetrahydropyran (THP), Acvc, alpha-MeLys, alpha-MeLeu, alpha-MeArg, alpha-MePhe, alpha-MeLeu, alpha-MeLys, alpha-MeAsn, alpha-MeTyr, Ala, cyclohexylAla, Lys, or Aib
  MISC_FEATURE (10)..(11): Xaa is any amino acid
  MISC_FEATURE (12)..(12): Xaa is any amino acid
  MISC_FEATURE (13)..(13): Xaa is Sarc
XNTXQXFXXXXXX

SEQ ID NO: 459 - protein, 13 aa, Artificial sequence
  Synthetic construct
  MISC_FEATURE (1)..(1): Xaa is Pen
  MISC_FEATURE (4)..(4): Xaa is is unsubstituted Trp, or Trp substituted with cyano, halo, alkyl, haloalkyl, hydroxy, alkoxy, substituted or unsubstituted aryl, or substituted or unsubstituted heteroaryl
  MISC_FEATURE (6)..(6): Xaa is Pen
  MISC_FEATURE (7)..(7): Phe is Phe[4-(2-aminoethoxy)
  MISC_FEATURE (8)..(8): Xaa is 2-Nal, Phe(2-Me), Phe(3-Me), Phe(4-Me), Phe(3,4-dimethoxy), 2Quin, 3Quin, 1-Nal, unsubstituted Trp, or Trp substituted with cyano, halo, alkyl, haloalkyl, hydroxy, or alkoxy
  MISC_FEATURE (9)..(9): Xaa is 4-amino-4-carboxy-tetrahydropyran (THP), Acvc, alpha-MeLys, alpha-MeLeu, alpha-MeArg, alpha-MePhe, alpha-MeLeu, alpha-MeLys, alpha-MeAsn, alpha-MeTyr, Ala, cyclohexylAla, Lys, or Aib
  MISC_FEATURE (10)..(11): Xaa is 4-amino-4-carboxy-tetrahydropyran (THP), Acvc, alpha-MeLys, alpha-MeLeu, alpha-MeArg, alpha-MePhe, alpha-MeLeu, alpha-MeLys, alpha-MeAsn, alpha-MeTyr, Ala, cyclohexylAla, Lys, or Aib
  MISC_FEATURE (12)..(12): Xaa is any amino acid
  MISC_FEATURE (13)..(13): Xaa is Sarc
XQTXQXFXXXXXX

SEQ ID NO: 460 - protein, 13 aa, Artificial sequence
  Synthetic construct
  MISC_FEATURE (1)..(1): Xaa is Abu
  MISC_FEATURE (4)..(4): Xaa is is unsubstituted Trp, or Trp substituted with cyano, halo, alkyl, haloalkyl, hydroxy, alkoxy, substituted or unsubstituted aryl, or substituted or unsubstituted heteroaryl
  MISC_FEATURE (7)..(7): Phe is Phe[4-(2-aminoethoxy)
  MISC_FEATURE (8)..(8): Xaa is 2-Nal, Phe(2-Me), Phe(3-Me), Phe(4-Me), Phe(3,4-dimethoxy), 2Quin, 3Quin, 1-Nal, unsubstituted Trp, or Trp substituted with cyano, halo, alkyl, haloalkyl, hydroxy, or alkoxy
  MISC_FEATURE (9)..(9): Xaa is 4-amino-4-carboxy-tetrahydropyran (THP), Acvc, alpha-MeLys, alpha-MeLeu, alpha-MeArg, alpha-MePhe, alpha-MeLeu, alpha-MeLys, alpha-MeAsn, alpha-MeTyr, Ala, cyclohexylAla, Lys, or Aib
  MISC_FEATURE (10)..(11): Xaa is any amino acid
  MISC_FEATURE (12)..(12): Xaa is any amino acid
  MISC_FEATURE (13)..(13): Xaa is Sarc
XNTXQCFXXXXXX

SEQ ID NO: 461 - protein, 13 aa, Artificial sequence
  Synthetic construct
  MISC_FEATURE (1)..(1): Xaa is Abu
  MISC_FEATURE (4)..(4): Xaa is is unsubstituted Trp, or Trp substituted with cyano, halo, alkyl, haloalkyl, hydroxy, alkoxy, substituted or unsubstituted aryl, or substituted or unsubstituted heteroaryl
  MISC_FEATURE (6)..(6): Xaa is Pen
  MISC_FEATURE (7)..(7): Phe is Phe[4-(2-aminoethoxy)
  MISC_FEATURE (8)..(8): Xaa is 2-Nal, Phe(2-Me), Phe(3-Me), Phe(4-Me), Phe(3,4-dimethoxy), 2Quin, 3Quin, 1-Nal, unsubstituted Trp, or Trp substituted with cyano, halo, alkyl, haloalkyl, hydroxy, or alkoxy
  MISC_FEATURE (9)..(9): Xaa is 4-amino-4-carboxy-tetrahydropyran (THP), Acvc, alpha-MeLys, alpha-MeLeu, alpha-MeArg, alpha-MePhe, alpha-MeLeu, alpha-MeLys, alpha-MeAsn, alpha-MeTyr, Ala, cyclohexylAla, Lys, or Aib
  MISC_FEATURE (10)..(11): Xaa is any amino acid
  MISC_FEATURE (12)..(12): Xaa is any amino acid
  MISC_FEATURE (13)..(13): Xaa is Sarc
XQTXQXFXXXXXX

SEQ ID NO: 462 - protein, 13 aa, Artificial sequence
  Synthetic construct
  MISC_FEATURE (1)..(1): Xaa is Pen
  MISC_FEATURE (4)..(4): Xaa is is unsubstituted Trp, or Trp substituted with cyano, halo, alkyl, haloalkyl, hydroxy, alkoxy, substituted or unsubstituted aryl, or substituted or unsubstituted heteroaryl
  MISC_FEATURE (6)..(6): Xaa is Pen
  MISC_FEATURE (7)..(7): Phe is Phe[4-(2-aminoethoxy)
  MISC_FEATURE (8)..(8): Xaa is 2-Nal, Phe(2-Me), Phe(3-Me), Phe(4-Me), Phe(3,4-dimethoxy), 2Quin, 3Quin, 1-Nal, unsubstituted Trp, or Trp substituted with cyano, halo, alkyl, haloalkyl, hydroxy, or alkoxy
  MISC_FEATURE (9)..(9): Xaa is 4-amino-4-carboxy-tetrahydropyran (THP), Acvc, alpha-MeLys, alpha-MeLeu, alpha-MeArg, alpha-MePhe, alpha-MeLeu, alpha-MeLys, alpha-MeAsn, alpha-MeTyr, Ala, cyclohexylAla, Lys, or Aib
  MISC_FEATURE (10)..(11): Xaa is any amino acid
  MISC_FEATURE (12)..(12): Xaa is any amino acid
  MISC_FEATURE (13)..(13): Tyr is (D)NMeTyr
XNTXQXFXXXXXY

SEQ ID NO: 463 - protein, 13 aa, Artificial sequence
  Synthetic construct
  MISC_FEATURE (1)..(1): Xaa is Pen
  MISC_FEATURE (4)..(4): Xaa is is unsubstituted Trp, or Trp substituted with cyano, halo, alkyl, haloalkyl, hydroxy, alkoxy, substituted or unsubstituted aryl, or substituted or unsubstituted heteroaryl
  MISC_FEATURE (6)..(6): Xaa is Pen
  MISC_FEATURE (7)..(7): Phe is Phe[4-(2-aminoethoxy)
  MISC_FEATURE (8)..(8): Xaa is 2-Nal, Phe(2-Me), Phe(3-Me), Phe(4-Me), Phe(3,4-dimethoxy), 2Quin, 3Quin, 1-Nal, unsubstituted Trp, or Trp substituted with cyano, halo, alkyl, haloalkyl, hydroxy, or alkoxy
  MISC_FEATURE (9)..(9): Xaa is 4-amino-4-carboxy-tetrahydropyran (THP), Acvc, alpha-MeLys, alpha-MeLeu, alpha-MeArg, alpha-MePhe, alpha-MeLeu, alpha-MeLys, alpha-MeAsn, alpha-MeTyr, Ala, cyclohexylAla, Lys, or Aib
  MISC_FEATURE (10)..(11): Xaa is any amino acid
  MISC_FEATURE (12)..(12): Xaa is any amino acid
  MISC_FEATURE (13)..(13): Tyr is (D)NMeTyr
XQTXQXFXXXXXY

SEQ ID NO: 464 - protein, 13 aa, Artificial sequence
  Synthetic construct
  MISC_FEATURE (1)..(1): Xaa is Abu
  MISC_FEATURE (4)..(4): Xaa is is unsubstituted Trp, or Trp substituted with cyano, halo, alkyl, haloalkyl, hydroxy, alkoxy, substituted or unsubstituted aryl, or substituted or unsubstituted heteroaryl
  MISC_FEATURE (7)..(7): Phe is Phe[4-(2-aminoethoxy)
  MISC_FEATURE (8)..(8): Xaa is 2-Nal, Phe(2-Me), Phe(3-Me), Phe(4-Me), Phe(3,4-dimethoxy), 2Quin, 3Quin, 1-Nal, unsubstituted Trp, or Trp substituted with cyano, halo, alkyl, haloalkyl, hydroxy, or alkoxy
  MISC_FEATURE (9)..(9): Xaa is 4-amino-4-carboxy-tetrahydropyran (THP), Acvc, alpha-MeLys, alpha-MeLeu, alpha-MeArg, alpha-MePhe, alpha-MeLeu, alpha-MeLys, alpha-MeAsn, alpha-MeTyr, Ala, cyclohexylAla, Lys, or Aib
  MISC_FEATURE (10)..(11): Xaa is any amino acid
  MISC_FEATURE (12)..(12): Xaa is any amino acid
  MISC_FEATURE (13)..(13): Tyr is (D)NMeTyr
XNTXQCFXXXXXY

SEQ ID NO: 465 - protein, 13 aa, Artificial sequence
  Synthetic construct
  MISC_FEATURE (1)..(1): Xaa is Abu
  MISC_FEATURE (4)..(4): Xaa is is unsubstituted Trp, or Trp substituted with cyano, halo, alkyl, haloalkyl, hydroxy, alkoxy, substituted or unsubstituted aryl, or substituted or unsubstituted heteroaryl
  MISC_FEATURE (6)..(6): Xaa is Pen
  MISC_FEATURE (7)..(7): Phe is Phe[4-(2-aminoethoxy)
  MISC_FEATURE (8)..(8): Xaa is 2-Nal, Phe(2-Me), Phe(3-Me), Phe(4-Me), Phe(3,4-dimethoxy), 2Quin, 3Quin, 1-Nal, unsubstituted Trp, or Trp substituted with cyano, halo, alkyl, haloalkyl, hydroxy, or alkoxy
  MISC_FEATURE (9)..(9): Xaa is 4-amino-4-carboxy-tetrahydropyran (THP), Acvc, alpha-MeLys, alpha-MeLeu, alpha-MeArg, alpha-MePhe, alpha-MeLeu, alpha-MeLys, alpha-MeAsn, alpha-MeTyr, Ala, cyclohexylAla, Lys, or Aib
  MISC_FEATURE (10)..(11): Xaa is any amino acid
  MISC_FEATURE (12)..(12): Xaa is any amino acid
  MISC_FEATURE (13)..(13): Tyr is (D)NMeTyr
XQTXQXFXXXXXY

SEQ ID NO: 466 - protein, 13 aa, Artificial sequence
  Synthetic construct
  MISC_FEATURE (1)..(1): Xaa is Pen
  MISC_FEATURE (4)..(4): Xaa is is unsubstituted Trp, or Trp substituted with cyano, halo, alkyl, haloalkyl, hydroxy, alkoxy, substituted or unsubstituted aryl, or substituted or unsubstituted heteroaryl
  MISC_FEATURE (6)..(6): Xaa is Pen
  MISC_FEATURE (7)..(7): Phe is Phe[4-(2-aminoethoxy)
  MISC_FEATURE (8)..(8): Xaa is 2-Nal, Phe(2-Me), Phe(3-Me), Phe(4-Me), Phe(3,4-dimethoxy), 2Quin, 3Quin, 1-Nal, unsubstituted Trp, or Trp substituted with cyano, halo, alkyl, haloalkyl, hydroxy, or alkoxy
  MISC_FEATURE (9)..(9): Leu is a-MeLeu
  MISC_FEATURE (10)..(10): Lys is Lys(Ac)
  MISC_FEATURE (11)..(11): Xaa is any amino acid
  MISC_FEATURE (12)..(12): Xaa is 2Pal, 3Pal, or 4Pal
  MISC_FEATURE (13)..(13): Xaa is any amino acid
XNTXQXFXLKXXX

SEQ ID NO: 467 - protein, 13 aa, Artificial sequence
  Synthetic construct
  MISC_FEATURE (1)..(1): Xaa is Pen
  MISC_FEATURE (4)..(4): Xaa is is unsubstituted Trp, or Trp substituted with cyano, halo, alkyl, haloalkyl, hydroxy, alkoxy, substituted or unsubstituted aryl, or substituted or unsubstituted heteroaryl
  MISC_FEATURE (6)..(6): Xaa is Pen
  MISC_FEATURE (7)..(7): Phe is Phe[4-(2-aminoethoxy)]
  MISC_FEATURE (8)..(8): Xaa is 2-Nal, Phe(2-Me), Phe(3-Me), Phe(4-Me), Phe(3,4-dimethoxy), 2Quin, 3Quin, 1-Nal, unsubstituted Trp, or Trp substituted with cyano, halo, alkyl, haloalkyl, hydroxy, or alkoxy
  MISC_FEATURE (9)..(9): Leu is a-MeLeu
  MISC_FEATURE (10)..(10): Lys is Lys(Ac)
  MISC_FEATURE (11)..(11): Xaa is any amino acid
  MISC_FEATURE (12)..(12): Xaa is 2Pal, 3Pal, or 4Pal
  MISC_FEATURE (13)..(13): Xaa is any amino acid
XQTXQXFXLKXXX

SEQ ID NO: 468 - protein, 13 aa, Artificial sequence
  Synthetic construct
  MISC_FEATURE (1)..(1): Xaa is Abu
  MISC_FEATURE (4)..(4): Xaa is is unsubstituted Trp, or Trp substituted with cyano, halo, alkyl, haloalkyl, hydroxy, alkoxy, substituted or unsubstituted aryl, or substituted or unsubstituted heteroaryl
  MISC_FEATURE (7)..(7): Phe is Phe[4-(2-aminoethoxy)]
  MISC_FEATURE (8)..(8): Xaa is 2-Nal, Phe(2-Me), Phe(3-Me), Phe(4-Me), Phe(3,4-dimethoxy), 2Quin, 3Quin, 1-Nal, unsubstituted Trp, or Trp substituted with cyano, halo, alkyl, haloalkyl, hydroxy, or alkoxy
  MISC_FEATURE (9)..(9): Leu is a-MeLeu
  MISC_FEATURE (10)..(10): Lys is Lys(Ac)
  MISC_FEATURE (11)..(11): Xaa is any amino acid
  MISC_FEATURE (12)..(12): Xaa is 2Pal, 3Pal, or 4Pal
  MISC_FEATURE (13)..(13): Xaa is any amino acid
XNTXQCFXLKXXX

SEQ ID NO: 469 - protein, 13 aa, Artificial sequence
  Synthetic construct
  MISC_FEATURE (1)..(1): Xaa is Abu
  MISC_FEATURE (4)..(4): Xaa is is unsubstituted Trp, or Trp substituted with cyano, halo, alkyl, haloalkyl, hydroxy, alkoxy, substituted or unsubstituted aryl, or substituted or unsubstituted heteroaryl
  MISC_FEATURE (6)..(6): Xaa is Pen
  MISC_FEATURE (7)..(7): Phe is Phe[4-(2-aminoethoxy)]
  MISC_FEATURE (8)..(8): Xaa is 2-Nal, Phe(2-Me), Phe(3-Me), Phe(4-Me), Phe(3,4-dimethoxy), 2Quin, 3Quin, 1-Nal, unsubstituted Trp, or Trp substituted with cyano, halo, alkyl, haloalkyl, hydroxy, or alkoxy
  MISC_FEATURE (9)..(9): Leu is a-MeLeu
  MISC_FEATURE (10)..(10): Lys is Lys(Ac)
  MISC_FEATURE (11)..(11): Xaa is any amino acid
  MISC_FEATURE (12)..(12): Xaa is 2Pal, 3Pal, or 4Pal
  MISC_FEATURE (13)..(13): Xaa is any amino acid
XQTXQXFXLKXXX

SEQ ID NO: 470 - protein, 13 aa, Artificial sequence
  Synthetic construct
  MISC_FEATURE (1)..(1): Xaa is Pen
  MISC_FEATURE (4)..(4): Xaa is is unsubstituted Trp, or Trp substituted with cyano, halo, alkyl, haloalkyl, hydroxy, alkoxy, substituted or unsubstituted aryl, or substituted or unsubstituted heteroaryl
  MISC_FEATURE (6)..(6): Xaa is Pen
  MISC_FEATURE (7)..(7): Phe is Phe[4-(2-aminoethoxy)]
  MISC_FEATURE (8)..(8): Xaa is 2-Nal, Phe(2-Me), Phe(3-Me), Phe(4-Me), Phe(3,4-dimethoxy), 2Quin, 3Quin, 1-Nal, unsubstituted Trp, or Trp substituted with cyano, halo, alkyl, haloalkyl, hydroxy, or alkoxy
  MISC_FEATURE (9)..(9): Leu is a-MeLeu
  MISC_FEATURE (10)..(10): Lys is Lys(Ac)
  MISC_FEATURE (11)..(12): Xaa is any amino acid
  MISC_FEATURE (13)..(13): Xaa is Sarc
XNTXQXFXLKXXX

SEQ ID NO: 471 - protein, 13 aa, Artificial sequence
  Synthetic construct
  MISC_FEATURE (1)..(1): Xaa is Pen
  MISC_FEATURE (4)..(4): Xaa is is unsubstituted Trp, or Trp substituted with cyano, halo, alkyl, haloalkyl, hydroxy, alkoxy, substituted or unsubstituted aryl, or substituted or unsubstituted heteroaryl
  MISC_FEATURE (6)..(6): Xaa is Pen
  MISC_FEATURE (7)..(7): Phe is Phe[4-(2-aminoethoxy)]
  MISC_FEATURE (8)..(8): Xaa is 2-Nal, Phe(2-Me), Phe(3-Me), Phe(4-Me), Phe(3,4-dimethoxy), 2Quin, 3Quin, 1-Nal, unsubstituted Trp, or Trp substituted with cyano, halo, alkyl, haloalkyl, hydroxy, or alkoxy
  MISC_FEATURE (9)..(9): Leu is a-MeLeu
  MISC_FEATURE (10)..(10): Lys is Lys(Ac)
  MISC_FEATURE (11)..(12): Xaa is any amino acid
  MISC_FEATURE (13)..(13): Xaa is Sarc
XQTXQXFXLKXXX

SEQ ID NO: 472 - protein, 13 aa, Artificial sequence
  Synthetic construct
  MISC_FEATURE (1)..(1): Xaa is Abu
  MISC_FEATURE (4)..(4): Xaa is is unsubstituted Trp, or Trp substituted with cyano, halo, alkyl, haloalkyl, hydroxy, alkoxy, substituted or unsubstituted aryl, or substituted or unsubstituted heteroaryl
  MISC_FEATURE (7)..(7): Phe is Phe[4-(2-aminoethoxy)]
  MISC_FEATURE (8)..(8): Xaa is 2-Nal, Phe(2-Me), Phe(3-Me), Phe(4-Me), Phe(3,4-dimethoxy), 2Quin, 3Quin, 1-Nal, unsubstituted Trp, or Trp substituted with cyano, halo, alkyl, haloalkyl, hydroxy, or alkoxy
  MISC_FEATURE (9)..(9): Leu is a-MeLeu
  MISC_FEATURE (10)..(10): Lys is Lys(Ac)
  MISC_FEATURE (11)..(12): Xaa is any amino acid
  MISC_FEATURE (13)..(13): Xaa is Sarc
XNTXQCFXLKXXX

SEQ ID NO: 473 - protein, 13 aa, Artificial sequence
  Synthetic construct
  MISC_FEATURE (1)..(1): Xaa is Abu
  MISC_FEATURE (4)..(4): Xaa is is unsubstituted Trp, or Trp substituted with cyano, halo, alkyl, haloalkyl, hydroxy, alkoxy, substituted or unsubstituted aryl, or substituted or unsubstituted heteroaryl
  MISC_FEATURE (6)..(6): Xaa is Pen
  MISC_FEATURE (7)..(7): Phe is Phe[4-(2-aminoethoxy)]
  MISC_FEATURE (8)..(8): Xaa is 2-Nal, Phe(2-Me), Phe(3-Me), Phe(4-Me), Phe(3,4-dimethoxy), 2Quin, 3Quin, 1-Nal, unsubstituted Trp, or Trp substituted with cyano, halo, alkyl, haloalkyl, hydroxy, or alkoxy
  MISC_FEATURE (9)..(9): Leu is a-MeLeu
  MISC_FEATURE (10)..(10): Lys is Lys(Ac)
  MISC_FEATURE (11)..(12): Xaa is any amino acid
  MISC_FEATURE (13)..(13): Xaa is Sarc
XQTXQXFXLKXXX

SEQ ID NO: 474 - protein, 13 aa, Artificial sequence
  Synthetic construct
  MISC_FEATURE (1)..(1): Xaa is Pen
  MISC_FEATURE (4)..(4): Xaa is is unsubstituted Trp, or Trp substituted with cyano, halo, alkyl, haloalkyl, hydroxy, alkoxy, substituted or unsubstituted aryl, or substituted or unsubstituted heteroaryl
  MISC_FEATURE (6)..(6): Xaa is Pen
  MISC_FEATURE (7)..(7): Phe is Phe[4-(2-aminoethoxy)]
  MISC_FEATURE (8)..(8): Xaa is 2-Nal, Phe(2-Me), Phe(3-Me), Phe(4-Me), Phe(3,4-dimethoxy), 2Quin, 3Quin, 1-Nal, unsubstituted Trp, or Trp substituted with cyano, halo, alkyl, haloalkyl, hydroxy, or alkoxy
  MISC_FEATURE (9)..(9): Leu is a-MeLeu
  MISC_FEATURE (10)..(10): Lys is Lys(Ac)
  MISC_FEATURE (11)..(12): Xaa is any amino acid
  MISC_FEATURE (13)..(13): Tyr is (D)NMeTyr
XNTXQXFXLKXXY

SEQ ID NO: 475 - protein, 13 aa, Artificial sequence
  Synthetic construct
  MISC_FEATURE (1)..(1): Xaa is Pen
  MISC_FEATURE (4)..(4): Xaa is is unsubstituted Trp, or Trp substituted with cyano, halo, alkyl, haloalkyl, hydroxy, alkoxy, substituted or unsubstituted aryl, or substituted or unsubstituted heteroaryl
  MISC_FEATURE (6)..(6): Xaa is Pen
  MISC_FEATURE (7)..(7): Phe is Phe[4-(2-aminoethoxy)]
  MISC_FEATURE (8)..(8): Xaa is 2-Nal, Phe(2-Me), Phe(3-Me), Phe(4-Me), Phe(3,4-dimethoxy), 2Quin, 3Quin, 1-Nal, unsubstituted Trp, or Trp substituted with cyano, halo, alkyl, haloalkyl, hydroxy, or alkoxy
  MISC_FEATURE (9)..(9): Leu is a-MeLeu
  MISC_FEATURE (10)..(10): Lys is Lys(Ac)
  MISC_FEATURE (11)..(12): Xaa is any amino acid
  MISC_FEATURE (13)..(13): Tyr is (D)NMeTyr
XQTXQXFXLKXXY

SEQ ID NO: 476 - protein, 13 aa, Artificial sequence
  Synthetic construct
  MISC_FEATURE (1)..(1): Xaa is Pen
  MISC_FEATURE (4)..(4): Xaa is is unsubstituted Trp, or Trp substituted with cyano, halo, alkyl, haloalkyl, hydroxy, alkoxy, substituted or unsubstituted aryl, or substituted or unsubstituted heteroaryl
  MISC_FEATURE (7)..(7): Phe is Phe[4-(2-aminoethoxy)]
  MISC_FEATURE (8)..(8): Xaa is 2-Nal, Phe(2-Me), Phe(3-Me), Phe(4-Me), Phe(3,4-dimethoxy), 2Quin, 3Quin, 1-Nal, unsubstituted Trp, or Trp substituted with cyano, halo, alkyl, haloalkyl, hydroxy, or alkoxy
  MISC_FEATURE (9)..(9): Leu is a-MeLeu
  MISC_FEATURE (10)..(10): Lys is Lys(Ac)
  MISC_FEATURE (11)..(12): Xaa is any amino acid
  MISC_FEATURE (13)..(13): Tyr is (D)NMeTyr
XNTXQCFXLKXXY

SEQ ID NO: 477 - protein, 13 aa, Artificial sequence
  Synthetic construct
  MISC_FEATURE (1)..(1): Xaa is Abu
  MISC_FEATURE (4)..(4): Xaa is is unsubstituted Trp, or Trp substituted with cyano, halo, alkyl, haloalkyl, hydroxy, alkoxy, substituted or unsubstituted aryl, or substituted or unsubstituted heteroaryl
  MISC_FEATURE (6)..(6): Xaa is Pen
  MISC_FEATURE (7)..(7): Phe is Phe[4-(2-aminoethoxy)]
  MISC_FEATURE (8)..(8): Xaa is 2-Nal, Phe(2-Me), Phe(3-Me), Phe(4-Me), Phe(3,4-dimethoxy), 2Quin, 3Quin, 1-Nal, unsubstituted Trp, or Trp substituted with cyano, halo, alkyl, haloalkyl, hydroxy, or alkoxy
  MISC_FEATURE (9)..(9): Leu is a-MeLeu
  MISC_FEATURE (10)..(10): Lys is Lys(Ac)
  MISC_FEATURE (11)..(12): Xaa is any amino acid
  MISC_FEATURE (13)..(13): Tyr is (D)NMeTyr
XQTXQXFXLKXXY

SEQ ID NO: 478 - protein, 13 aa, Artificial sequence
  Synthetic construct
  MISC_FEATURE (1)..(1): Xaa is Pen
  MISC_FEATURE (4)..(4): Xaa is is unsubstituted Trp, or Trp substituted with cyano, halo, alkyl, haloalkyl, hydroxy, alkoxy, substituted or unsubstituted aryl, or substituted or unsubstituted heteroaryl
  MISC_FEATURE (6)..(6): Xaa is Pen
  MISC_FEATURE (7)..(7): Phe is Phe[4-(2-aminoethoxy)]
  MISC_FEATURE (8)..(8): Xaa is 2-Nal, Phe(2-Me), Phe(3-Me), Phe(4-Me), Phe(3,4-dimethoxy), 2Quin, 3Quin, 1-Nal, unsubstituted Trp, or Trp substituted with cyano, halo, alkyl, haloalkyl, hydroxy, or alkoxy
  MISC_FEATURE (9)..(9): Leu is a-MeLeu
  MISC_FEATURE (10)..(10): Lys is Lys(Ac)
  MISC_FEATURE (12)..(12): Xaa is 2Pal, 3Pal, or 4Pal
  MISC_FEATURE (13)..(13): Xaa is any amino acid
XNTXQXFXLKNXX

SEQ ID NO: 479 - protein, 13 aa, Artificial sequence
  Synthetic construct
  MISC_FEATURE (1)..(1): Xaa is Pen
  MISC_FEATURE (4)..(4): Xaa is is unsubstituted Trp, or Trp substituted with cyano, halo, alkyl, haloalkyl, hydroxy, alkoxy, substituted or unsubstituted aryl, or substituted or unsubstituted heteroaryl
  MISC_FEATURE (6)..(6): Xaa is Pen
  MISC_FEATURE (7)..(7): Phe is Phe[4-(2-aminoethoxy)]
  MISC_FEATURE (8)..(8): Xaa is 2-Nal, Phe(2-Me), Phe(3-Me), Phe(4-Me), Phe(3,4-dimethoxy), 2Quin, 3Quin, 1-Nal, unsubstituted Trp, or Trp substituted with cyano, halo, alkyl, haloalkyl, hydroxy, or alkoxy
  MISC_FEATURE (9)..(9): Leu is a-MeLeu
  MISC_FEATURE (10)..(10): Lys is Lys(Ac)
  MISC_FEATURE (12)..(12): Xaa is 2Pal, 3Pal, or 4Pal
  MISC_FEATURE (13)..(13): Xaa is any amino acid
XQTXQXFXLKNXX

SEQ ID NO: 480 - protein, 13 aa, Artificial sequence
  Synthetic construct
  MISC_FEATURE (1)..(1): Xaa is Abu
  MISC_FEATURE (4)..(4): Xaa is is unsubstituted Trp, or Trp substituted with cyano, halo, alkyl, haloalkyl, hydroxy, alkoxy, substituted or unsubstituted aryl, or substituted or unsubstituted heteroaryl
  MISC_FEATURE (7)..(7): Phe is Phe[4-(2-aminoethoxy)]
  MISC_FEATURE (8)..(8): Xaa is 2-Nal, Phe(2-Me), Phe(3-Me), Phe(4-Me), Phe(3,4-dimethoxy), 2Quin, 3Quin, 1-Nal, unsubstituted Trp, or Trp substituted with cyano, halo, alkyl, haloalkyl, hydroxy, or alkoxy
  MISC_FEATURE (9)..(9): Leu is a-MeLeu
  MISC_FEATURE (10)..(10): Lys is Lys(Ac)
  MISC_FEATURE (12)..(12): Xaa is 2Pal, 3Pal, or 4Pal
  MISC_FEATURE (13)..(13): Xaa is any amino acid
XNTXQCFXLKNXX

SEQ ID NO: 481 - protein, 13 aa, Artificial sequence
  Synthetic construct
  MISC_FEATURE (1)..(1): Xaa is Abu
  MISC_FEATURE (4)..(4): Xaa is is unsubstituted Trp, or Trp substituted with cyano, halo, alkyl, haloalkyl, hydroxy, alkoxy, substituted or unsubstituted aryl, or substituted or unsubstituted heteroaryl
  MISC_FEATURE (6)..(6): Xaa is Pen
  MISC_FEATURE (7)..(7): Phe is Phe[4-(2-aminoethoxy)]
  MISC_FEATURE (8)..(8): Xaa is 2-Nal, Phe(2-Me), Phe(3-Me), Phe(4-Me), Phe(3,4-dimethoxy), 2Quin, 3Quin, 1-Nal, unsubstituted Trp, or Trp substituted with cyano, halo, alkyl, haloalkyl, hydroxy, or alkoxy
  MISC_FEATURE (9)..(9): Leu is a-MeLeu
  MISC_FEATURE (10)..(10): Lys is Lys(Ac)
  MISC_FEATURE (12)..(12): Xaa is 2Pal, 3Pal, or 4Pal
  MISC_FEATURE (13)..(13): Xaa is any amino acid
XQTXQXFXLKNXX

SEQ ID NO: 482 - protein, 13 aa, Artificial sequence
  Synthetic construct
  MISC_FEATURE (1)..(1): Xaa is Pen
  MISC_FEATURE (4)..(4): Xaa is is unsubstituted Trp, or Trp substituted with cyano, halo, alkyl, haloalkyl, hydroxy, alkoxy, substituted or unsubstituted aryl, or substituted or unsubstituted heteroaryl
  MISC_FEATURE (6)..(6): Xaa is Pen
  MISC_FEATURE (7)..(7): Phe is Phe[4-(2-aminoethoxy)]
  MISC_FEATURE (8)..(8): Xaa is 2-Nal, Phe(2-Me), Phe(3-Me), Phe(4-Me), Phe(3,4-dimethoxy), 2Quin, 3Quin, 1-Nal, unsubstituted Trp, or Trp substituted with cyano, halo, alkyl, haloalkyl, hydroxy, or alkoxy
  MISC_FEATURE (9)..(9): Leu is a-MeLeu
  MISC_FEATURE (10)..(10): Lys is Lys(Ac)
  MISC_FEATURE (12)..(12): Xaa is any amino acid
  MISC_FEATURE (13)..(13): Xaa is Sarc
XNTXQXFXLKNXX

SEQ ID NO: 483 - protein, 13 aa, Artificial sequence
  Synthetic construct
  MISC_FEATURE (1)..(1): Xaa is Pen
  MISC_FEATURE (4)..(4): Xaa is is unsubstituted Trp, or Trp substituted with cyano, halo, alkyl, haloalkyl, hydroxy, alkoxy, substituted or unsubstituted aryl, or substituted or unsubstituted heteroaryl
  MISC_FEATURE (6)..(6): Xaa is Pen
  MISC_FEATURE (7)..(7): Phe is Phe[4-(2-aminoethoxy)]
  MISC_FEATURE (8)..(8): Xaa is 2-Nal, Phe(2-Me), Phe(3-Me), Phe(4-Me), Phe(3,4-dimethoxy), 2Quin, 3Quin, 1-Nal, unsubstituted Trp, or Trp substituted with cyano, halo, alkyl, haloalkyl, hydroxy, or alkoxy
  MISC_FEATURE (9)..(9): Leu is a-MeLeu
  MISC_FEATURE (10)..(10): Lys is Lys(Ac)
  MISC_FEATURE (12)..(12): Xaa is any amino acid
  MISC_FEATURE (13)..(13): Xaa is Sarc
XQTXQXFXLKNXX

SEQ ID NO: 484 - protein, 13 aa, Artificial sequence
  Synthetic construct
  MISC_FEATURE (1)..(1): Xaa is Abu
  MISC_FEATURE (4)..(4): Xaa is is unsubstituted Trp, or Trp substituted with cyano, halo, alkyl, haloalkyl, hydroxy, alkoxy, substituted or unsubstituted aryl, or substituted or unsubstituted heteroaryl
  MISC_FEATURE (7)..(7): Phe is Phe[4-(2-aminoethoxy)]
  MISC_FEATURE (8)..(8): Xaa is 2-Nal, Phe(2-Me), Phe(3-Me), Phe(4-Me), Phe(3,4-dimethoxy), 2Quin, 3Quin, 1-Nal, unsubstituted Trp, or Trp substituted with cyano, halo, alkyl, haloalkyl, hydroxy, or alkoxy
  MISC_FEATURE (9)..(9): Leu is a-MeLeu
  MISC_FEATURE (10)..(10): Lys is Lys(Ac)
  MISC_FEATURE (12)..(12): Xaa is any amino acid
  MISC_FEATURE (13)..(13): Xaa is Sarc
XNTXQCFXLKNXX

SEQ ID NO: 485 - protein, 13 aa, Artificial sequence
  Synthetic construct
  MISC_FEATURE (1)..(1): Xaa is Abu
  MISC_FEATURE (4)..(4): Xaa is is unsubstituted Trp, or Trp substituted with cyano, halo, alkyl, haloalkyl, hydroxy, alkoxy, substituted or unsubstituted aryl, or substituted or unsubstituted heteroaryl
  MISC_FEATURE (6)..(6): Xaa is Pen
  MISC_FEATURE (7)..(7): Phe is Phe[4-(2-aminoethoxy)]
  MISC_FEATURE (8)..(8): Xaa is 2-Nal, Phe(2-Me), Phe(3-Me), Phe(4-Me), Phe(3,4-dimethoxy), 2Quin, 3Quin, 1-Nal, unsubstituted Trp, or Trp substituted with cyano, halo, alkyl, haloalkyl, hydroxy, or alkoxy
  MISC_FEATURE (9)..(9): Leu is a-MeLeu
  MISC_FEATURE (10)..(10): Lys is Lys(Ac)
  MISC_FEATURE (12)..(12): Xaa is any amino acid
  MISC_FEATURE (13)..(13): Xaa is Sarc
XQTXQXFXLKNXX

SEQ ID NO: 486 - protein, 13 aa, Artificial sequence
  Synthetic construct
  MISC_FEATURE (1)..(1): Xaa is Pen
  MISC_FEATURE (4)..(4): Xaa is is unsubstituted Trp, or Trp substituted with cyano, halo, alkyl, haloalkyl, hydroxy, alkoxy, substituted or unsubstituted aryl, or substituted or unsubstituted heteroaryl
  MISC_FEATURE (6)..(6): Xaa is Pen
  MISC_FEATURE (7)..(7): Phe is Phe[4-(2-aminoethoxy)]
  MISC_FEATURE (8)..(8): Xaa is 2-Nal, Phe(2-Me), Phe(3-Me), Phe(4-Me), Phe(3,4-dimethoxy), 2Quin, 3Quin, 1-Nal, unsubstituted Trp, or Trp substituted with cyano, halo, alkyl, haloalkyl, hydroxy, or alkoxy
  MISC_FEATURE (9)..(9): Leu is a-MeLeu
  MISC_FEATURE (10)..(10): Lys is Lys(Ac)
  MISC_FEATURE (12)..(12): Xaa is any amino acid
  MISC_FEATURE (13)..(13): Tyr is (D)NMeTyr
XNTXQXFXLKNXY

SEQ ID NO: 487 - protein, 13 aa, Artificial sequence
  Synthetic construct
  MISC_FEATURE (1)..(1): Xaa is Pen
  MISC_FEATURE (4)..(4): Xaa is is unsubstituted Trp, or Trp substituted with cyano, halo, alkyl, haloalkyl, hydroxy, alkoxy, substituted or unsubstituted aryl, or substituted or unsubstituted heteroaryl
  MISC_FEATURE (6)..(6): Xaa is Pen
  MISC_FEATURE (7)..(7): Phe is Phe[4-(2-aminoethoxy)]
  MISC_FEATURE (8)..(8): Xaa is 2-Nal, Phe(2-Me), Phe(3-Me), Phe(4-Me), Phe(3,4-dimethoxy), 2Quin, 3Quin, 1-Nal, unsubstituted Trp, or Trp substituted with cyano, halo, alkyl, haloalkyl, hydroxy, or alkoxy
  MISC_FEATURE (9)..(9): Leu is a-MeLeu
  MISC_FEATURE (10)..(10): Lys is Lys(Ac)
  MISC_FEATURE (12)..(12): Xaa is any amino acid
  MISC_FEATURE (13)..(13): Tyr is (D)MeTyr
XQTXQXFXLKNXY

SEQ ID NO: 488 - protein, 13 aa, Artificial sequence
  Synthetic construct
  MISC_FEATURE (1)..(1): Xaa is Abu
  MISC_FEATURE (4)..(4): Xaa is is unsubstituted Trp, or Trp substituted with cyano, halo, alkyl, haloalkyl, hydroxy, alkoxy, substituted or unsubstituted aryl, or substituted or unsubstituted heteroaryl
  MISC_FEATURE (7)..(7): Phe is Phe[4-(2-aminoethoxy)]
  MISC_FEATURE (8)..(8): Xaa is 2-Nal, Phe(2-Me), Phe(3-Me), Phe(4-Me), Phe(3,4-dimethoxy), 2Quin, 3Quin, 1-Nal, unsubstituted Trp, or Trp substituted with cyano, halo, alkyl, haloalkyl, hydroxy, or alkoxy
  MISC_FEATURE (9)..(9): Leu is a-MeLeu
  MISC_FEATURE (10)..(10): Lys is Lys(Ac)
  MISC_FEATURE (12)..(12): Xaa is any amino acid
  MISC_FEATURE (13)..(13): Tyr is (D)MeTyr
XNTXQCFXLKNXY

SEQ ID NO: 489 - protein, 13 aa, Artificial sequence
  Synthetic construct
  MISC_FEATURE (1)..(1): Xaa is Abu
  MISC_FEATURE (4)..(4): Xaa is is unsubstituted Trp, or Trp substituted with cyano, halo, alkyl, haloalkyl, hydroxy, alkoxy, substituted or unsubstituted aryl, or substituted or unsubstituted heteroaryl
  MISC_FEATURE (6)..(6): Xaa is Pen
  MISC_FEATURE (7)..(7): Phe is Phe[4-(2-aminoethoxy)]
  MISC_FEATURE (8)..(8): Xaa is 2-Nal, Phe(2-Me), Phe(3-Me), Phe(4-Me), Phe(3,4-dimethoxy), 2Quin, 3Quin, 1-Nal, unsubstituted Trp, or Trp substituted with cyano, halo, alkyl, haloalkyl, hydroxy, or alkoxy
  MISC_FEATURE (9)..(9): Leu is a-MeLeu
  MISC_FEATURE (10)..(10): Lys is Lys(Ac)
  MISC_FEATURE (12)..(12): Xaa is any amino acid
  MISC_FEATURE (13)..(13): Tyr is (D)NMeTyr
XQTXQXFXLKNXY

SEQ ID NO: 490 - protein, 13 aa, Artificial sequence
  Synthetic construct
  MISC_FEATURE (1)..(1): Xaa is Pen
  MISC_FEATURE (4)..(4): Xaa is W(7-Me)
  MISC_FEATURE (6)..(6): Xaa is Pen
  MISC_FEATURE (7)..(7): Phe is Phe[4-(2-aminoethoxy)]
  MISC_FEATURE (8)..(8): Xaa is 2-Nal, Phe(2-Me), Phe(3-Me), Phe(4-Me), Phe(3,4-dimethoxy), 2Quin, 3Quin, 1-Nal, unsubstituted Trp, or Trp substituted with cyano, halo, alkyl, haloalkyl, hydroxy, or alkoxy
  MISC_FEATURE (9)..(9): Leu is a-MeLeu
  MISC_FEATURE (10)..(10): Lys is Lys(Ac)
  MISC_FEATURE (12)..(12): Xaa is 2Pal, 3Pal, or 4Pal
  MISC_FEATURE (13)..(13): Xaa is any amino acid
XNTXQXFXLKNXX

SEQ ID NO: 491 - protein, 13 aa, Artificial sequence
  Synthetic construct
  MISC_FEATURE (1)..(1): Xaa is Pen
  MISC_FEATURE (4)..(4): Xaa is W(7-Me)
  MISC_FEATURE (6)..(6): Xaa is Pen
  MISC_FEATURE (7)..(7): Phe is Phe[4-(2-aminoethoxy)]
  MISC_FEATURE (8)..(8): Xaa is 2-Nal, Phe(2-Me), Phe(3-Me), Phe(4-Me), Phe(3,4-dimethoxy), 2Quin, 3Quin, 1-Nal, unsubstituted Trp, or Trp substituted with cyano, halo, alkyl, haloalkyl, hydroxy, or alkoxy
  MISC_FEATURE (9)..(9): Leu is a-MeLeu
  MISC_FEATURE (10)..(10): Lys is Lys(Ac)
  MISC_FEATURE (12)..(12): Xaa is 2Pal, 3Pal, or 4Pal
  MISC_FEATURE (13)..(13): Xaa is any amino acid
XQTXQXFXLKNXX

SEQ ID NO: 492 - protein, 13 aa, Artificial sequence
  Synthetic construct
  MISC_FEATURE (1)..(1): Xaa is Abu
  MISC_FEATURE (4)..(4): Xaa is W(7-Me)
  MISC_FEATURE (7)..(7): Phe is Phe[4-(2-aminoethoxy)]
  MISC_FEATURE (7)..(7): Phe is Phe[4-(2-aminoethoxy)]
  MISC_FEATURE (8)..(8): Xaa is 2-Nal, Phe(2-Me), Phe(3-Me), Phe(4-Me), Phe(3,4-dimethoxy), 2Quin, 3Quin, 1-Nal, unsubstituted Trp, or Trp substituted with cyano, halo, alkyl, haloalkyl, hydroxy, or alkoxy
  MISC_FEATURE (9)..(9): Leu is a-MeLeu
  MISC_FEATURE (10)..(10): Lys is Lys(Ac)
  MISC_FEATURE (12)..(12): Xaa is 2Pal, 3Pal, or 4Pal
  MISC_FEATURE (13)..(13): Xaa is any amino acid
XNTXQCFXLKNXX

SEQ ID NO: 493 - protein, 13 aa, Artificial sequence
  Synthetic construct
  MISC_FEATURE (1)..(1): Xaa is Abu
  MISC_FEATURE (4)..(4): Xaa is W(7-Me)
  MISC_FEATURE (6)..(6): Xaa is Pen
  MISC_FEATURE (7)..(7): Phe is Phe[4-(2-aminoethoxy)]
  MISC_FEATURE (8)..(8): Xaa is 2-Nal, Phe(2-Me), Phe(3-Me), Phe(4-Me), Phe(3,4-dimethoxy), 2Quin, 3Quin, 1-Nal, unsubstituted Trp, or Trp substituted with cyano, halo, alkyl, haloalkyl, hydroxy, or alkoxy
  MISC_FEATURE (9)..(9): Leu is a-MeLeu
  MISC_FEATURE (10)..(10): Lys is Lys(Ac)
  MISC_FEATURE (12)..(12): Xaa is 2Pal, 3Pal, or 4Pal
  MISC_FEATURE (13)..(13): Xaa is any amino acid
XQTXQXFXLKNXX

SEQ ID NO: 494 - protein, 13 aa, Artificial sequence
  Synthetic construct
  MISC_FEATURE (1)..(1): Xaa is Pen
  MISC_FEATURE (4)..(4): Xaa is W(7-Me)
  MISC_FEATURE (6)..(6): Xaa is Pen
  MISC_FEATURE (7)..(7): Phe is Phe[4-(2-aminoethoxy)]
  MISC_FEATURE (8)..(8): Xaa is 2-Nal, Phe(2-Me), Phe(3-Me), Phe(4-Me), Phe(3,4-dimethoxy), 2Quin, 3Quin, 1-Nal, unsubstituted Trp, or Trp substituted with cyano, halo, alkyl, haloalkyl, hydroxy, or alkoxy
  MISC_FEATURE (9)..(9): Leu is a-MeLeu
  MISC_FEATURE (10)..(10): Lys is Lys(Ac)
  MISC_FEATURE (12)..(12): Xaa is any amino acid
  MISC_FEATURE (13)..(13): Xaa is Sarc
XNTXQXFXLKNXX

SEQ ID NO: 495 - protein, 13 aa, Artificial sequence
  Synthetic construct
  MISC_FEATURE (1)..(1): Xaa is Pen
  MISC_FEATURE (4)..(4): Xaa is W(7-Me)
  MISC_FEATURE (6)..(6): Xaa is Pen
  MISC_FEATURE (7)..(7): Phe is Phe[4-(2-aminoethoxy)]
  MISC_FEATURE (8)..(8): Xaa is 2-Nal, Phe(2-Me), Phe(3-Me), Phe(4-Me), Phe(3,4-dimethoxy), 2Quin, 3Quin, 1-Nal, unsubstituted Trp, or Trp substituted with cyano, halo, alkyl, haloalkyl, hydroxy, or alkoxy
  MISC_FEATURE (9)..(9): Leu is a-MeLeu
  MISC_FEATURE (10)..(10): Lys is Lys(Ac)
  MISC_FEATURE (12)..(12): Xaa is any amino acid
  MISC_FEATURE (13)..(13): Xaa is Sarc
XQTXQXFXLKNXX

SEQ ID NO: 496 - protein, 13 aa, Artificial sequence
  Synthetic construct
  MISC_FEATURE (1)..(1): Xaa is Abu
  MISC_FEATURE (4)..(4): Xaa is W(7-Me)
  MISC_FEATURE (7)..(7): Phe is Phe[4-(2-aminoethoxy)]
  MISC_FEATURE (8)..(8): Xaa is 2-Nal, Phe(2-Me), Phe(3-Me), Phe(4-Me), Phe(3,4-dimethoxy), 2Quin, 3Quin, 1-Nal, unsubstituted Trp, or Trp substituted with cyano, halo, alkyl, haloalkyl, hydroxy, or alkoxy
  MISC_FEATURE (9)..(9): Leu is a-MeLeu
  MISC_FEATURE (10)..(10): Lys is Lys(Ac)
  MISC_FEATURE (12)..(12): Xaa is any amino acid
  MISC_FEATURE (13)..(13): Xaa is Sarc
XNTXQCFXLKNXX

SEQ ID NO: 497 - protein, 13 aa, Artificial sequence
  Synthetic construct
  MISC_FEATURE (1)..(1): Xaa is Abu
  MISC_FEATURE (4)..(4): Xaa is W(7-Me)
  MISC_FEATURE (6)..(6): Xaa is Pen
  MISC_FEATURE (7)..(7): Phe is Phe[4-(2-aminoethoxy)]
  MISC_FEATURE (8)..(8): Xaa is 2-Nal, Phe(2-Me), Phe(3-Me), Phe(4-Me), Phe(3,4-dimethoxy), 2Quin, 3Quin, 1-Nal, unsubstituted Trp, or Trp substituted with cyano, halo, alkyl, haloalkyl, hydroxy, or alkoxy
  MISC_FEATURE (9)..(9): Leu is a-MeLeu
  MISC_FEATURE (10)..(10): Lys is Lys(Ac)
  MISC_FEATURE (12)..(12): Xaa is any amino acid
  MISC_FEATURE (13)..(13): Xaa is Sarc
XQTXQXFXLKNXX

SEQ ID NO: 498 - protein, 13 aa, Artificial sequence
  Synthetic construct
  MISC_FEATURE (1)..(1): Xaa is Pen
  MISC_FEATURE (4)..(4): Xaa is W(7-Me)
  MISC_FEATURE (6)..(6): Xaa is Pen
  MISC_FEATURE (7)..(7): Phe is Phe[4-(2-aminoethoxy)]
  MISC_FEATURE (8)..(8): Xaa is 2-Nal, Phe(2-Me), Phe(3-Me), Phe(4-Me), Phe(3,4-dimethoxy), 2Quin, 3Quin, 1-Nal, unsubstituted Trp, or Trp substituted with cyano, halo, alkyl, haloalkyl, hydroxy, or alkoxy
  MISC_FEATURE (9)..(9): Leu is a-MeLeu
  MISC_FEATURE (10)..(10): Lys is Lys(Ac)
  MISC_FEATURE (12)..(12): Xaa is any amino acid
  MISC_FEATURE (13)..(13): Tyr is (D)NMeTyr
XNTXQXFXLKNXY

SEQ ID NO: 499 - protein, 13 aa, Artificial sequence
  Synthetic construct
  MISC_FEATURE (1)..(1): Xaa is Pen
  MISC_FEATURE (4)..(4): Xaa is W(7-Me)
  MISC_FEATURE (6)..(6): Xaa is Pen
  MISC_FEATURE (7)..(7): Phe is Phe[4-(2-aminoethoxy)]
  MISC_FEATURE (8)..(8): Xaa is 2-Nal, Phe(2-Me), Phe(3-Me), Phe(4-Me), Phe(3,4-dimethoxy), 2Quin, 3Quin, 1-Nal, unsubstituted Trp, or Trp substituted with cyano, halo, alkyl, haloalkyl, hydroxy, or alkoxy
  MISC_FEATURE (9)..(9): Leu is a-MeLeu
  MISC_FEATURE (10)..(10): Lys is Lys(Ac)
  MISC_FEATURE (12)..(12): Xaa is any amino acid
  MISC_FEATURE (13)..(13): Tyr is (D)NMeTyr
XQTXQXFXLKNXY

SEQ ID NO: 500 - protein, 13 aa, Artificial sequence
  Synthetic construct
  MISC_FEATURE (1)..(1): Xaa is Abu
  MISC_FEATURE (4)..(4): Xaa is W(7-Me)
  MISC_FEATURE (7)..(7): Phe is Phe[4-(2-aminoethoxy)]
  MISC_FEATURE (8)..(8): Xaa is 2-Nal, Phe(2-Me), Phe(3-Me), Phe(4-Me), Phe(3,4-dimethoxy), 2Quin, 3Quin, 1-Nal, unsubstituted Trp, or Trp substituted with cyano, halo, alkyl, haloalkyl, hydroxy, or alkoxy
  MISC_FEATURE (9)..(9): Leu is a-MeLeu
  MISC_FEATURE (10)..(10): Lys is Lys(Ac)
  MISC_FEATURE (12)..(12): Xaa is any amino acid
  MISC_FEATURE (13)..(13): Tyr is (D)NMeTyr
XNTXQCFXLKNXY

SEQ ID NO: 501 - protein, 13 aa, Artificial sequence
  Synthetic construct
  MISC_FEATURE (1)..(1): Xaa is Abu
  MISC_FEATURE (4)..(4): Xaa is W(7-Me)
  MISC_FEATURE (6)..(6): Xaa is Pen
  MISC_FEATURE (7)..(7): Phe is Phe[4-(2-aminoethoxy)]
  MISC_FEATURE (8)..(8): Xaa is 2-Nal, Phe(2-Me), Phe(3-Me), Phe(4-Me), Phe(3,4-dimethoxy), 2Quin, 3Quin, 1-Nal, unsubstituted Trp, or Trp substituted with cyano, halo, alkyl, haloalkyl, hydroxy, or alkoxy
  MISC_FEATURE (9)..(9): Leu is a-MeLeu
  MISC_FEATURE (10)..(10): Lys is Lys(Ac)
  MISC_FEATURE (12)..(12): Xaa is any amino acid
  MISC_FEATURE (13)..(13): Tyr is (D)NMeTyr
XQTXQXFXLKNXY

SEQ ID NO: 502 - protein, 13 aa, Artificial sequence
  Synthetic construct
  MISC_FEATURE (1)..(1): Xaa is Pen
  MISC_FEATURE (4)..(4): Xaa is W(7-Me)
  MISC_FEATURE (6)..(6): Xaa is Pen
  MISC_FEATURE (7)..(7): Phe is Phe[4-(2-aminoethoxy)]
  MISC_FEATURE (8)..(8): Xaa is 2-Nal
  MISC_FEATURE (9)..(9): Leu is a-MeLeu
  MISC_FEATURE (10)..(10): Lys is Lys(Ac)
  MISC_FEATURE (12)..(12): Xaa is 2Pal, 3Pal, or 4Pal
  MISC_FEATURE (13)..(13): Xaa is any amino acid
XNTXQXFXLKNXX

SEQ ID NO: 503 - protein, 13 aa, Artificial sequence
  Synthetic construct
  MISC_FEATURE (1)..(1): Xaa is Pen
  MISC_FEATURE (4)..(4): Xaa is W(7-Me)
  MISC_FEATURE (6)..(6): Xaa is Pen
  MISC_FEATURE (7)..(7): Phe is Phe[4-(2-aminoethoxy)]
  MISC_FEATURE (8)..(8): Xaa is 2-Nal
  MISC_FEATURE (9)..(9): Leu is a-MeLeu
  MISC_FEATURE (10)..(10): Lys is Lys(Ac)
  MISC_FEATURE (12)..(12): Xaa is 2Pal, 3Pal, or 4Pal
  MISC_FEATURE (13)..(13): Xaa is any amino acid
XQTXQXFXLKNXX

SEQ ID NO: 504 - protein, 13 aa, Artificial sequence
  Synthetic construct
  MISC_FEATURE (1)..(1): Xaa is Abu
  MISC_FEATURE (4)..(4): Xaa is W(7-Me)
  MISC_FEATURE (7)..(7): Phe is Phe[4-(2-aminoethoxy)]
  MISC_FEATURE (8)..(8): Xaa is 2-Nal
  MISC_FEATURE (9)..(9): Leu is a-MeLeu
  MISC_FEATURE (10)..(10): Lys is Lys(Ac)
  MISC_FEATURE (12)..(12): Xaa is 2Pal, 3Pal, or 4Pal
  MISC_FEATURE (13)..(13): Xaa is any amino acid
XNTXQCFXLKNXX

SEQ ID NO: 505 - protein, 13 aa, Artificial sequence
  Synthetic construct
  MISC_FEATURE (1)..(1): Xaa is Abu
  MISC_FEATURE (4)..(4): Xaa is W(7-Me)
  MISC_FEATURE (6)..(6): Xaa is Pen
  MISC_FEATURE (7)..(7): Phe is Phe[4-(2-aminoethoxy)]
  MISC_FEATURE (8)..(8): Xaa is 2-Nal
  MISC_FEATURE (9)..(9): Leu is a-MeLeu
  MISC_FEATURE (10)..(10): Lys is Lys(Ac)
  MISC_FEATURE (12)..(12): Xaa is 2Pal, 3Pal, or 4Pal
  MISC_FEATURE (13)..(13): Xaa is any amino acid
XQTXQXFXLKNXX

SEQ ID NO: 506 - protein, 13 aa, Artificial sequence
  Synthetic construct
  MISC_FEATURE (1)..(1): Xaa is Pen
  MISC_FEATURE (4)..(4): Xaa is W(7-Me)
  MISC_FEATURE (6)..(6): Xaa is Pen
  MISC_FEATURE (7)..(7): Phe is Phe[4-(2-aminoethoxy)]
  MISC_FEATURE (8)..(8): Xaa is 2-Nal
  MISC_FEATURE (9)..(9): Leu is a-MeLeu
  MISC_FEATURE (10)..(10): Lys is Lys(Ac)
  MISC_FEATURE (12)..(12): Xaa is any amino acid
  MISC_FEATURE (13)..(13): Xaa is Sarc
XNTXQXFXLKNXX

SEQ ID NO: 507 - protein, 13 aa, Artificial sequence
  Synthetic construct
  MISC_FEATURE (1)..(1): Xaa is Pen
  MISC_FEATURE (4)..(4): Xaa is W(7-Me)
  MISC_FEATURE (6)..(6): Xaa is Pen
  MISC_FEATURE (7)..(7): Phe is Phe[4-(2-aminoethoxy)]
  MISC_FEATURE (8)..(8): Xaa is 2-Nal
  MISC_FEATURE (9)..(9): Leu is a-MeLeu
  MISC_FEATURE (10)..(10): Lys is Lys(Ac)
  MISC_FEATURE (12)..(12): Xaa is any amino acid
  MISC_FEATURE (13)..(13): Xaa is Sarc
XQTXQXFXLKNXX

SEQ ID NO: 508 - protein, 13 aa, Artificial sequence
  Synthetic construct
  MISC_FEATURE (1)..(1): Xaa is Abu
  MISC_FEATURE (4)..(4): Xaa is W(7-Me)
  MISC_FEATURE (7)..(7): Phe is Phe[4-(2-aminoethoxy)]
  MISC_FEATURE (8)..(8): Xaa is 2-Nal
  MISC_FEATURE (9)..(9): Leu is a-MeLeu
  MISC_FEATURE (10)..(10): Lys is Lys(Ac)
  MISC_FEATURE (12)..(12): Xaa is any amino acid
  MISC_FEATURE (13)..(13): Xaa is Sarc
XNTXQCFXLKNXX

SEQ ID NO: 509 - protein, 13 aa, Artificial sequence
  Synthetic construct
  MISC_FEATURE (1)..(1): Xaa is Abu
  MISC_FEATURE (4)..(4): Xaa is W(7-Me)
  MISC_FEATURE (6)..(6): Xaa is Pen
  MISC_FEATURE (7)..(7): Phe is Phe[4-(2-aminoethoxy)]
  MISC_FEATURE (8)..(8): Xaa is 2-Nal
  MISC_FEATURE (9)..(9): Leu is a-MeLeu
  MISC_FEATURE (10)..(10): Lys is Lys(Ac)
  MISC_FEATURE (12)..(12): Xaa is any amino acid
  MISC_FEATURE (13)..(13): Xaa is Sarc
XQTXQXFXLKNXX

SEQ ID NO: 510 - protein, 13 aa, Artificial sequence
  Synthetic construct
  MISC_FEATURE (1)..(1): Xaa is Pen
  MISC_FEATURE (4)..(4): Xaa is W(7-Me)
  MISC_FEATURE (6)..(6): Xaa is Pen
  MISC_FEATURE (7)..(7): Phe is Phe[4-(2-aminoethoxy)]
  MISC_FEATURE (8)..(8): Xaa is 2-Nal
  MISC_FEATURE (9)..(9): Leu is a-MeLeu
  MISC_FEATURE (10)..(10): Lys is Lys(Ac)
  MISC_FEATURE (12)..(12): Xaa is any amino acid
  MISC_FEATURE (13)..(13): Tyr is (D)NMeTyr
XNTXQXFXLKNXY

SEQ ID NO: 511 - protein, 13 aa, Artificial sequence
  Synthetic construct
  MISC_FEATURE (1)..(1): Xaa is Pen
  MISC_FEATURE (4)..(4): Xaa is W(7-Me)
  MISC_FEATURE (6)..(6): Xaa is Pen
  MISC_FEATURE (7)..(7): Phe is Phe[4-(2-aminoethoxy)]
  MISC_FEATURE (8)..(8): Xaa is 2-Nal
  MISC_FEATURE (9)..(9): Leu is a-MeLeu
  MISC_FEATURE (10)..(10): Lys is Lys(Ac)
  MISC_FEATURE (12)..(12): Xaa is any amino acid
  MISC_FEATURE (13)..(13): Tyr is (D)NMeTyr
XQTXQXFXLKNXY

SEQ ID NO: 512 - protein, 13 aa, Artificial sequence
  Synthetic construct
  MISC_FEATURE (1)..(1): Xaa is Abu
  MISC_FEATURE (4)..(4): Xaa is W(7-Me)
  MISC_FEATURE (7)..(7): Phe is Phe[4-(2-aminoethoxy)]
  MISC_FEATURE (8)..(8): Xaa is 2-Nal
  MISC_FEATURE (9)..(9): Leu is a-MeLeu
  MISC_FEATURE (10)..(10): Lys is Lys(Ac)
  MISC_FEATURE (12)..(12): Xaa is any amino acid
  MISC_FEATURE (13)..(13): Tyr is (D)NMeTyr
XNTXQCFXLKNXY

SEQ ID NO: 513 - protein, 13 aa, Artificial sequence
  Synthetic construct
  MISC_FEATURE (1)..(1): Xaa is Abu
  MISC_FEATURE (4)..(4): Xaa is W(7-Me)
  MISC_FEATURE (6)..(6): Xaa is Pen
  MISC_FEATURE (7)..(7): Phe is Phe[4-(2-aminoethoxy)]
  MISC_FEATURE (8)..(8): Xaa is 2-Nal
  MISC_FEATURE (9)..(9): Leu is a-MeLeu
  MISC_FEATURE (10)..(10): Lys is Lys(Ac)
  MISC_FEATURE (12)..(12): Xaa is any amino acid
  MISC_FEATURE (13)..(13): Tyr is (D)NMeTyr
XQTXQXFXLKNXY

SEQ ID NO: 514 - protein, 14 aa, Artificial sequence
  Synthetic construct
  MISC_FEATURE (1)..(1): Xaa is absent or represent any amino acid
  MISC_FEATURE (2)..(2): Xaa is Pen
  MISC_FEATURE (5)..(5): Xaa is is unsubstituted Trp, or Trp substituted with cyano, halo, alkyl, haloalkyl, hydroxy, alkoxy, substituted or unsubstituted aryl, or substituted or unsubstituted heteroaryl
  MISC_FEATURE (6)..(6): Lys is Lys(Ac)
  MISC_FEATURE (7)..(7): Xaa is Pen
  MISC_FEATURE (9)..(14): Xaa is any amino acid as defined in Claim 1
XXNTXKXFXXXXXX

SEQ ID NO: 515 - protein, 14 aa, Artificial sequence
  Synthetic construct
  MISC_FEATURE (1)..(1): Xaa is absent or represents any amino acid
  MISC_FEATURE (2)..(2): Xaa is Pen
  MISC_FEATURE (5)..(5): Xaa is is unsubstituted Trp, or Trp substituted with cyano, halo, alkyl, haloalkyl, hydroxy, alkoxy, substituted or unsubstituted aryl, or substituted or unsubstituted heteroaryl
  MISC_FEATURE (6)..(6): Lys is Lys(Ac)
  MISC_FEATURE (7)..(7): Xaa is Pen
  MISC_FEATURE (8)..(8): Phe is Phe[4-(2-aminoethoxy)]
  MISC_FEATURE (9)..(9): Xaa is 2-Nal
  MISC_FEATURE (10)..(14): Xaa is any amino acid as defined in Claim 1
XXNTXKXFXXXXXX

SEQ ID NO: 516 - protein, 14 aa, Artificial sequence
  Synthetic construct
  MISC_FEATURE (1)..(1): Xaa is absent or represents any amino acid
  MISC_FEATURE (2)..(2): Xaa is Pen
  MISC_FEATURE (5)..(5): Xaa is is unsubstituted Trp, or Trp substituted with cyano, halo, alkyl, haloalkyl, hydroxy, alkoxy, substituted or unsubstituted aryl, or substituted or unsubstituted heteroaryl
  MISC_FEATURE (6)..(6): Lys is Lys(Ac)
  MISC_FEATURE (7)..(7): Xaa is Pen
  MISC_FEATURE (8)..(8): Phe is Phe[4-(2-aminoethoxy)]
  MISC_FEATURE (9)..(9): Xaa is 2-Nal
  MISC_FEATURE (10)..(10): Xaa is THP
  MISC_FEATURE (11)..(14): Xaa is any amino acid as defined in Claim 1
XXNTXKXFXXXXXX

SEQ ID NO: 517 - protein, 14 aa, Artificial sequence
  Synthetic construct
  MISC_FEATURE (1)..(1): Xaa is absent or represents any amino acid
  MISC_FEATURE (2)..(2): Xaa is Pen
  MISC_FEATURE (5)..(5): Xaa is is unsubstituted Trp, or Trp substituted with cyano, halo, alkyl, haloalkyl, hydroxy, alkoxy, substituted or unsubstituted aryl, or substituted or unsubstituted heteroaryl
  MISC_FEATURE (6)..(6): Lys is Lys(Ac)
  MISC_FEATURE (7)..(7): Xaa is Pen
  MISC_FEATURE (8)..(8): Phe is Phe[4-(2-aminoethoxy)]
  MISC_FEATURE (9)..(9): Xaa is 2-Nal
  MISC_FEATURE (10)..(10): Xaa is THP
  MISC_FEATURE (12)..(14): Xaa is any amino acid as defined in Claim 1
XXNTXKXFXXEXXX

SEQ ID NO: 518 - protein, 14 aa, Artificial sequence
  Synthetic construct
  MISC_FEATURE (1)..(1): Xaa is absent or represent any amino acid
  MISC_FEATURE (2)..(2): Xaa is Pen
  MISC_FEATURE (5)..(5): Xaa is is unsubstituted Trp, or Trp substituted with cyano, halo, alkyl, haloalkyl, hydroxy, alkoxy, substituted or unsubstituted aryl, or substituted or unsubstituted heteroaryl
  MISC_FEATURE (6)..(6): Lys is Lys(Ac)
  MISC_FEATURE (7)..(7): Xaa is Pen
  MISC_FEATURE (8)..(8): Phe is Phe[4-(2-aminoethoxy)]
  MISC_FEATURE (9)..(9): Xaa is 2-Nal
  MISC_FEATURE (10)..(10): Xaa is THP
  MISC_FEATURE (13)..(14): Xaa is any amino acid as defined in Claim 1
XXNTXKXFXXENXX

SEQ ID NO: 519 - protein, 14 aa, Artificial sequence
  Synthetic construct
  MISC_FEATURE (1)..(1): Xaa is absent or represents any amino acid
  MISC_FEATURE (2)..(2): Xaa is Pen
  MISC_FEATURE (5)..(5): Xaa is W(7-Me)
  MISC_FEATURE (6)..(6): Lys is Lys(Ac)
  MISC_FEATURE (7)..(7): Xaa is Pen
  MISC_FEATURE (8)..(8): Phe is Phe[4-(2-aminoethoxy)]
  MISC_FEATURE (9)..(9): Xaa is 2-Nal
  MISC_FEATURE (10)..(10): Xaa is THP
  MISC_FEATURE (13)..(14): Xaa is any amino acid as defined in Claim 1
XXNTXKXFXXENXX

SEQ ID NO: 520 - protein, 13 aa, Artificial sequence
  Synthetic construct
  MISC_FEATURE (1)..(1): Xaa is Pen
  MISC_FEATURE (4)..(4): Xaa is W(7-Me)
  MISC_FEATURE (5)..(5): Lys is Lys(Ac)
  MISC_FEATURE (6)..(6): Xaa is Pen
  MISC_FEATURE (7)..(7): Phe is Phe[4-(2-aminoethoxy)]
  MISC_FEATURE (8)..(8): Xaa is 2-Nal
  MISC_FEATURE (9)..(9): Xaa is THP
  MISC_FEATURE (12)..(13): Xaa is any amino acid as defined in Claim 1
XNTXKXFXXENXX

SEQ ID NO: 521 - protein, 13 aa, Artificial sequence
  Synthetic construct
  MISC_FEATURE (1)..(1): Xaa is Pen
  MISC_FEATURE (4)..(4): Xaa is W(7-Me)
  MISC_FEATURE (5)..(5): Lys is Lys(Ac)
  MISC_FEATURE (6)..(6): Xaa is Pen
  MISC_FEATURE (7)..(7): Phe is Phe[4-(2-aminoethoxy)]
  MISC_FEATURE (8)..(8): Xaa is 2-Nal
  MISC_FEATURE (9)..(9): Xaa is THP
  MISC_FEATURE (12)..(12): Xaa is 3-Pal
  MISC_FEATURE (13)..(13): Xaa is any amino acid
XNTXKXFXXENXX

SEQ ID NO: 522 - protein, 13 aa, Artificial sequence
  Synthetic construct
  MISC_FEATURE (1)..(1): Xaa is Pen
  MISC_FEATURE (4)..(4): Xaa is W(7-Me)
  MISC_FEATURE (5)..(5): Lys is Lys(Ac)
  MISC_FEATURE (6)..(6): Xaa is Pen
  MISC_FEATURE (7)..(7): Phe is Phe[4-(2-aminoethoxy)]
  MISC_FEATURE (8)..(8): Xaa is 2-Nal
  MISC_FEATURE (9)..(9): Xaa is THP
  MISC_FEATURE (12)..(12): Xaa is any amino acid as defined in Claim 1
  MISC_FEATURE (13)..(13): Xaa is Sarc
XNTXKXFXXENXX

SEQ ID NO: 523 - protein, 13 aa, Artificial sequence
  Synthetic construct
  MISC_FEATURE (1)..(1): Xaa is Pen
  MISC_FEATURE (5)..(5): Xaa is Cit
  MISC_FEATURE (6)..(6): Xaa is Pen
  MISC_FEATURE (7)..(7): Phe is Phe[4-(2-aminoethoxy)]
  MISC_FEATURE (8)..(8): Xaa is 2-Nal
  MISC_FEATURE (9)..(9): Xaa is THP
  MISC_FEATURE (12)..(12): Xaa is 3-Pal
  MISC_FEATURE (13)..(13): Xaa is Sarc
XNTWXXFXXENXX

SEQ ID NO: 524 - protein, 13 aa, Artificial sequence
  Synthetic construct
  MISC_FEATURE (1)..(1): Xaa is Pen
  MISC_FEATURE (6)..(6): Xaa is Pen
  MISC_FEATURE (7)..(7): Phe is Phe[4-(2-aminoethoxy)]
  MISC_FEATURE (8)..(8): Xaa is 2-Nal
  MISC_FEATURE (9)..(9): Xaa is THP
  MISC_FEATURE (12)..(12): Xaa is 3-Pal
  MISC_FEATURE (13)..(13): Xaa is Sarc
XNTWQXFXXENXX

SEQ ID NO: 525 - protein, 13 aa, Artificial sequence
  Synthetic construct
  MISC_FEATURE (1)..(1): Xaa is Abu
  MISC_FEATURE (7)..(7): Phe[4-(2-aminoethoxy)]
  MISC_FEATURE (8)..(8): Xaa is 2-Nal
  MISC_FEATURE (9)..(9): Xaa is THP
  MISC_FEATURE (12)..(12): Xaa is 3-Pal
  MISC_FEATURE (13)..(13): Xaa is Sarc
XQTWQCFXXENXX

SEQ ID NO: 526 - protein, 13 aa, Artificial sequence
  Synthetic construct
  MISC_FEATURE (1)..(1): Xaa is Abu
  MISC_FEATURE (7)..(7): Phe[4-(2-aminoethoxy)]
  MISC_FEATURE (8)..(8): Xaa is 2-Nal
  MISC_FEATURE (9)..(9): Lys is a-MeLys
  MISC_FEATURE (10)..(10): Lys is Lys(Ac)
  MISC_FEATURE (12)..(12): Xaa is 3-Pal
  MISC_FEATURE (13)..(13): Xaa is Sarc
XQTWQCFXKKNXX

SEQ ID NO: 527 - protein, 13 aa, Artificial sequence
  Synthetic construct
  MISC_FEATURE (1)..(1): Xaa is Pen
  MISC_FEATURE (5)..(5): Lys is Lys(Ac)
  MISC_FEATURE (6)..(6): Xaa is Pen
  MISC_FEATURE (7)..(7): Phe[4-(2-aminoethoxy)]
  MISC_FEATURE (8)..(8): Xaa is 2-Nal
  MISC_FEATURE (9)..(9): Xaa is THP
  MISC_FEATURE (10)..(10): Lys is Lys(Ac)
  MISC_FEATURE (12)..(12): Xaa is 3-Pal
  MISC_FEATURE (13)..(13): Xaa is Sarc
XNTWKXFXXKNXX

SEQ ID NO: 528 - protein, 13 aa, Artificial sequence
  Synthetic construct
  MISC_FEATURE (1)..(1): Xaa is Pen
  MISC_FEATURE (5)..(5): Lys is Lys(Ac)
  MISC_FEATURE (6)..(6): Xaa is Pen
  MISC_FEATURE (7)..(7): Phe[4-(2-aminoethoxy)]
  MISC_FEATURE (8)..(8): Xaa is 2-Nal
  MISC_FEATURE (9)..(9): Xaa is THP
  MISC_FEATURE (10)..(10): Lys is Lys(Ac)
  MISC_FEATURE (12)..(12): Xaa is 3-Pal
  MISC_FEATURE (13)..(13): Xaa is Sarc
XETWKXFXXKNXX

SEQ ID NO: 529 - protein, 10 aa, Artificial sequence
  Synthetic construct
  MISC_FEATURE (1)..(1): Trp is 7MeTrp
  MISC_FEATURE (2)..(2): Lys is Lys(Ac)
  MISC_FEATURE (3)..(3): Xaa is Pen(Trt)
  MISC_FEATURE (4)..(4): Xaa is AEF
  MISC_FEATURE (5)..(5): Xaa is Nal
  MISC_FEATURE (6)..(6): Xaa is THP
  MISC_FEATURE (7)..(7): Glu is Glu(OtBu)
  MISC_FEATURE (8)..(8): Asn is Asn(Trt)
  MISC_FEATURE (9)..(9): Xaa is 3-Pal
  MISC_FEATURE (10)..(10): Xaa is Sarc
WKXXXXENXX

SEQ ID NO: 530 - protein, 11 aa, Artificial sequence
  Synthetic construct
  MISC_FEATURE (1)..(1): Thr is Thr(tBu)
  MISC_FEATURE (2)..(2): Trp is 7MeTrp
  MISC_FEATURE (3)..(3): Lys is Lys(Ac)
  MISC_FEATURE (4)..(4): Xaa is Pen(Trt)
  MISC_FEATURE (5)..(5): Xaa is AEF
  MISC_FEATURE (6)..(6): Xaa is Nal
  MISC_FEATURE (7)..(7): Xaa is THP
  MISC_FEATURE (8)..(8): Glu is Glu(OtBu)
  MISC_FEATURE (9)..(9): Asn is Asn(Trt)
  MISC_FEATURE (10)..(10): Xaa is 3-Pal
  MISC_FEATURE (11)..(11): Xaa is Sarc
TWKXXXXENXX

SEQ ID NO: 531 - protein, 12 aa, Artificial sequence
  Synthetic construct
  MISC_FEATURE (1)..(1): Asn is Asn(Trt)
  MISC_FEATURE (2)..(2): Thr is Thr(tBu)
  MISC_FEATURE (3)..(3): Trp is 7MeTrp
  MISC_FEATURE (4)..(4): Lys is Lys(Ac)
  MISC_FEATURE (5)..(5): Pen is Pen(Trt)
  MISC_FEATURE (6)..(6): Xaa is AEF
  MISC_FEATURE (7)..(7): Xaa is Nal
  MISC_FEATURE (8)..(8): Xaa is THP
  MISC_FEATURE (9)..(9): Glu is Glu(OtBu)
  MISC_FEATURE (10)..(10): Asn is Asn(Trt)
  MISC_FEATURE (11)..(11): Xaa is 3-Pal
  MISC_FEATURE (12)..(12): Xaa is Sarc
NTWKXXXXENXX

SEQ ID NO: 532 - protein, 13 aa, Artificial sequence
  Synthetic construct
  MISC_FEATURE (1)..(1): Xaa is Pen(Trt)
  MISC_FEATURE (2)..(2): Asn is Asn(Trt)
  MISC_FEATURE (3)..(3): Thr is Thr(tBu)
  MISC_FEATURE (4)..(4): Trp is 7MeTrp
  MISC_FEATURE (5)..(5): Lys is Lys(Ac)
  MISC_FEATURE (6)..(6): Xaa is Pen(trt)
  MISC_FEATURE (7)..(7): Xaa is AEF
  MISC_FEATURE (8)..(8): Xaa is Nal
  MISC_FEATURE (9)..(9): Xaa is THP
  MISC_FEATURE (10)..(10): Glu is Glu(OtBu)
  MISC_FEATURE (11)..(11): Asn is Asn(Trt)
  MISC_FEATURE (12)..(12): Xaa is 3-Pal
  MISC_FEATURE (13)..(13): Xaa is Sarc
XNTWKXXXXENXX

SEQ ID NO: 533 - protein, 11 aa, Artificial sequence
  Synthetic construct
  MISC_FEATURE (1)..(1): Thr is Thr(tBu)
  MISC_FEATURE (2)..(2): Trp is 7PhTrp
  MISC_FEATURE (3)..(3): Lys is Lys(Ac)
  MISC_FEATURE (4)..(4): Xaa is Pen(Trt)
  MISC_FEATURE (5)..(5): Xaa is AEF
  MISC_FEATURE (6)..(6): Xaa is Nal
  MISC_FEATURE (7)..(7): Xaa is THP
  MISC_FEATURE (8)..(8): Glu is Glu(OtBu)
  MISC_FEATURE (9)..(9): Asn is Asn(Trt)
  MISC_FEATURE (10)..(10): Xaa is 3-Pal
  MISC_FEATURE (11)..(11): Xaa is Sarc
TWKXXXXENXX

SEQ ID NO: 534 - protein, 12 aa, Artificial sequence
  Synthetic construct
  MISC_FEATURE (1)..(1): Asn is Asn(Trt)
  MISC_FEATURE (2)..(2): Thr is Thr(tBu)
  MISC_FEATURE (3)..(3): Trp is 7PhTrp
  MISC_FEATURE (4)..(4): Lys is Lys(Ac)
  MISC_FEATURE (5)..(5): Xaa is Pen(Trt)
  MISC_FEATURE (6)..(6): Xaa is AEF
  MISC_FEATURE (7)..(7): Xaa is Nal
  MISC_FEATURE (8)..(8): Xaa is THP
  MISC_FEATURE (9)..(9): Glu is Glu(OtBu)
  MISC_FEATURE (10)..(10): Asn is Asn(Trt)
  MISC_FEATURE (11)..(11): Xaa is 3-Pal
  MISC_FEATURE (12)..(12): Xaa is Sarc
NTWKXXXXENXX

SEQ ID NO: 535 - protein, 13 aa, Artificial sequence
  Synthetic construct
  MISC_FEATURE (1)..(1): Xaa is Pen(Trt)
  MISC_FEATURE (2)..(2): Asn is Asn(Trt)
  MISC_FEATURE (3)..(3): Thr is Thr(tBu)
  MISC_FEATURE (4)..(4): Trp is 7PhTrp
  MISC_FEATURE (5)..(5): Lys is Lys(Ac)
  MISC_FEATURE (6)..(6): Xaa is Pen(Trt)
  MISC_FEATURE (7)..(7): Xaa is AEF
  MISC_FEATURE (8)..(8): Xaa is Nal
  MISC_FEATURE (9)..(9): Xaa is THP
  MISC_FEATURE (10)..(10): Glu is Glu(OtBu)
  MISC_FEATURE (11)..(11): Asn is Asn(Trt)
  MISC_FEATURE (12)..(12): Xaa is 3-Pal
  MISC_FEATURE (13)..(13): Xaa is Sarc
XNTWKXXXXENXX

SEQ ID NO: 536 - protein, 13 aa, Artificial sequence
  Synthetic construct
  MISC_FEATURE (1)..(1): Xaa is Abu
  MISC_FEATURE (4)..(5): Xaa is any amino acid as defined in Claim 1
  MISC_FEATURE (7)..(12): Xaa is any amino acid as defined in Claim 1
  MISC_FEATURE (13)..(13): Tyr is (D)NMeTyr
XNTXXCXXXXXXY